European Patent Application EP 4 368 713 A1, published May 15, 2024. Title: 절단비활성Cas12f1, 절단비활성 Cas12f1 기반 융합 단백질, 이를 포함하는 CRISPR 유전자 조절 시스템, 그 제조방법 및 용도. Applicant: GenKOre Co., Ltd. The sequence listing filed with the application follows.

SEQUENCE LISTING (540 sequences)

SEQ ID NO: 1 - protein, 529 aa, synthetic construct
  REGION 1..529: note = Wild-type Cas12f1 (Cas14a1)
MAKNTITKTLKLRIVRPYNSAEVEKIVADEKNNREKIALEKNKDKVKEACSKHLKVAAYCTTQVERNACLFCKARKLDDKFYQKLRGQFPDAVFWQEISEIFRQLQKQAAEIYNQSLIELYYEIFIKGKGIANASSVEHYLSDVCYTRAAELFKNAAIASGLRSKIKSNFRLKELKNMKSGLPTTKSDNFPIPLVKQKGGQYTGFEISNHNSDFIIKIPFGRWQVKKEIDKYRPWEKFDFEQVQKSPKPISLLLSTQRRKRNKGWSKDEGTEAEIKKVMNGDYQTSYIEVKRGSKIGEKSAWMLNLSIDVPKIDKGVDPSIIGGIDVGVKSPLVCAINNAFSRYSISDNDLFHFNKKMFARRRILLKKNRHKRAGHGAKNKLKPITILTEKSERFRKKLIERWACEIADFFIKNKVGTVQMENLESMKRKEDSYFNIRLRGFWPYAEMQNKIEFKLKQYGIEIRKVAPNNTSKTCSKCGHLNNYFNFEYRKKNKFPHFKCEKCNFKENADYNAALNISNPKLKSTKEEP

SEQ ID NO: 2 - protein, 529 aa, synthetic construct
  REGION 1..529: note = Dead Cas12f1 D326A
MAKNTITKTLKLRIVRPYNSAEVEKIVADEKNNREKIALEKNKDKVKEACSKHLKVAAYCTTQVERNACLFCKARKLDDKFYQKLRGQFPDAVFWQEISEIFRQLQKQAAEIYNQSLIELYYEIFIKGKGIANASSVEHYLSDVCYTRAAELFKNAAIASGLRSKIKSNFRLKELKNMKSGLPTTKSDNFPIPLVKQKGGQYTGFEISNHNSDFIIKIPFGRWQVKKEIDKYRPWEKFDFEQVQKSPKPISLLLSTQRRKRNKGWSKDEGTEAEIKKVMNGDYQTSYIEVKRGSKIGEKSAWMLNLSIDVPKIDKGVDPSIIGGIAVGVKSPLVCAINNAFSRYSISDNDLFHFNKKMFARRRILLKKNRHKRAGHGAKNKLKPITILTEKSERFRKKLIERWACEIADFFIKNKVGTVQMENLESMKRKEDSYFNIRLRGFWPYAEMQNKIEFKLKQYGIEIRKVAPNNTSKTCSKCGHLNNYFNFEYRKKNKFPHFKCEKCNFKENADYNAALNISNPKLKSTKEEP

SEQ ID NO: 3 - protein, 529 aa, synthetic construct
  REGION 1..529: note = Dead Cas12f1 E422A
MAKNTITKTLKLRIVRPYNSAEVEKIVADEKNNREKIALEKNKDKVKEACSKHLKVAAYCTTQVERNACLFCKARKLDDKFYQKLRGQFPDAVFWQEISEIFRQLQKQAAEIYNQSLIELYYEIFIKGKGIANASSVEHYLSDVCYTRAAELFKNAAIASGLRSKIKSNFRLKELKNMKSGLPTTKSDNFPIPLVKQKGGQYTGFEISNHNSDFIIKIPFGRWQVKKEIDKYRPWEKFDFEQVQKSPKPISLLLSTQRRKRNKGWSKDEGTEAEIKKVMNGDYQTSYIEVKRGSKIGEKSAWMLNLSIDVPKIDKGVDPSIIGGIDVGVKSPLVCAINNAFSRYSISDNDLFHFNKKMFARRRILLKKNRHKRAGHGAKNKLKPITILTEKSERFRKKLIERWACEIADFFIKNKVGTVQMANLESMKRKEDSYFNIRLRGFWPYAEMQNKIEFKLKQYGIEIRKVAPNNTSKTCSKCGHLNNYFNFEYRKKNKFPHFKCEKCNFKENADYNAALNISNPKLKSTKEEP

SEQ ID NO: 4 - protein, 529 aa, synthetic construct
  REGION 1..529: note = Dead Cas12f1 R490A
MAKNTITKTLKLRIVRPYNSAEVEKIVADEKNNREKIALEKNKDKVKEACSKHLKVAAYCTTQVERNACLFCKARKLDDKFYQKLRGQFPDAVFWQEISEIFRQLQKQAAEIYNQSLIELYYEIFIKGKGIANASSVEHYLSDVCYTRAAELFKNAAIASGLRSKIKSNFRLKELKNMKSGLPTTKSDNFPIPLVKQKGGQYTGFEISNHNSDFIIKIPFGRWQVKKEIDKYRPWEKFDFEQVQKSPKPISLLLSTQRRKRNKGWSKDEGTEAEIKKVMNGDYQTSYIEVKRGSKIGEKSAWMLNLSIDVPKIDKGVDPSIIGGIDVGVKSPLVCAINNAFSRYSISDNDLFHFNKKMFARRRILLKKNRHKRAGHGAKNKLKPITILTEKSERFRKKLIERWACEIADFFIKNKVGTVQMENLESMKRKEDSYFNIRLRGFWPYAEMQNKIEFKLKQYGIEIRKVAPNNTSKTCSKCGHLNNYFNFEYAKKNKFPHFKCEKCNFKENADYNAALNISNPKLKSTKEEP

SEQ ID NO: 5 - protein, 529 aa, synthetic construct
  REGION 1..529: note = Dead Cas12f1 D510A
MAKNTITKTLKLRIVRPYNSAEVEKIVADEKNNREKIALEKNKDKVKEACSKHLKVAAYCTTQVERNACLFCKARKLDDKFYQKLRGQFPDAVFWQEISEIFRQLQKQAAEIYNQSLIELYYEIFIKGKGIANASSVEHYLSDVCYTRAAELFKNAAIASGLRSKIKSNFRLKELKNMKSGLPTTKSDNFPIPLVKQKGGQYTGFEISNHNSDFIIKIPFGRWQVKKEIDKYRPWEKFDFEQVQKSPKPISLLLSTQRRKRNKGWSKDEGTEAEIKKVMNGDYQTSYIEVKRGSKIGEKSAWMLNLSIDVPKIDKGVDPSIIGGIDVGVKSPLVCAINNAFSRYSISDNDLFHFNKKMFARRRILLKKNRHKRAGHGAKNKLKPITILTEKSERFRKKLIERWACEIADFFIKNKVGTVQMENLESMKRKEDSYFNIRLRGFWPYAEMQNKIEFKLKQYGIEIRKVAPNNTSKTCSKCGHLNNYFNFEYRKKNKFPHFKCEKCNFKENAAYNAALNISNPKLKSTKEEP

SEQ ID NO: 6 - protein, 529 aa, synthetic construct
  REGION 1..529: note = Dead Cas12f1 D510A, I131W
MAKNTITKTLKLRIVRPYNSAEVEKIVADEKNNREKIALEKNKDKVKEACSKHLKVAAYCTTQVERNACLFCKARKLDDKFYQKLRGQFPDAVFWQEISEIFRQLQKQAAEIYNQSLIELYYEIFIKGKGWANASSVEHYLSDVCYTRAAELFKNAAIASGLRSKIKSNFRLKELKNMKSGLPTTKSDNFPIPLVKQKGGQYTGFEISNHNSDFIIKIPFGRWQVKKEIDKYRPWEKFDFEQVQKSPKPISLLLSTQRRKRNKGWSKDEGTEAEIKKVMNGDYQTSYIEVKRGSKIGEKSAWMLNLSIDVPKIDKGVDPSIIGGIDVGVKSPLVCAINNAFSRYSISDNDLFHFNKKMFARRRILLKKNRHKRAGHGAKNKLKPITILTEKSERFRKKLIERWACEIADFFIKNKVGTVQMENLESMKRKEDSYFNIRLRGFWPYAEMQNKIEFKLKQYGIEIRKVAPNNTSKTCSKCGHLNNYFNFEYRKKNKFPHFKCEKCNFKENAAYNAALNISNPKLKSTKEEP

SEQ ID NO: 7 - protein, 529 aa, synthetic construct
  REGION 1..529: note = Dead Cas12f1 D510A, S136Y
MAKNTITKTLKLRIVRPYNSAEVEKIVADEKNNREKIALEKNKDKVKEACSKHLKVAAYCTTQVERNACLFCKARKLDDKFYQKLRGQFPDAVFWQEISEIFRQLQKQAAEIYNQSLIELYYEIFIKGKGIANASYVEHYLSDVCYTRAAELFKNAAIASGLRSKIKSNFRLKELKNMKSGLPTTKSDNFPIPLVKQKGGQYTGFEISNHNSDFIIKIPFGRWQVKKEIDKYRPWEKFDFEQVQKSPKPISLLLSTQRRKRNKGWSKDEGTEAEIKKVMNGDYQTSYIEVKRGSKIGEKSAWMLNLSIDVPKIDKGVDPSIIGGIDVGVKSPLVCAINNAFSRYSISDNDLFHFNKKMFARRRILLKKNRHKRAGHGAKNKLKPITILTEKSERFRKKLIERWACEIADFFIKNKVGTVQMENLESMKRKEDSYFNIRLRGFWPYAEMQNKIEFKLKQYGIEIRKVAPNNTSKTCSKCGHLNNYFNFEYRKKNKFPHFKCEKCNFKENAAYNAALNISNPKLKSTKEEP

SEQ ID NO: 8 - protein, 529 aa, synthetic construct
  REGION 1..529: note = Dead Cas12f1 D510A, I131W/S136Y
MAKNTITKTLKLRIVRPYNSAEVEKIVADEKNNREKIALEKNKDKVKEACSKHLKVAAYCTTQVERNACLFCKARKLDDKFYQKLRGQFPDAVFWQEISEIFRQLQKQAAEIYNQSLIELYYEIFIKGKGWANASYVEHYLSDVCYTRAAELFKNAAIASGLRSKIKSNFRLKELKNMKSGLPTTKSDNFPIPLVKQKGGQYTGFEISNHNSDFIIKIPFGRWQVKKEIDKYRPWEKFDFEQVQKSPKPISLLLSTQRRKRNKGWSKDEGTEAEIKKVMNGDYQTSYIEVKRGSKIGEKSAWMLNLSIDVPKIDKGVDPSIIGGIDVGVKSPLVCAINNAFSRYSISDNDLFHFNKKMFARRRILLKKNRHKRAGHGAKNKLKPITILTEKSERFRKKLIERWACEIADFFIKNKVGTVQMENLESMKRKEDSYFNIRLRGFWPYAEMQNKIEFKLKQYGIEIRKVAPNNTSKTCSKCGHLNNYFNFEYRKKNKFPHFKCEKCNFKENAAYNAALNISNPKLKSTKEEP

SEQ ID NO: 9 - protein, 529 aa, synthetic construct
  REGION 1..529: note = Dead Cas12f1 using X
  SITE 131: note = misc_feature - Xaa can be any naturally occurring amino acid
  SITE 136: note = misc_feature - Xaa can be any naturally occurring amino acid
  SITE 326: note = misc_feature - Xaa can be any naturally occurring amino acid
  SITE 422: note = misc_feature - Xaa can be any naturally occurring amino acid
  SITE 490: note = misc_feature - Xaa can be any naturally occurring amino acid
  SITE 510: note = misc_feature - Xaa can be any naturally occurring amino acid
MAKNTITKTLKLRIVRPYNSAEVEKIVADEKNNREKIALEKNKDKVKEACSKHLKVAAYCTTQVERNACLFCKARKLDDKFYQKLRGQFPDAVFWQEISEIFRQLQKQAAEIYNQSLIELYYEIFIKGKGXANASXVEHYLSDVCYTRAAELFKNAAIASGLRSKIKSNFRLKELKNMKSGLPTTKSDNFPIPLVKQKGGQYTGFEISNHNSDFIIKIPFGRWQVKKEIDKYRPWEKFDFEQVQKSPKPISLLLSTQRRKRNKGWSKDEGTEAEIKKVMNGDYQTSYIEVKRGSKIGEKSAWMLNLSIDVPKIDKGVDPSIIGGIXVGVKSPLVCAINNAFSRYSISDNDLFHFNKKMFARRRILLKKNRHKRAGHGAKNKLKPITILTEKSERFRKKLIERWACEIADFFIKNKVGTVQMXNLESMKRKEDSYFNIRLRGFWPYAEMQNKIEFKLKQYGIEIRKVAPNNTSKTCSKCGHLNNYFNFEYXKKNKFPHFKCEKCNFKENAXYNAALNISNPKLKSTKEEP

SEQ ID NO: 10 - protein, 28 aa, synthetic construct
  REGION 1..28: note = Added sequence of Tnpb
MGEKSSRRRRNGKSGAWTAAITSCVGGK

SEQ ID NO: 11 - protein, 28 aa, synthetic construct
  REGION 1..28: note = Added sequence of 28 random aa
MAGGPGAGSAAPVSSTSSLPLAALNMRV

SEQ ID NO: 12 - protein, 26 aa, synthetic construct
  REGION 1..26: note = Added sequence of 26 random aa
MAGGPGAGSAAPVSSTSSLPLAALNM

SEQ ID NO: 13 - protein, 26 aa, synthetic construct
  REGION 1..26: note = Added sequence of Cas X
MEKRINKIRKKLSADNATKPVSRSGP

SEQ ID NO: 14 - protein, 557 aa, synthetic construct
  REGION 1..557: note = Wild-type TnpB = Variant 1
MGEKSSRRRRNGKSGAWTAAITSCVGGKMAKNTITKTLKLRIVRPYNSAEVEKIVADEKNNREKIALEKNKDKVKEACSKHLKVAAYCTTQVERNACLFCKARKLDDKFYQKLRGQFPDAVFWQEISEIFRQLQKQAAEIYNQSLIELYYEIFIKGKGIANASSVEHYLSDVCYTRAAELFKNAAIASGLRSKIKSNFRLKELKNMKSGLPTTKSDNFPIPLVKQKGGQYTGFEISNHNSDFIIKIPFGRWQVKKEIDKYRPWEKFDFEQVQKSPKPISLLLSTQRRKRNKGWSKDEGTEAEIKKVMNGDYQTSYIEVKRGSKIGEKSAWMLNLSIDVPKIDKGVDPSIIGGIDVGVKSPLVCAINNAFSRYSISDNDLFHFNKKMFARRRILLKKNRHKRAGHGAKNKLKPITILTEKSERFRKKLIERWACEIADFFIKNKVGTVQMENLESMKRKEDSYFNIRLRGFWPYAEMQNKIEFKLKQYGIEIRKVAPNNTSKTCSKCGHLNNYFNFEYRKKNKFPHFKCEKCNFKENADYNAALNISNPKLKSTKEEP

SEQ ID NO: 15 - protein, 557 aa, synthetic construct
  REGION 1..557: note = Dead TnpB D354A
MGEKSSRRRRNGKSGAWTAAITSCVGGKMAKNTITKTLKLRIVRPYNSAEVEKIVADEKNNREKIALEKNKDKVKEACSKHLKVAAYCTTQVERNACLFCKARKLDDKFYQKLRGQFPDAVFWQEISEIFRQLQKQAAEIYNQSLIELYYEIFIKGKGIANASSVEHYLSDVCYTRAAELFKNAAIASGLRSKIKSNFRLKELKNMKSGLPTTKSDNFPIPLVKQKGGQYTGFEISNHNSDFIIKIPFGRWQVKKEIDKYRPWEKFDFEQVQKSPKPISLLLSTQRRKRNKGWSKDEGTEAEIKKVMNGDYQTSYIEVKRGSKIGEKSAWMLNLSIDVPKIDKGVDPSIIGGIAVGVKSPLVCAINNAFSRYSISDNDLFHFNKKMFARRRILLKKNRHKRAGHGAKNKLKPITILTEKSERFRKKLIERWACEIADFFIKNKVGTVQMENLESMKRKEDSYFNIRLRGFWPYAEMQNKIEFKLKQYGIEIRKVAPNNTSKTCSKCGHLNNYFNFEYRKKNKFPHFKCEKCNFKENADYNAALNISNPKLKSTKEEP

SEQ ID NO: 16 - protein, 557 aa, synthetic construct
  REGION 1..557: note = Dead TnpB E450A
MGEKSSRRRRNGKSGAWTAAITSCVGGKMAKNTITKTLKLRIVRPYNSAEVEKIVADEKNNREKIALEKNKDKVKEACSKHLKVAAYCTTQVERNACLFCKARKLDDKFYQKLRGQFPDAVFWQEISEIFRQLQKQAAEIYNQSLIELYYEIFIKGKGIANASSVEHYLSDVCYTRAAELFKNAAIASGLRSKIKSNFRLKELKNMKSGLPTTKSDNFPIPLVKQKGGQYTGFEISNHNSDFIIKIPFGRWQVKKEIDKYRPWEKFDFEQVQKSPKPISLLLSTQRRKRNKGWSKDEGTEAEIKKVMNGDYQTSYIEVKRGSKIGEKSAWMLNLSIDVPKIDKGVDPSIIGGIDVGVKSPLVCAINNAFSRYSISDNDLFHFNKKMFARRRILLKKNRHKRAGHGAKNKLKPITILTEKSERFRKKLIERWACEIADFFIKNKVGTVQMANLESMKRKEDSYFNIRLRGFWPYAEMQNKIEFKLKQYGIEIRKVAPNNTSKTCSKCGHLNNYFNFEYRKKNKFPHFKCEKCNFKENADYNAALNISNPKLKSTKEEP

SEQ ID NO: 17 - protein, 557 aa, synthetic construct
  REGION 1..557: note = Dead TnpB R518A
MGEKSSRRRRNGKSGAWTAAITSCVGGKMAKNTITKTLKLRIVRPYNSAEVEKIVADEKNNREKIALEKNKDKVKEACSKHLKVAAYCTTQVERNACLFCKARKLDDKFYQKLRGQFPDAVFWQEISEIFRQLQKQAAEIYNQSLIELYYEIFIKGKGIANASSVEHYLSDVCYTRAAELFKNAAIASGLRSKIKSNFRLKELKNMKSGLPTTKSDNFPIPLVKQKGGQYTGFEISNHNSDFIIKIPFGRWQVKKEIDKYRPWEKFDFEQVQKSPKPISLLLSTQRRKRNKGWSKDEGTEAEIKKVMNGDYQTSYIEVKRGSKIGEKSAWMLNLSIDVPKIDKGVDPSIIGGIDVGVKSPLVCAINNAFSRYSISDNDLFHFNKKMFARRRILLKKNRHKRAGHGAKNKLKPITILTEKSERFRKKLIERWACEIADFFIKNKVGTVQMENLESMKRKEDSYFNIRLRGFWPYAEMQNKIEFKLKQYGIEIRKVAPNNTSKTCSKCGHLNNYFNFEYAKKNKFPHFKCEKCNFKENADYNAALNISNPKLKSTKEEP

SEQ ID NO: 18 - protein, 557 aa, synthetic construct
  REGION 1..557: note = Dead TnpB D538A
MGEKSSRRRRNGKSGAWTAAITSCVGGKMAKNTITKTLKLRIVRPYNSAEVEKIVADEKNNREKIALEKNKDKVKEACSKHLKVAAYCTTQVERNACLFCKARKLDDKFYQKLRGQFPDAVFWQEISEIFRQLQKQAAEIYNQSLIELYYEIFIKGKGIANASSVEHYLSDVCYTRAAELFKNAAIASGLRSKIKSNFRLKELKNMKSGLPTTKSDNFPIPLVKQKGGQYTGFEISNHNSDFIIKIPFGRWQVKKEIDKYRPWEKFDFEQVQKSPKPISLLLSTQRRKRNKGWSKDEGTEAEIKKVMNGDYQTSYIEVKRGSKIGEKSAWMLNLSIDVPKIDKGVDPSIIGGIDVGVKSPLVCAINNAFSRYSISDNDLFHFNKKMFARRRILLKKNRHKRAGHGAKNKLKPITILTEKSERFRKKLIERWACEIADFFIKNKVGTVQMENLESMKRKEDSYFNIRLRGFWPYAEMQNKIEFKLKQYGIEIRKVAPNNTSKTCSKCGHLNNYFNFEYRKKNKFPHFKCEKCNFKENAAYNAALNISNPKLKSTKEEP

SEQ ID NO: 19 - protein, 557 aa, synthetic construct
  REGION 1..557: note = Dead TnpB D538A, I159W
MGEKSSRRRRNGKSGAWTAAITSCVGGKMAKNTITKTLKLRIVRPYNSAEVEKIVADEKNNREKIALEKNKDKVKEACSKHLKVAAYCTTQVERNACLFCKARKLDDKFYQKLRGQFPDAVFWQEISEIFRQLQKQAAEIYNQSLIELYYEIFIKGKGWANASSVEHYLSDVCYTRAAELFKNAAIASGLRSKIKSNFRLKELKNMKSGLPTTKSDNFPIPLVKQKGGQYTGFEISNHNSDFIIKIPFGRWQVKKEIDKYRPWEKFDFEQVQKSPKPISLLLSTQRRKRNKGWSKDEGTEAEIKKVMNGDYQTSYIEVKRGSKIGEKSAWMLNLSIDVPKIDKGVDPSIIGGIDVGVKSPLVCAINNAFSRYSISDNDLFHFNKKMFARRRILLKKNRHKRAGHGAKNKLKPITILTEKSERFRKKLIERWACEIADFFIKNKVGTVQMENLESMKRKEDSYFNIRLRGFWPYAEMQNKIEFKLKQYGIEIRKVAPNNTSKTCSKCGHLNNYFNFEYRKKNKFPHFKCEKCNFKENAAYNAALNISNPKLKSTKEEP

SEQ ID NO: 20 - protein, 557 aa, synthetic construct
  REGION 1..557: note = Dead TnpB D538A, S164Y
MGEKSSRRRRNGKSGAWTAAITSCVGGKMAKNTITKTLKLRIVRPYNSAEVEKIVADEKNNREKIALEKNKDKVKEACSKHLKVAAYCTTQVERNACLFCKARKLDDKFYQKLRGQFPDAVFWQEISEIFRQLQKQAAEIYNQSLIELYYEIFIKGKGIANASYVEHYLSDVCYTRAAELFKNAAIASGLRSKIKSNFRLKELKNMKSGLPTTKSDNFPIPLVKQKGGQYTGFEISNHNSDFIIKIPFGRWQVKKEIDKYRPWEKFDFEQVQKSPKPISLLLSTQRRKRNKGWSKDEGTEAEIKKVMNGDYQTSYIEVKRGSKIGEKSAWMLNLSIDVPKIDKGVDPSIIGGIDVGVKSPLVCAINNAFSRYSISDNDLFHFNKKMFARRRILLKKNRHKRAGHGAKNKLKPITILTEKSERFRKKLIERWACEIADFFIKNKVGTVQMENLESMKRKEDSYFNIRLRGFWPYAEMQNKIEFKLKQYGIEIRKVAPNNTSKTCSKCGHLNNYFNFEYRKKNKFPHFKCEKCNFKENAAYNAALNISNPKLKSTKEEP

SEQ ID NO: 21 - protein, 557 aa, synthetic construct
  REGION 1..557: note = Dead TnpB D538A, I159W/S164Y
MGEKSSRRRRNGKSGAWTAAITSCVGGKMAKNTITKTLKLRIVRPYNSAEVEKIVADEKNNREKIALEKNKDKVKEACSKHLKVAAYCTTQVERNACLFCKARKLDDKFYQKLRGQFPDAVFWQEISEIFRQLQKQAAEIYNQSLIELYYEIFIKGKGWANASYVEHYLSDVCYTRAAELFKNAAIASGLRSKIKSNFRLKELKNMKSGLPTTKSDNFPIPLVKQKGGQYTGFEISNHNSDFIIKIPFGRWQVKKEIDKYRPWEKFDFEQVQKSPKPISLLLSTQRRKRNKGWSKDEGTEAEIKKVMNGDYQTSYIEVKRGSKIGEKSAWMLNLSIDVPKIDKGVDPSIIGGIDVGVKSPLVCAINNAFSRYSISDNDLFHFNKKMFARRRILLKKNRHKRAGHGAKNKLKPITILTEKSERFRKKLIERWACEIADFFIKNKVGTVQMENLESMKRKEDSYFNIRLRGFWPYAEMQNKIEFKLKQYGIEIRKVAPNNTSKTCSKCGHLNNYFNFEYRKKNKFPHFKCEKCNFKENAAYNAALNISNPKLKSTKEEP

SEQ ID NO: 22 - protein, 557 aa, synthetic construct
  REGION 1..557: note = Dead TnpB D354A, D538A
MGEKSSRRRRNGKSGAWTAAITSCVGGKMAKNTITKTLKLRIVRPYNSAEVEKIVADEKNNREKIALEKNKDKVKEACSKHLKVAAYCTTQVERNACLFCKARKLDDKFYQKLRGQFPDAVFWQEISEIFRQLQKQAAEIYNQSLIELYYEIFIKGKGIANASSVEHYLSDVCYTRAAELFKNAAIASGLRSKIKSNFRLKELKNMKSGLPTTKSDNFPIPLVKQKGGQYTGFEISNHNSDFIIKIPFGRWQVKKEIDKYRPWEKFDFEQVQKSPKPISLLLSTQRRKRNKGWSKDEGTEAEIKKVMNGDYQTSYIEVKRGSKIGEKSAWMLNLSIDVPKIDKGVDPSIIGGIAVGVKSPLVCAINNAFSRYSISDNDLFHFNKKMFARRRILLKKNRHKRAGHGAKNKLKPITILTEKSERFRKKLIERWACEIADFFIKNKVGTVQMENLESMKRKEDSYFNIRLRGFWPYAEMQNKIEFKLKQYGIEIRKVAPNNTSKTCSKCGHLNNYFNFEYRKKNKFPHFKCEKCNFKENAAYNAALNISNPKLKSTKEEP

SEQ ID NO: 23 - protein, 557 aa, synthetic construct
  REGION 1..557: note = Dead TnpB D354A, E450A, R518A
MGEKSSRRRRNGKSGAWTAAITSCVGGKMAKNTITKTLKLRIVRPYNSAEVEKIVADEKNNREKIALEKNKDKVKEACSKHLKVAAYCTTQVERNACLFCKARKLDDKFYQKLRGQFPDAVFWQEISEIFRQLQKQAAEIYNQSLIELYYEIFIKGKGIANASSVEHYLSDVCYTRAAELFKNAAIASGLRSKIKSNFRLKELKNMKSGLPTTKSDNFPIPLVKQKGGQYTGFEISNHNSDFIIKIPFGRWQVKKEIDKYRPWEKFDFEQVQKSPKPISLLLSTQRRKRNKGWSKDEGTEAEIKKVMNGDYQTSYIEVKRGSKIGEKSAWMLNLSIDVPKIDKGVDPSIIGGIAVGVKSPLVCAINNAFSRYSISDNDLFHFNKKMFARRRILLKKNRHKRAGHGAKNKLKPITILTEKSERFRKKLIERWACEIADFFIKNKVGTVQMANLESMKRKEDSYFNIRLRGFWPYAEMQNKIEFKLKQYGIEIRKVAPNNTSKTCSKCGHLNNYFNFEYAKKNKFPHFKCEKCNFKENADYNAALNISNPKLKSTKEEP

SEQ ID NO: 24 - protein, 557 aa, synthetic construct
  REGION 1..557: note = Dead TnpB D354A, E450A, R518A, D538A
MGEKSSRRRRNGKSGAWTAAITSCVGGKMAKNTITKTLKLRIVRPYNSAEVEKIVADEKNNREKIALEKNKDKVKEACSKHLKVAAYCTTQVERNACLFCKARKLDDKFYQKLRGQFPDAVFWQEISEIFRQLQKQAAEIYNQSLIELYYEIFIKGKGIANASSVEHYLSDVCYTRAAELFKNAAIASGLRSKIKSNFRLKELKNMKSGLPTTKSDNFPIPLVKQKGGQYTGFEISNHNSDFIIKIPFGRWQVKKEIDKYRPWEKFDFEQVQKSPKPISLLLSTQRRKRNKGWSKDEGTEAEIKKVMNGDYQTSYIEVKRGSKIGEKSAWMLNLSIDVPKIDKGVDPSIIGGIAVGVKSPLVCAINNAFSRYSISDNDLFHFNKKMFARRRILLKKNRHKRAGHGAKNKLKPITILTEKSERFRKKLIERWACEIADFFIKNKVGTVQMANLESMKRKEDSYFNIRLRGFWPYAEMQNKIEFKLKQYGIEIRKVAPNNTSKTCSKCGHLNNYFNFEYAKKNKFPHFKCEKCNFKENAAYNAALNISNPKLKSTKEEP

SEQ ID NO: 25 - protein, 557 aa, synthetic construct
  REGION 1..557: note = 28aa-extension Cas12f1 = Variant 2
MAGGPGAGSAAPVSSTSSLPLAALNMRVMAKNTITKTLKLRIVRPYNSAEVEKIVADEKNNREKIALEKNKDKVKEACSKHLKVAAYCTTQVERNACLFCKARKLDDKFYQKLRGQFPDAVFWQEISEIFRQLQKQAAEIYNQSLIELYYEIFIKGKGIANASSVEHYLSDVCYTRAAELFKNAAIASGLRSKIKSNFRLKELKNMKSGLPTTKSDNFPIPLVKQKGGQYTGFEISNHNSDFIIKIPFGRWQVKKEIDKYRPWEKFDFEQVQKSPKPISLLLSTQRRKRNKGWSKDEGTEAEIKKVMNGDYQTSYIEVKRGSKIGEKSAWMLNLSIDVPKIDKGVDPSIIGGIDVGVKSPLVCAINNAFSRYSISDNDLFHFNKKMFARRRILLKKNRHKRAGHGAKNKLKPITILTEKSERFRKKLIERWACEIADFFIKNKVGTVQMENLESMKRKEDSYFNIRLRGFWPYAEMQNKIEFKLKQYGIEIRKVAPNNTSKTCSKCGHLNNYFNFEYRKKNKFPHFKCEKCNFKENADYNAALNISNPKLKSTKEEP

SEQ ID NO: 26 - protein, 557 aa, synthetic construct
  REGION 1..557: note = Dead 28-aa extension Cas12f1 D354A
MAGGPGAGSAAPVSSTSSLPLAALNMRVMAKNTITKTLKLRIVRPYNSAEVEKIVADEKNNREKIALEKNKDKVKEACSKHLKVAAYCTTQVERNACLFCKARKLDDKFYQKLRGQFPDAVFWQEISEIFRQLQKQAAEIYNQSLIELYYEIFIKGKGIANASSVEHYLSDVCYTRAAELFKNAAIASGLRSKIKSNFRLKELKNMKSGLPTTKSDNFPIPLVKQKGGQYTGFEISNHNSDFIIKIPFGRWQVKKEIDKYRPWEKFDFEQVQKSPKPISLLLSTQRRKRNKGWSKDEGTEAEIKKVMNGDYQTSYIEVKRGSKIGEKSAWMLNLSIDVPKIDKGVDPSIIGGIAVGVKSPLVCAINNAFSRYSISDNDLFHFNKKMFARRRILLKKNRHKRAGHGAKNKLKPITILTEKSERFRKKLIERWACEIADFFIKNKVGTVQMENLESMKRKEDSYFNIRLRGFWPYAEMQNKIEFKLKQYGIEIRKVAPNNTSKTCSKCGHLNNYFNFEYRKKNKFPHFKCEKCNFKENADYNAALNISNPKLKSTKEEP

SEQ ID NO: 27 - protein, 557 aa, synthetic construct
  REGION 1..557: note = Dead 28-aa extension Cas12f1 E450A
MAGGPGAGSAAPVSSTSSLPLAALNMRVMAKNTITKTLKLRIVRPYNSAEVEKIVADEKNNREKIALEKNKDKVKEACSKHLKVAAYCTTQVERNACLFCKARKLDDKFYQKLRGQFPDAVFWQEISEIFRQLQKQAAEIYNQSLIELYYEIFIKGKGIANASSVEHYLSDVCYTRAAELFKNAAIASGLRSKIKSNFRLKELKNMKSGLPTTKSDNFPIPLVKQKGGQYTGFEISNHNSDFIIKIPFGRWQVKKEIDKYRPWEKFDFEQVQKSPKPISLLLSTQRRKRNKGWSKDEGTEAEIKKVMNGDYQTSYIEVKRGSKIGEKSAWMLNLSIDVPKIDKGVDPSIIGGIDVGVKSPLVCAINNAFSRYSISDNDLFHFNKKMFARRRILLKKNRHKRAGHGAKNKLKPITILTEKSERFRKKLIERWACEIADFFIKNKVGTVQMANLESMKRKEDSYFNIRLRGFWPYAEMQNKIEFKLKQYGIEIRKVAPNNTSKTCSKCGHLNNYFNFEYRKKNKFPHFKCEKCNFKENADYNAALNISNPKLKSTKEEP

SEQ ID NO: 28 - protein, 557 aa, synthetic construct
  REGION 1..557: note = Dead 28-aa extension Cas12f1 R518A
MAGGPGAGSAAPVSSTSSLPLAALNMRVMAKNTITKTLKLRIVRPYNSAEVEKIVADEKNNREKIALEKNKDKVKEACSKHLKVAAYCTTQVERNACLFCKARKLDDKFYQKLRGQFPDAVFWQEISEIFRQLQKQAAEIYNQSLIELYYEIFIKGKGIANASSVEHYLSDVCYTRAAELFKNAAIASGLRSKIKSNFRLKELKNMKSGLPTTKSDNFPIPLVKQKGGQYTGFEISNHNSDFIIKIPFGRWQVKKEIDKYRPWEKFDFEQVQKSPKPISLLLSTQRRKRNKGWSKDEGTEAEIKKVMNGDYQTSYIEVKRGSKIGEKSAWMLNLSIDVPKIDKGVDPSIIGGIDVGVKSPLVCAINNAFSRYSISDNDLFHFNKKMFARRRILLKKNRHKRAGHGAKNKLKPITILTEKSERFRKKLIERWACEIADFFIKNKVGTVQMENLESMKRKEDSYFNIRLRGFWPYAEMQNKIEFKLKQYGIEIRKVAPNNTSKTCSKCGHLNNYFNFEYAKKNKFPHFKCEKCNFKENADYNAALNISNPKLKSTKEEP

SEQ ID NO: 29 - protein, 557 aa, synthetic construct
  REGION 1..557: note = Dead 28-aa extension Cas12f1 D538A
MAGGPGAGSAAPVSSTSSLPLAALNMRVMAKNTITKTLKLRIVRPYNSAEVEKIVADEKNNREKIALEKNKDKVKEACSKHLKVAAYCTTQVERNACLFCKARKLDDKFYQKLRGQFPDAVFWQEISEIFRQLQKQAAEIYNQSLIELYYEIFIKGKGIANASSVEHYLSDVCYTRAAELFKNAAIASGLRSKIKSNFRLKELKNMKSGLPTTKSDNFPIPLVKQKGGQYTGFEISNHNSDFIIKIPFGRWQVKKEIDKYRPWEKFDFEQVQKSPKPISLLLSTQRRKRNKGWSKDEGTEAEIKKVMNGDYQTSYIEVKRGSKIGEKSAWMLNLSIDVPKIDKGVDPSIIGGIDVGVKSPLVCAINNAFSRYSISDNDLFHFNKKMFARRRILLKKNRHKRAGHGAKNKLKPITILTEKSERFRKKLIERWACEIADFFIKNKVGTVQMENLESMKRKEDSYFNIRLRGFWPYAEMQNKIEFKLKQYGIEIRKVAPNNTSKTCSKCGHLNNYFNFEYRKKNKFPHFKCEKCNFKENAAYNAALNISNPKLKSTKEEP

SEQ ID NO: 30 - protein, 555 aa, synthetic construct
  REGION 1..555: note = 26aa-extension Cas12f1 = Variant 3
MAGGPGAGSAAPVSSTSSLPLAALNMMAKNTITKTLKLRIVRPYNSAEVEKIVADEKNNREKIALEKNKDKVKEACSKHLKVAAYCTTQVERNACLFCKARKLDDKFYQKLRGQFPDAVFWQEISEIFRQLQKQAAEIYNQSLIELYYEIFIKGKGIANASSVEHYLSDVCYTRAAELFKNAAIASGLRSKIKSNFRLKELKNMKSGLPTTKSDNFPIPLVKQKGGQYTGFEISNHNSDFIIKIPFGRWQVKKEIDKYRPWEKFDFEQVQKSPKPISLLLSTQRRKRNKGWSKDEGTEAEIKKVMNGDYQTSYIEVKRGSKIGEKSAWMLNLSIDVPKIDKGVDPSIIGGIDVGVKSPLVCAINNAFSRYSISDNDLFHFNKKMFARRRILLKKNRHKRAGHGAKNKLKPITILTEKSERFRKKLIERWACEIADFFIKNKVGTVQMENLESMKRKEDSYFNIRLRGFWPYAEMQNKIEFKLKQYGIEIRKVAPNNTSKTCSKCGHLNNYFNFEYRKKNKFPHFKCEKCNFKENADYNAALNISNPKLKSTKEEP

SEQ ID NO: 31 - protein, 557 aa, synthetic construct; identical to SEQ ID NO: 26
  REGION 1..557: note = Dead 26aa-extension Cas12f1 D352A

SEQ ID NO: 32 - protein, 555 aa, synthetic construct
  REGION 1..555: note = Dead 26aa-extension Cas12f1 E448A
MAGGPGAGSAAPVSSTSSLPLAALNMMAKNTITKTLKLRIVRPYNSAEVEKIVADEKNNREKIALEKNKDKVKEACSKHLKVAAYCTTQVERNACLFCKARKLDDKFYQKLRGQFPDAVFWQEISEIFRQLQKQAAEIYNQSLIELYYEIFIKGKGIANASSVEHYLSDVCYTRAAELFKNAAIASGLRSKIKSNFRLKELKNMKSGLPTTKSDNFPIPLVKQKGGQYTGFEISNHNSDFIIKIPFGRWQVKKEIDKYRPWEKFDFEQVQKSPKPISLLLSTQRRKRNKGWSKDEGTEAEIKKVMNGDYQTSYIEVKRGSKIGEKSAWMLNLSIDVPKIDKGVDPSIIGGIDVGVKSPLVCAINNAFSRYSISDNDLFHFNKKMFARRRILLKKNRHKRAGHGAKNKLKPITILTEKSERFRKKLIERWACEIADFFIKNKVGTVQMANLESMKRKEDSYFNIRLRGFWPYAEMQNKIEFKLKQYGIEIRKVAPNNTSKTCSKCGHLNNYFNFEYRKKNKFPHFKCEKCNFKENADYNAALNISNPKLKSTKEEP

SEQ ID NO: 33 - protein, 555 aa, synthetic construct
  REGION 1..555: note = Dead 26aa-extension Cas12f1 R516A
MAGGPGAGSAAPVSSTSSLPLAALNMMAKNTITKTLKLRIVRPYNSAEVEKIVADEKNNREKIALEKNKDKVKEACSKHLKVAAYCTTQVERNACLFCKARKLDDKFYQKLRGQFPDAVFWQEISEIFRQLQKQAAEIYNQSLIELYYEIFIKGKGIANASSVEHYLSDVCYTRAAELFKNAAIASGLRSKIKSNFRLKELKNMKSGLPTTKSDNFPIPLVKQKGGQYTGFEISNHNSDFIIKIPFGRWQVKKEIDKYRPWEKFDFEQVQKSPKPISLLLSTQRRKRNKGWSKDEGTEAEIKKVMNGDYQTSYIEVKRGSKIGEKSAWMLNLSIDVPKIDKGVDPSIIGGIDVGVKSPLVCAINNAFSRYSISDNDLFHFNKKMFARRRILLKKNRHKRAGHGAKNKLKPITILTEKSERFRKKLIERWACEIADFFIKNKVGTVQMENLESMKRKEDSYFNIRLRGFWPYAEMQNKIEFKLKQYGIEIRKVAPNNTSKTCSKCGHLNNYFNFEYAKKNKFPHFKCEKCNFKENADYNAALNISNPKLKSTKEEP

SEQ ID NO: 34 - protein, 555 aa, synthetic construct
  REGION 1..555: note = Dead 26aa-extension Cas12f1 D536A
MAGGPGAGSAAPVSSTSSLPLAALNMMAKNTITKTLKLRIVRPYNSAEVEKIVADEKNNREKIALEKNKDKVKEACSKHLKVAAYCTTQVERNACLFCKARKLDDKFYQKLRGQFPDAVFWQEISEIFRQLQKQAAEIYNQSLIELYYEIFIKGKGIANASSVEHYLSDVCYTRAAELFKNAAIASGLRSKIKSNFRLKELKNMKSGLPTTKSDNFPIPLVKQKGGQYTGFEISNHNSDFIIKIPFGRWQVKKEIDKYRPWEKFDFEQVQKSPKPISLLLSTQRRKRNKGWSKDEGTEAEIKKVMNGDYQTSYIEVKRGSKIGEKSAWMLNLSIDVPKIDKGVDPSIIGGIDVGVKSPLVCAINNAFSRYSISDNDLFHFNKKMFARRRILLKKNRHKRAGHGAKNKLKPITILTEKSERFRKKLIERWACEIADFFIKNKVGTVQMENLESMKRKEDSYFNIRLRGFWPYAEMQNKIEFKLKQYGIEIRKVAPNNTSKTCSKCGHLNNYFNFEYRKKNKFPHFKCEKCNFKENAAYNAALNISNPKLKSTKEEP

SEQ ID NO: 35 - protein, 555 aa, synthetic construct
  REGION 1..555: note = CasX-Cas12f1 = Variant 4
MEKRINKIRKKLSADNATKPVSRSGPMAKNTITKTLKLRIVRPYNSAEVEKIVADEKNNREKIALEKNKDKVKEACSKHLKVAAYCTTQVERNACLFCKARKLDDKFYQKLRGQFPDAVFWQEISEIFRQLQKQAAEIYNQSLIELYYEIFIKGKGIANASSVEHYLSDVCYTRAAELFKNAAIASGLRSKIKSNFRLKELKNMKSGLPTTKSDNFPIPLVKQKGGQYTGFEISNHNSDFIIKIPFGRWQVKKEIDKYRPWEKFDFEQVQKSPKPISLLLSTQRRKRNKGWSKDEGTEAEIKKVMNGDYQTSYIEVKRGSKIGEKSAWMLNLSIDVPKIDKGVDPSIIGGIDVGVKSPLVCAINNAFSRYSISDNDLFHFNKKMFARRRILLKKNRHKRAGHGAKNKLKPITILTEKSERFRKKLIERWACEIADFFIKNKVGTVQMENLESMKRKEDSYFNIRLRGFWPYAEMQNKIEFKLKQYGIEIRKVAPNNTSKTCSKCGHLNNYFNFEYRKKNKFPHFKCEKCNFKENADYNAALNISNPKLKSTKEEP

SEQ ID NO: 36 - protein, 555 aa, synthetic construct
  REGION 1..555: note = Dead CasX-Cas12f1 D352A
MEKRINKIRKKLSADNATKPVSRSGPMAKNTITKTLKLRIVRPYNSAEVEKIVADEKNNREKIALEKNKDKVKEACSKHLKVAAYCTTQVERNACLFCKARKLDDKFYQKLRGQFPDAVFWQEISEIFRQLQKQAAEIYNQSLIELYYEIFIKGKGIANASSVEHYLSDVCYTRAAELFKNAAIASGLRSKIKSNFRLKELKNMKSGLPTTKSDNFPIPLVKQKGGQYTGFEISNHNSDFIIKIPFGRWQVKKEIDKYRPWEKFDFEQVQKSPKPISLLLSTQRRKRNKGWSKDEGTEAEIKKVMNGDYQTSYIEVKRGSKIGEKSAWMLNLSIDVPKIDKGVDPSIIGGIAVGVKSPLVCAINNAFSRYSISDNDLFHFNKKMFARRRILLKKNRHKRAGHGAKNKLKPITILTEKSERFRKKLIERWACEIADFFIKNKVGTVQMENLESMKRKEDSYFNIRLRGFWPYAEMQNKIEFKLKQYGIEIRKVAPNNTSKTCSKCGHLNNYFNFEYRKKNKFPHFKCEKCNFKENADYNAALNISNPKLKSTKEEP

SEQ ID NO: 37 - protein, 555 aa, synthetic construct
  REGION 1..555: note = Dead CasX-Cas12f1 E448A
MEKRINKIRKKLSADNATKPVSRSGPMAKNTITKTLKLRIVRPYNSAEVEKIVADEKNNREKIALEKNKDKVKEACSKHLKVAAYCTTQVERNACLFCKARKLDDKFYQKLRGQFPDAVFWQEISEIFRQLQKQAAEIYNQSLIELYYEIFIKGKGIANASSVEHYLSDVCYTRAAELFKNAAIASGLRSKIKSNFRLKELKNMKSGLPTTKSDNFPIPLVKQKGGQYTGFEISNHNSDFIIKIPFGRWQVKKEIDKYRPWEKFDFEQVQKSPKPISLLLSTQRRKRNKGWSKDEGTEAEIKKVMNGDYQTSYIEVKRGSKIGEKSAWMLNLSIDVPKIDKGVDPSIIGGIDVGVKSPLVCAINNAFSRYSISDNDLFHFNKKMFARRRILLKKNRHKRAGHGAKNKLKPITILTEKSERFRKKLIERWACEIADFFIKNKVGTVQMANLESMKRKEDSYFNIRLRGFWPYAEMQNKIEFKLKQYGIEIRKVAPNNTSKTCSKCGHLNNYFNFEYRKKNKFPHFKCEKCNFKENADYNAALNISNPKLKSTKEEP

SEQ ID NO: 38 - protein, 555 aa, synthetic construct
  REGION 1..555: note = Dead CasX-Cas12f1 R516A
MEKRINKIRKKLSADNATKPVSRSGPMAKNTITKTLKLRIVRPYNSAEVEKIVADEKNNREKIALEKNKDKVKEACSKHLKVAAYCTTQVERNACLFCKARKLDDKFYQKLRGQFPDAVFWQEISEIFRQLQKQAAEIYNQSLIELYYEIFIKGKGIANASSVEHYLSDVCYTRAAELFKNAAIASGLRSKIKSNFRLKELKNMKSGLPTTKSDNFPIPLVKQKGGQYTGFEISNHNSDFIIKIPFGRWQVKKEIDKYRPWEKFDFEQVQKSPKPISLLLSTQRRKRNKGWSKDEGTEAEIKKVMNGDYQTSYIEVKRGSKIGEKSAWMLNLSIDVPKIDKGVDPSIIGGIDVGVKSPLVCAINNAFSRYSISDNDLFHFNKKMFARRRILLKKNRHKRAGHGAKNKLKPITILTEKSERFRKKLIERWACEIADFFIKNKVGTVQMENLESMKRKEDSYFNIRLRGFWPYAEMQNKIEFKLKQYGIEIRKVAPNNTSKTCSKCGHLNNYFNFEYAKKNKFPHFKCEKCNFKENADYNAALNISNPKLKSTKEEP

SEQ ID NO: 39 - protein, 555 aa, synthetic construct
  REGION 1..555: note = Dead CasX-Cas12f1 D536A
MEKRINKIRKKLSADNATKPVSRSGPMAKNTITKTLKLRIVRPYNSAEVEKIVADEKNNREKIALEKNKDKVKEACSKHLKVAAYCTTQVERNACLFCKARKLDDKFYQKLRGQFPDAVFWQEISEIFRQLQKQAAEIYNQSLIELYYEIFIKGKGIANASSVEHYLSDVCYTRAAELFKNAAIASGLRSKIKSNFRLKELKNMKSGLPTTKSDNFPIPLVKQKGGQYTGFEISNHNSDFIIKIPFGRWQVKKEIDKYRPWEKFDFEQVQKSPKPISLLLSTQRRKRNKGWSKDEGTEAEIKKVMNGDYQTSYIEVKRGSKIGEKSAWMLNLSIDVPKIDKGVDPSIIGGIDVGVKSPLVCAINNAFSRYSISDNDLFHFNKKMFARRRILLKKNRHKRAGHGAKNKLKPITILTEKSERFRKKLIERWACEIADFFIKNKVGTVQMENLESMKRKEDSYFNIRLRGFWPYAEMQNKIEFKLKQYGIEIRKVAPNNTSKTCSKCGHLNNYFNFEYRKKNKFPHFKCEKCNFKENAAYNAALNISNPKLKSTKEEP

SEQ ID NO: 40 - protein, 557 aa, synthetic construct
  REGION 1..557: note = TnpB Mutant (ABE Window variant), I159/S164Y
MGEKSSRRRRNGKSGAWTAAITSCVGGKMAKNTITKTLKLRIVRPYNSAEVEKIVADEKNNREKIALEKNKDKVKEACSKHLKVAAYCTTQVERNACLFCKARKLDDKFYQKLRGQFPDAVFWQEISEIFRQLQKQAAEIYNQSLIELYYEIFIKGKGWANASYVEHYLSDVCYTRAAELFKNAAIASGLRSKIKSNFRLKELKNMKSGLPTTKSDNFPIPLVKQKGGQYTGFEISNHNSDFIIKIPFGRWQVKKEIDKYRPWEKFDFEQVQKSPKPISLLLSTQRRKRNKGWSKDEGTEAEIKKVMNGDYQTSYIEVKRGSKIGEKSAWMLNLSIDVPKIDKGVDPSIIGGIDVGVKSPLVCAINNAFSRYSISDNDLFHFNKKMFARRRILLKKNRHKRAGHGAKNKLKPITILTEKSERFRKKLIERWACEIADFFIKNKVGTVQMENLESMKRKEDSYFNIRLRGFWPYAEMQNKIEFKLKQYGIEIRKVAPNNTSKTCSKCGHLNNYFNFEYRKKNKFPHFKCEKCNFKENADYNAALNISNPKLKSTKEEP

SEQ ID NO: 41 - RNA, 161 nt, synthetic construct
  misc_feature 1..161: note = tracrRNA scaffold of Cas12f1, WT
  source 1..161: mol_type = other RNA
cttcactgataaagtggagaaccgcttcaccaaaagctgtcccttaggggattagaacttgagtgaaggtgggctgcttgcatcagcctaatgtcgagaagtgctttcttcggaaagtaaccctcgaaacaaattcatttttcctctccaattctgcacaa

SEQ ID NO: 42 - RNA, 140 nt, synthetic construct
  misc_feature 1..140: note = tracrRNA scaffold of Cas12f1, MF
  source 1..140: mol_type = other RNA
cttcactgataaagtggagaaccgcttcaccaaaagctgtcccttaggggattagaacttgagtgaaggtgggctgcttgcatcagcctaatgtcgagaagtgctttcttcggaaagtaaccctcgaaacaaattcattt

SEQ ID NO: 43 - RNA, 37 nt, synthetic construct
  misc_feature 1..37: note = crRNA scaffold of Cas12f1, WT
  source 1..37: mol_type = other RNA
gttgcagaacccgaatagacgaatgaaggaatgcaac

SEQ ID NO: 44 - RNA, 17 nt, synthetic construct
  misc_feature 1..17: note = crRNA scaffold of Cas12f1, MF
  source 1..17: mol_type = other RNA
gaatgaaggaatgcaac

SEQ ID NO: 45 - RNA, 32 nt, synthetic construct
  misc_feature 1..32: note = 1st Fragment of engineered tracrRNA scaffold
  misc_feature 9..11: note = n is a, c, g, or u
  misc_feature 13: note = n is a, c, g, or u
  source 1..32: mol_type = other RNA
caaattcannncncctctccaattctgcacaa

SEQ ID NO: 46 - RNA, 31 nt, synthetic construct
  misc_feature 1..31: note = 1st Fragment of engineered tracrRNA scaffold
  misc_feature 9..11: note = n is a, c, g, or u
  misc_feature 13: note = n is a, c, g, or u
  source 1..31: mol_type = other RNA
caaattcannncncctctccaattctgcaca

SEQ ID NO: 47 - RNA, 30 nt, synthetic construct
  misc_feature 1..30: note = 1st Fragment of engineered tracrRNA scaffold
  misc_feature 9..11: note = n is a, c, g, or u
  misc_feature 13: note = n is a, c, g, or u
  source 1..30: mol_type = other RNA
caaattcannncncctctccaattctgcac

SEQ ID NO: 48 - RNA, 29 nt, synthetic construct
  misc_feature 1..29: note = 1st Fragment of engineered tracrRNA scaffold
  misc_feature 9..11: note = n is a, c, g, or u
  misc_feature 13: note = n is a, c, g, or u
  source 1..29: mol_type = other RNA
caaattcannncncctctccaattctgca

SEQ ID NO: 49 - RNA, 28 nt, synthetic construct
  misc_feature 1..28: note = 1st Fragment of engineered tracrRNA scaffold
  misc_feature 9..11: note = n is a, c, g, or u
  misc_feature 13: note = n is a, c, g, or u
  source 1..28: mol_type = other RNA
caaattcannncncctctccaattctgc

SEQ ID NO: 50 - RNA, 27 nt, synthetic construct
  misc_feature 1..27: note = 1st Fragment of engineered tracrRNA scaffold
  misc_feature 9..11: note = n is a, c, g, or u
  misc_feature 13: note = n is a, c, g, or u
  source 1..27: mol_type = other RNA
caaattcannncncctctccaattctg

SEQ ID NO: 51 - RNA, 26 nt, synthetic construct
  misc_feature 1..26: note = 1st Fragment of engineered tracrRNA scaffold
  misc_feature 9..11: note = n is a, c, g, or u
  misc_feature 13: note = n is a, c, g, or u
  source 1..26: mol_type = other RNA
caaattcannncncctctccaattct

SEQ ID NO: 52 - RNA, 25 nt, synthetic construct
  misc_feature 1..25: note = 1st Fragment of engineered tracrRNA scaffold
  misc_feature 9..11: note = n is a, c, g, or u
  misc_feature 13: note = n is a, c, g, or u
  source 1..25: mol_type = other RNA
caaattcannncncctctccaattc

SEQ ID NO: 53 - RNA, 24 nt, synthetic construct
  misc_feature 1..24: note = 1st Fragment of engineered tracrRNA scaffold
  misc_feature 9..11: note = n is a, c, g, or u
  misc_feature 13: note = n is a, c, g, or u
  source 1..24: mol_type = other RNA
caaattcannncncctctccaatt

SEQ ID NO: 54 - RNA, 23 nt, synthetic construct
  misc_feature 1..23: note = 1st Fragment of engineered tracrRNA scaffold
  misc_feature 9..11: note = n is a, c, g, or u
  misc_feature 13: note = n is a, c, g, or u
  source 1..23: mol_type = other RNA
caaattcannncncctctccaat

SEQ ID NO: 55 - RNA, 22 nt, synthetic construct
  misc_feature 1..22: note = 1st Fragment of engineered tracrRNA scaffold
  misc_feature 9..11: note = n is a, c, g, or u
  misc_feature 13: note = n is a, c, g, or u
  source 1..22: mol_type = other RNA
caaattcannncncctctccaa

SEQ ID NO: 56 - RNA, 21 nt, synthetic construct
  misc_feature 1..21: note = 1st Fragment of engineered tracrRNA scaffold
  misc_feature 9..11: note = n is a, c, g, or u
  misc_feature 13: note = n is a, c, g, or u
  source 1..21: mol_type = other RNA
caaattcannncncctctcca

SEQ ID NO: 57 - RNA, 20 nt, synthetic construct
  misc_feature 1..20: note = 1st Fragment of engineered tracrRNA scaffold
  misc_feature 9..11: note = n is a, c, g, or u
  misc_feature 13: note = n is a, c, g, or u
  source 1..20: mol_type = other RNA
caaattcannncncctctcc

SEQ ID NO: 58 - RNA, 19 nt, synthetic construct
  misc_feature 1..19: note = 1st Fragment of engineered tracrRNA scaffold
  misc_feature 9..11: note = n is a, c, g, or u
  misc_feature 13: note = n is a, c, g, or u
  source 1..19: mol_type = other RNA
caaattcannncncctctc

SEQ ID NO: 59 - RNA, 18 nt, synthetic construct
  misc_feature 1..18: note = 1st Fragment of engineered tracrRNA scaffold
  misc_feature 9..11: note = n is a, c, g, or u
  misc_feature 13: note = n is a, c, g, or u
  source 1..18: mol_type = other RNA
caaattcannncncctct

SEQ ID NO: 60 - RNA, 17 nt, synthetic construct
  misc_feature 1..17: note = 1st Fragment of engineered tracrRNA scaffold
  misc_feature 9..11: note = n is a, c, g, or u
  misc_feature 13: note = n is a, c, g, or u
  source 1..17: mol_type = other RNA
caaattcannncncctc

SEQ ID NO: 61 - RNA, 16 nt, synthetic construct
  misc_feature 1..16: note = 1st Fragment of engineered tracrRNA scaffold
  misc_feature 9..11: note = n is a, c, g, or u
  misc_feature 13: note = n is a, c, g, or u
  source 1..16: mol_type = other RNA
caaattcannncncct

SEQ ID NO: 62 - RNA, 15 nt, synthetic construct
  misc_feature 1..15: note = 1st Fragment of engineered tracrRNA scaffold
  misc_feature 9..11: note = n is a, c, g, or u
  misc_feature 13: note = n is a, c, g, or u
  source 1..15: mol_type = other RNA
caaattcannncncc

SEQ ID NO: 63 - RNA, 14 nt, synthetic construct
  misc_feature 1..14: note = 1st Fragment of engineered tracrRNA scaffold
  misc_feature 9..11: note = n is a, c, g, or u
  misc_feature 13: note = n is a, c, g, or u
  source 1..14: mol_type = other RNA
caaattcannncnc

SEQ ID NO: 64 - skipped

SEQ ID NO: 65 - RNA, 39 nt, synthetic construct
  misc_feature 1..39: note = 2nd Fragment of engineered tracrRNA scaffold
  source 1..39: mol_type = other RNA
atgtcgagaagtgctttcttcggaaagtaaccctcgaaa

SEQ ID NO: 66 - RNA, 19 nt, synthetic construct
  misc_feature 1..19: note = 3rd Fragment of engineered tracrRNA scaffold
  source 1..19: mol_type = other RNA
ggctgcttgcatcagccta

SEQ ID NO: 67 - RNA, 50 nt, synthetic construct
  misc_feature 1..50: note = 4th Fragment of engineered tracrRNA scaffold
  source 1..50: mol_type = other RNA
ccgcttcaccaaaagctgtcccttaggggattagaacttgagtgaaggtg

SEQ ID NO: 68 - RNA, 48 nt, synthetic construct
  misc_feature 1..48: note = 4th Fragment of engineered tracrRNA scaffold
  source 1..48: mol_type = other RNA
ccgcttcaccaaaagctgtccttagggattagaacttgagtgaaggtg

SEQ ID NO: 69 - RNA, 46 nt, synthetic construct
  misc_feature 1..46: note = 4th Fragment of engineered tracrRNA scaffold
  source 1..46: mol_type = other RNA
ccgcttcaccaaaagctgtcttaggattagaacttgagtgaaggtg

SEQ ID NO: 70 - RNA, 44 nt, synthetic construct
  misc_feature 1..44: note = 4th Fragment of engineered tracrRNA scaffold
  source 1..44: mol_type = other RNA
ccgcttcaccaaaagctgtttagattagaacttgagtgaaggtg

SEQ ID NO: 71 - RNA, 42 nt, synthetic construct
  misc_feature 1..42: note = 4th Fragment of engineered tracrRNA scaffold
  source 1..42: mol_type = other RNA
ccgcttcaccaaaagctgttagttagaacttgagtgaaggtg

SEQ ID NO: 72 - RNA, 41 nt, synthetic construct
  misc_feature 1..41: note = 4th Fragment of engineered tracrRNA scaffold
  source 1..41: mol_type = other RNA
ccgcttcaccaaaagctgttagtagaacttgagtgaaggtg

SEQ ID NO: 73 - RNA, 39 nt, synthetic construct
  misc_feature 1..39: note = 4th Fragment of engineered tracrRNA scaffold
  source 1..39: mol_type = other RNA
ccgcttcaccaaaagctttagagaacttgagtgaaggtg

SEQ ID NO: 74 - RNA, 37 nt, synthetic construct
  misc_feature 1..37: note = 4th Fragment of engineered tracrRNA scaffold
  source 1..37: mol_type = other RNA
ccgcttcaccaaaagcttaggaacttgagtgaaggtg

SEQ ID NO: 75 - RNA, 35 nt, synthetic construct
  misc_feature 1..35: note = 4th Fragment of engineered tracrRNA scaffold
  source 1..35: mol_type = other RNA
ccgcttcaccaaaagttagaacttgagtgaaggtg

SEQ ID NO: 76 - RNA, 33 nt, synthetic construct
  misc_feature 1..33: note = 4th Fragment of engineered tracrRNA scaffold
  source 1..33: mol_type = other RNA
ccgcttcaccaaaattagacttgagtgaaggtg

SEQ ID NO: 77 - RNA, 31 nt, synthetic construct
  misc_feature 1..31: note = 4th Fragment of engineered tracrRNA scaffold
  source 1..31: mol_type = other RNA
ccgcttcaccaaattagcttgagtgaaggtg

SEQ ID NO: 78 - RNA, 29 nt, synthetic construct
  misc_feature 1..29: note = 4th Fragment of engineered tracrRNA scaffold
  source 1..29: mol_type = other RNA
ccgcttcaccaattagttgagtgaaggtg

SEQ ID NO: 79 - RNA, 27 nt, synthetic construct
  misc_feature 1..27: note = 4th Fragment of engineered tracrRNA scaffold
  source 1..27: mol_type = other RNA
ccgcttcaccattagtgagtgaaggtg

SEQ ID NO: 80 - RNA, 25 nt, synthetic construct
  misc_feature 1..25: note = 4th Fragment of engineered tracrRNA scaffold
  source 1..25: mol_type = other RNA
ccgcttcaccttaggagtgaaggtg

SEQ ID NO: 81 - RNA, 23 nt, synthetic construct
  misc_feature 1..23: note = 4th Fragment of engineered tracrRNA scaffold
  source 1..23: mol_type = other RNA
ccgcttcacttagagtgaaggtg

SEQ ID NO: 82 - RNA, 22 nt, synthetic construct
  misc_feature 1..22: note = 4th Fragment of engineered tracrRNA scaffold
  source 1..22: mol_type = other RNA
ccgcttcacttaggtgaaggtg

SEQ ID NO: 83 - RNA, 20 nt, synthetic construct
  misc_feature 1..20: note = 4th Fragment of engineered tracrRNA scaffold
  source 1..20: mol_type = other RNA
ccgcttcattagtgaaggtg

SEQ ID NO: 84 - RNA, 18 nt, synthetic construct
  misc_feature 1..18: note = 4th Fragment of engineered tracrRNA scaffold
  source 1..18: mol_type = other RNA
ccgcttcttaggaaggtg

SEQ ID NO: 85 - RNA, 16 nt, synthetic construct
  misc_feature 1..16: note = 4th Fragment of engineered tracrRNA scaffold
  source 1..16: mol_type = other RNA
ccgcttttagaaggtg

SEQ ID NO: 86 - RNA, 14 nt, synthetic construct
  misc_feature 1..14: note = 4th Fragment of engineered tracrRNA scaffold
  source 1..14: mol_type = other RNA
ccgctttagaggtg

SEQ ID NO: 87 - RNA, 12 nt, synthetic construct
  misc_feature 1..12: note = 4th Fragment of engineered tracrRNA scaffold
  source 1..12: mol_type = other RNA
ccgcttagggtg

SEQ ID NO: 88 - RNA, 10 nt, synthetic construct
  misc_feature 1..10: note = 4th Fragment of engineered tracrRNA scaffold
  source 1..10: mol_type = other RNA
ccgttaggtg

SEQ ID NO: 89 - RNA, 21 nt, synthetic construct
  misc_feature 1..21: note = 5th Fragment of engineered tracrRNA scaffold
  source 1..21: mol_type = other RNA
cttcactgataaagtggagaa

SEQ ID NO: 90 - RNA, 10 nt, synthetic construct
  misc_feature 1..10: note = 5th Fragment of engineered tracrRNA scaffold
  source 1..10: mol_type = other RNA
aagtggagaa

SEQ ID NO: 91 - RNA, 11 nt, synthetic construct
  misc_feature 1..11: note = 5th Fragment of engineered tracrRNA scaffold
  source 1..11: mol_type = other RNA
aaagtggagaa

SEQ ID NO: 92 - RNA, 12 nt, synthetic construct
  misc_feature 1..12: note = 5th Fragment of engineered tracrRNA scaffold
  source 1..12: mol_type = other RNA
taaagtggagaa

SEQ ID NO: 93 - RNA, 13 nt, synthetic construct
  misc_feature 1..13: note = 5th Fragment of engineered tracrRNA scaffold
  source 1..13: mol_type = other RNA
ataaagtggagaa

SEQ ID NO: 94 - RNA, 14 nt, synthetic construct
  misc_feature 1..14: note = 5th Fragment of engineered tracrRNA scaffold
  source 1..14: mol_type = other RNA
gataaagtggagaa

SEQ ID NO: 95 - RNA, 15 nt, synthetic construct
  misc_feature 1..15: note = 5th Fragment of engineered tracrRNA scaffold
  source 1..15: mol_type = other RNA
tgataaagtggagaa

SEQ ID NO: 96 - RNA, 16 nt, synthetic construct
  misc_feature 1..16: note = 5th Fragment of engineered tracrRNA scaffold
  source 1..16: mol_type = other RNA
ctgataaagtggagaa

SEQ ID NO: 97 - RNA, 17 nt, synthetic construct
  misc_feature 1..17: note = 5th Fragment of engineered tracrRNA scaffold
  source 1..17: mol_type = other RNA
actgataaagtggagaa

SEQ ID NO: 98 - RNA, 18 nt, synthetic construct
  misc_feature 1..18: note = 5th Fragment of engineered tracrRNA scaffold
  source 1..18: mol_type = other RNA
cactgataaagtggagaa

SEQ ID NO: 99 - RNA, 19 nt, synthetic construct
  misc_feature 1..19: note = 5th Fragment of engineered tracrRNA scaffold
  source 1..19: mol_type = other RNA
tcactgataaagtggagaa

SEQ ID NO: 100 - RNA, 20 nt, synthetic construct
  misc_feature 1..20: note = 5th Fragment of engineered tracrRNA scaffold
  source 1..20: mol_type = other RNA
ttcactgataaagtggagaa

SEQ ID NO: 101 - RNA, 10 nt, synthetic construct
  misc_feature 1..10: note = 1st region of engineered tracrRNA scaffold, MF
  source 1..10: mol_type = other RNA
aagtggagaa

SEQ ID NO: 102 - RNA, 11 nt, synthetic construct
  misc_feature 1..11: note = 1st region of engineered tracrRNA scaffold, MF
  source 1..11: mol_type = other RNA
aaagtggagaa

SEQ ID NO: 103 - RNA, 12 nt, synthetic construct
  misc_feature 1..12: note = 1st region of engineered tracrRNA scaffold, MF
  source 1..12: mol_type = other RNA
taaagtggagaa

SEQ ID NO: 104 - RNA, 13 nt, synthetic construct
  misc_feature 1..13: note = 1st region of engineered tracrRNA scaffold, MF
  source 1..13: mol_type = other RNA
ataaagtggagaa

SEQ ID NO: 105 - RNA, 14 nt, synthetic construct
  misc_feature 1..14: note = 1st region of engineered tracrRNA scaffold, MF
  source 1..14: mol_type = other RNA
gataaagtggagaa

SEQ ID NO: 106 - RNA, 15 nt, synthetic construct
  misc_feature 1..15: note = 1st region of engineered tracrRNA scaffold, MF
  source 1..15: mol_type = other RNA
tgataaagtggagaa

SEQ ID NO: 107 - RNA, 16 nt, synthetic construct
  misc_feature 1..16: note = 1st region of engineered tracrRNA scaffold, MF
  source 1..16: mol_type = other RNA
ctgataaagtggagaa

SEQ ID NO: 108 - RNA, 17 nt, synthetic construct
  misc_feature 1..17: note = 1st region of engineered tracrRNA scaffold, MF
  source 1..17: mol_type = other RNA
actgataaagtggagaa

SEQ ID NO: 109 - RNA, 18 nt, synthetic construct
  misc_feature 1..18: note = 1st region of engineered tracrRNA scaffold, MF
  source 1..18: mol_type = other RNA
cactgataaagtggagaa

SEQ ID NO: 110 - RNA, 19 nt, synthetic construct
  misc_feature 1..19: note = 1st region of engineered tracrRNA scaffold, MF
  source 1..19: mol_type = other RNA
tcactgataaagtggagaa

SEQ ID NO: 111 - RNA, 20 nt, synthetic construct
  misc_feature 1..20: note = 1st region of engineered tracrRNA scaffold, MF
  source 1..20: mol_type = other RNA
ttcactgataaagtggagaa

SEQ ID NO: 112 - RNA, 21 nt, synthetic construct
  misc_feature 1..21: note = 1st region of engineered tracrRNA scaffold, MF
  source 1..21: mol_type = other RNA
cttcactgataaagtggagaa

SEQ ID NO: 113 - RNA, 10 nt, synthetic construct
  misc_feature 1..10: note = 2nd region of engineered tracrRNA scaffold, MF
  source 1..10: mol_type = other RNA
ccttaggtgg

SEQ ID NO: 114 - RNA, 11 nt, synthetic construct
  misc_feature 1..11: note = 2nd region of engineered tracrRNA scaffold, MF
  source 1..11: mol_type = other RNA
ccgttaggtgg

SEQ ID NO: 115 - RNA, 13 nt, synthetic construct
  misc_feature 1..13: note = 2nd region of engineered tracrRNA scaffold, MF
  source 1..13: mol_type = other RNA
ccgcttagggtgg

SEQ ID NO: 116 - RNA, 15 nt, synthetic construct
  misc_feature 1..15: note = 2nd region of engineered tracrRNA scaffold, MF
  source 1..15: mol_type = other RNA
ccgctttagaggtgg

SEQ ID NO: 117 - RNA, 17 nt, synthetic construct
  misc_feature 1..17: note = 2nd region of engineered tracrRNA scaffold, MF
  source 1..17: mol_type = other RNA
ccgcttttagaaggtgg

SEQ ID NO: 118 - RNA, 19 nt, synthetic construct
  misc_feature 1..19: note = 2nd region of engineered tracrRNA scaffold, MF
  source 1..19: mol_type = other RNA
ccgcttcttaggaaggtgg

SEQ ID NO: 119 - RNA, 21 nt, synthetic construct
  misc_feature 1..21: note = 2nd region of engineered tracrRNA scaffold, MF
  source 1..21: mol_type = other RNA
ccgcttcattagtgaaggtgg

SEQ ID NO: 120 - RNA, 23 nt, synthetic construct
  misc_feature 1..23: note = 2nd region of engineered tracrRNA scaffold, MF
  source 1..23: mol_type = other RNA
ccgcttcacttaggtgaaggtgg

SEQ ID NO: 121 - RNA, 24 nt, synthetic construct
  misc_feature 1..24: note = 2nd region of engineered tracrRNA scaffold, MF
  source 1..24: mol_type = other RNA
ccgcttcacttagagtgaaggtgg

SEQ ID NO: 122 - RNA, 26 nt, synthetic construct
  misc_feature 1..26: note = 2nd region of engineered tracrRNA scaffold, MF
  source 1..26: mol_type = other RNA
ccgcttcaccttaggagtgaaggtgg

SEQ ID NO: 123 - RNA, 28 nt, synthetic construct
  misc_feature 1..28: note = 2nd region of engineered tracrRNA scaffold, MF
  source 1..28: mol_type = other RNA
ccgcttcaccattagtgagtgaaggtgg

SEQ ID NO: 124 - RNA, 30 nt, synthetic construct
  misc_feature 1..30: note = 2nd region of engineered tracrRNA scaffold, MF
  source 1..30: mol_type = other RNA
ccgcttcaccaattagttgagtgaaggtgg

SEQ ID NO: 125 - RNA, 32 nt, synthetic construct
  misc_feature 1..32: note = 2nd region of engineered tracrRNA scaffold, MF
  source 1..32: mol_type = other RNA
ccgcttcaccaaattagcttgagtgaaggtgg

SEQ ID NO: 126 - RNA, 34 nt, synthetic construct
  misc_feature 1..34: note = 2nd region of engineered tracrRNA scaffold, MF
  source 1..34: mol_type = other RNA
ccgcttcaccaaaattagacttgagtgaaggtgg

SEQ ID NO: 127 - RNA, 36 nt, synthetic construct
  misc_feature 1..36: note = 2nd region of engineered tracrRNA scaffold, MF
  source 1..36: mol_type = other RNA
ccgcttcaccaaaagttagaacttgagtgaaggtgg

SEQ ID NO: 128 - RNA, 38 nt, synthetic construct
  misc_feature 1..38: note = 2nd region of engineered tracrRNA scaffold, MF
  source 1..38: mol_type = other RNA
ccgcttcaccaaaagcttaggaacttgagtgaaggtgg

SEQ ID NO: 129 - RNA, 40 nt, synthetic construct
  misc_feature 1..40: note = 2nd region of engineered tracrRNA scaffold, MF
  source 1..40: mol_type = other RNA
ccgcttcaccaaaagctttagagaacttgagtgaaggtgg

SEQ ID NO: 130 - RNA, 42 nt, synthetic construct
  misc_feature 1..42: note = 2nd region of engineered tracrRNA scaffold, MF
  source 1..42: mol_type = other RNA
ccgcttcaccaaaagctgttagtagaacttgagtgaaggtgg

SEQ ID NO: 131 - RNA, 43 nt, synthetic construct
  misc_feature 1..43: note = 2nd region of engineered tracrRNA scaffold, MF
  source 1..43: mol_type = other RNA
ccgcttcaccaaaagctgttagttagaacttgagtgaaggtgg

SEQ ID NO: 132 - RNA, 45 nt, synthetic construct
  misc_feature 1..45: note = 2nd region of engineered tracrRNA scaffold, MF
  source 1..45: mol_type = other RNA
ccgcttcaccaaaagctgtttagattagaacttgagtgaaggtgg

SEQ ID NO: 133 - RNA, 47 nt, synthetic construct
  misc_feature 1..47: note = 2nd region of engineered tracrRNA scaffold, MF
  source 1..47: mol_type = other RNA
ccgcttcaccaaaagctgtcttaggattagaacttgagtgaaggtgg

SEQ ID NO: 134 - RNA, 51 nt, synthetic construct
  misc_feature 1..51: note = 2nd region of engineered tracrRNA scaffold, MF
  source 1..51: mol_type = other RNA
ccgcttcaccaaaagctgtcccttaggggattagaacttgagtgaaggtgg

SEQ ID NO: 135 - RNA, 55 nt, synthetic construct
  misc_feature 1..55: note = 3rd region of engineered tracrRNA scaffold, MF
  source 1..55: mol_type = other RNA
gctgcttgcatcagcctaatgtcgagaagtgctttcttcggaaagtaaccctcga

SEQ ID NO: 136 - RNA, 53 nt, synthetic construct
  misc_feature 1..53: note = 3rd region of engineered tracrRNA scaffold, MF
  source 1..53: mol_type = other RNA
gctgcttgcatcagcctaatgtcgagaagtgctttttcgaaagtaaccctcga

SEQ ID NO: 137 - RNA, 51 nt, synthetic construct
  misc_feature 1..51: note = 3rd region of engineered tracrRNA scaffold, MF
  source 1..51: mol_type = other RNA
gctgcttgcatcagcctaatgtcgagaagtgcttttcgaagtaaccctcga

SEQ ID NO: 138 - RNA, 51 nt, synthetic construct
  misc_feature 1..51: note = 3rd region of engineered tracrRNA scaffold, MF
  source 1..51: mol_type = other RNA
gctgcttgcatcagcctaatgtcgagaagtgctcttcggagtaaccctcga

SEQ ID NO: 139 - RNA, 49 nt, synthetic construct
  misc_feature 1..49: note = 3rd region of engineered tracrRNA scaffold, MF
  source 1..49: mol_type = other RNA
gctgcttgcatcagcctaatgtcgagaagtgctttcgagtaaccctcga

SEQ ID NO: 140 - RNA, 47 nt, synthetic construct
  misc_feature 1..47: note = 3rd region of engineered tracrRNA scaffold, MF
  source 1..47: mol_type = other RNA
gctgcttgcatcagcctaatgtcgagaagtgcttcggtaaccctcga

SEQ ID NO: 141 - RNA, 45 nt, synthetic construct
  misc_feature 1..45: note = 3rd region of engineered tracrRNA scaffold, MF
  source 1..45: mol_type = other RNA
gctgcttgcatcagcctaatgtcgagaagtgttcgtaaccctcga

SEQ ID NO: 142 - RNA, 43 nt, synthetic construct
  misc_feature 1..43: note = 3rd region of engineered tracrRNA scaffold, MF
  source 1..43: mol_type = other RNA
gctgcttgcatcagcctaatgtcgagaagtttcgaaccctcga

SEQ ID NO: 143 - RNA, 41 nt, synthetic construct
  misc_feature 1..41: note = 3rd region of engineered tracrRNA scaffold, MF
  source 1..41: mol_type = other RNA
gctgcttgcatcagcctaatgtcgagaagttcgaccctcga

SEQ ID NO: 144 - RNA, 40 nt, synthetic construct
  misc_feature 1..40: note = 3rd region of engineered tracrRNA scaffold, MF
  source 1..40: mol_type = other RNA
gctgcttgcatcagcctaatgtcgagaagttcgccctcga

SEQ ID NO: 145 - RNA, 39 nt, synthetic construct
  misc_feature 1..39: note = 3rd region of engineered tracrRNA scaffold, MF
  source 1..39: mol_type = other RNA
gctgcttgcatcagcctaatgtcgagaattcgccctcga

SEQ ID NO: 146 - RNA, 38 nt, synthetic construct
  misc_feature 1..38: note = 3rd region of engineered tracrRNA scaffold, MF
  source 1..38: mol_type = other RNA
gctgcttgcatcagcctaatgtcgagaattcgcctcga

SEQ ID NO: 147 - RNA, 37 nt, synthetic construct
  misc_feature 1..37: note = 3rd region of engineered tracrRNA scaffold, MF
  source 1..37: mol_type = other RNA
gctgcttgcatcagcctaatgtcgagattcgcctcga

SEQ ID NO: 148 - RNA, 35 nt, synthetic construct
  misc_feature 1..35: note = 3rd region of engineered tracrRNA scaffold, MF
  source 1..35: mol_type = other RNA
gctgcttgcatcagcctaatgtcgagttcgctcga

SEQ ID NO: 149 - RNA, 55 nt, synthetic construct; identical to SEQ ID NO: 135
  misc_feature 1..55: note = 3rd region of engineered tracrRNA scaffold, MF
  source 1..55: mol_type = other RNA

SEQ ID NO: 150-153 - skipped (4 entries)

SEQ ID NO: 154 - RNA, 10 nt, synthetic construct
  misc_feature 1..10: note = 4th region of engineered tracrRNA scaffold, MF
  source 1..10: mol_type = other RNA
aacaaattca

SEQ ID NO: 155 - RNA, 11 nt, synthetic construct
  misc_feature 1..11: note = 4th region of engineered tracrRNA scaffold, MF
  source 1..11: mol_type = other RNA
aacaaattcat

SEQ ID NO: 156 - RNA, 12 nt, synthetic construct
  misc_feature 1..12: note = 4th region of engineered tracrRNA scaffold, MF
  source 1..12: mol_type = other RNA
aacaaattcatt

SEQ ID NO: 157 - RNA, 13 nt, synthetic construct
  misc_feature 1..13: note = 4th region of engineered tracrRNA scaffold, MF
  source 1..13: mol_type = other RNA
aacaaattcattt

SEQ ID NO: 158 - RNA, 30 nt, synthetic construct
  misc_feature 1..30: note = 6th fragment of engineered crRNA scaffold, WT
  misc_feature 19: note = n is a, c, g, or u
  misc_feature 21..23: note = n is a, c, g, or u
  source 1..30: mol_type = other RNA
gttgcagaacccgaatagnbnnntgaagga

SEQ ID NO: 159 - RNA, 30 nt, synthetic construct
  misc_feature 1..30: note = 6th fragment of engineered crRNA scaffold, WT
  misc_feature 19: note = n is a, c, g, or u
  misc_feature 21..23: note = n is a, c, g, or u
  source 1..30: mol_type = other RNA
gttgcagaacccgaatagngnnntgaagga

SEQ ID NO: 160 - RNA, 29 nt, synthetic construct
  misc_feature 1..29: note = 6th fragment of engineered crRNA scaffold, WT
  misc_feature 18: note = n is a, c, g, or u
  misc_feature 20..22: note = n is a, c, g, or u
  source 1..29: mol_type = other RNA
ttgcagaacccgaatagngnnntgaagga

SEQ ID NO: 161 - RNA, 28 nt, synthetic construct
  misc_feature 1..28: note = 6th fragment of engineered crRNA scaffold, WT
  misc_feature 17: note = n is a, c, g, or u
  misc_feature 19..21: note = n is a, c, g, or u
  source 1..28: mol_type = other RNA
tgcagaacccgaatagngnnntgaagga

SEQ ID NO: 162 - RNA, 27 nt, synthetic construct
  misc_feature 1..27: note = 6th fragment of engineered crRNA scaffold, WT
  misc_feature 16: note = n is a, c, g, or u
  misc_feature 18..20: note = n is a, c, g, or u
  source 1..27: mol_type = other RNA
gcagaacccgaatagngnnntgaagga

SEQ ID NO: 163 - RNA, 26 nt, synthetic construct
  misc_feature 1..26: note = 6th fragment of engineered crRNA scaffold, WT
  misc_feature 15: note = n is a, c, g, or u
  misc_feature 17..19: note = n is a, c, g, or u
  source 1..26: mol_type = other RNA
cagaacccgaatagngnnntgaagga

SEQ ID NO: 164 - RNA, 25 nt, synthetic construct
  misc_feature 1..25: note = 6th fragment of engineered crRNA scaffold, WT
  misc_feature 14: note = n is a, c, g, or u
  misc_feature 16..18: note = n is a, c, g, or u
  source 1..25: mol_type = other RNA
agaacccgaatagngnnntgaagga

SEQ ID NO: 165 - RNA, 24 nt, synthetic construct
  misc_feature 1..24: note = 6th fragment of engineered crRNA scaffold, WT
  misc_feature 13: note = n is a, c, g, or u
  misc_feature 15..17: note = n is a, c, g, or u
  source 1..24: mol_type = other RNA
gaacccgaatagngnnntgaagga

SEQ ID NO: 166 - RNA, 23 nt, synthetic construct
  misc_feature 1..23: note = 6th fragment of engineered crRNA scaffold, WT
  misc_feature 12: note = n is a, c, g, or u
  misc_feature 14..16: note = n is a, c, g, or u
  source 1..23: mol_type = other RNA
aacccgaatagngnnntgaagga

SEQ ID NO: 167 - RNA, 22 nt, synthetic construct
  misc_feature 1..22: note = 6th fragment of engineered crRNA scaffold, WT
  misc_feature 11: note = n is a, c, g, or u
  misc_feature 13..15: note = n is a, c, g, or u
  source 1..22: mol_type = other RNA
acccgaatagngnnntgaagga

SEQ ID NO: 168 - RNA, 21 nt, synthetic construct
  misc_feature 1..21: note = 6th fragment of engineered crRNA scaffold, WT
  misc_feature 10: note = n is a, c, g, or u
  misc_feature 12..14: note = n is a, c, g, or u
  source 1..21: mol_type = other RNA
cccgaatagngnnntgaagga

SEQ ID NO: 169 - RNA, 20 nt, synthetic construct
  misc_feature 1..20: note = 6th fragment of engineered crRNA scaffold, WT
  misc_feature 9: note = n is a, c, g, or u
  misc_feature 11..13: note = n is a, c, g, or u
  source 1..20: mol_type = other RNA
ccgaatagngnnntgaagga

SEQ ID NO: 170 - RNA, 19 nt, synthetic construct
  misc_feature 1..19: note = 6th fragment of engineered crRNA scaffold, WT
  misc_feature 8: note = n is a, c, g, or u
  misc_feature 10..12: note = n is a, c, g, or u
  source 1..19: mol_type = other RNA
cgaatagngnnntgaagga

SEQ ID NO: 171 - RNA, 18 nt, synthetic construct
  misc_feature 1..18: note = 6th fragment of engineered crRNA scaffold, WT
  misc_feature 7: note = n is a, c, g, or u
  misc_feature 9..11: note = n is a, c, g, or u
  source 1..18: mol_type = other RNA
gaatagngnnntgaagga

SEQ ID NO: 172 - RNA, 17 nt, synthetic construct
  misc_feature 1..17: note = 6th fragment of engineered crRNA scaffold, WT
  misc_feature 6: note = n is a, c, g, or u
  misc_feature 8..10: note = n is a, c, g, or u
  source 1..17: mol_type = other RNA
aatagngnnntgaagga

SEQ ID NO: 173 - RNA, 16 nt, synthetic construct
  misc_feature 1..16: note = 6th fragment of engineered crRNA scaffold, WT
  misc_feature 5: note = n is a, c, g, or u
  misc_feature 7..9: note = n is a, c, g, or u
  source 1..16: mol_type = other RNA
atagngnnntgaagga

SEQ ID NO: 174 - RNA, 15 nt, synthetic construct
  misc_feature 1..15: note = 6th fragment of engineered crRNA scaffold, WT
  misc_feature 4: note = n is a, c, g, or u
  misc_feature 6..8: note = n is a, c, g, or u
  source 1..15: mol_type = other RNA
tagngnnntgaagga

SEQ ID NO: 175 - RNA, 14 nt, synthetic construct
  misc_feature 1..14: note = 6th fragment of engineered crRNA scaffold, WT
  misc_feature 3: note = n is a, c, g, or u
  misc_feature 5..7: note = n is a, c, g, or u
  source 1..14: mol_type = other RNA
agngnnntgaagga

SEQ ID NO: 176 - skipped

SEQ ID NO: 177 - RNA, 10 nt, synthetic construct
  misc_feature 1..10: note = 5th region of engineered crRNA scaffold, MF
  source 1..10: mol_type = other RNA
gaatgaagga

SEQ ID NO: 178 - RNA, 11 nt, synthetic construct
  misc_feature 1..11: note = 5th region of engineered crRNA scaffold, MF
  source 1..11: mol_type = other RNA
cgaatgaagga

SEQ ID NO: 179 - RNA, 12 nt, synthetic construct
  misc_feature 1..12: note = 5th region of engineered crRNA scaffold, MF
  source 1..12: mol_type = other RNA
acgaatgaagga

SEQ ID NO: 180 - RNA, 13 nt, synthetic construct
  misc_feature 1..13: note = 5th region of engineered crRNA scaffold, MF
  source 1..13: mol_type = other RNA
gacgaatgaagga

SEQ ID NO: 181 - RNA, 14 nt, synthetic construct
  misc_feature 1..14: note = 5th region of engineered crRNA scaffold, MF
  source 1..14: mol_type = other RNA
agacgaatgaagga

SEQ ID NO: 182 - RNA, 15 nt, synthetic construct
  misc_feature 1..15: note = 5th region of engineered crRNA scaffold, MF
  source 1..15: mol_type = other RNA
tagacgaatgaagga

SEQ ID NO: 183 - RNA, 16 nt, synthetic construct
  misc_feature 1..16: note = 5th region of engineered crRNA scaffold, MF
  source 1..16: mol_type = other RNA
atagacgaatgaagga

SEQ ID NO: 184 - RNA, 17 nt, synthetic construct
  misc_feature 1..17: note = 5th region of engineered crRNA scaffold, MF
  source 1..17: mol_type = other RNA
aatagacgaatgaagga

SEQ ID NO: 185 - RNA, 18 nt, synthetic construct
  misc_feature 1..18: note = 5th region of engineered crRNA scaffold, MF
  source 1..18: mol_type = other RNA
gaatagacgaatgaagga

SEQ ID NO: 186 - RNA, 19 nt, synthetic construct
  misc_feature 1..19: note = 5th region of engineered crRNA scaffold, MF
  source 1..19: mol_type = other RNA
cgaatagacgaatgaagga

SEQ ID NO: 187 - RNA, 20 nt, synthetic construct
  misc_feature 1..20: note = 5th region of engineered crRNA scaffold, MF
  source 1..20: mol_type = other RNA
ccgaatagacgaatgaagga

SEQ ID NO: 188 - RNA, 21 nt, synthetic construct
  misc_feature 1..21: note = 5th region of engineered crRNA scaffold, MF
  source 1..21: mol_type = other RNA
cccgaatagacgaatgaagga

SEQ ID NO: 189 - RNA, 22 nt, synthetic construct
  misc_feature 1..22: note = 5th region of engineered crRNA scaffold, MF
  source 1..22: mol_type = other RNA
acccgaatagacgaatgaagga

SEQ ID NO: 190 - RNA, 23 nt, synthetic construct
  misc_feature 1..23: note = 5th region of engineered crRNA scaffold, MF
  source 1..23: mol_type = other RNA
aacccgaatagacgaatgaagga

SEQ ID NO: 191 - RNA, 24 nt, synthetic construct
  misc_feature 1..24: note = 5th region of engineered crRNA scaffold, MF
  source 1..24: mol_type = other RNA
gaacccgaatagacgaatgaagga

SEQ ID NO: 192 - RNA, 25 nt, synthetic construct
  misc_feature 1..25: note = 5th region of engineered crRNA scaffold, MF
  source 1..25: mol_type = other RNA
agaacccgaatagacgaatgaagga

SEQ ID NO: 193 - RNA, 26 nt, synthetic construct
  misc_feature 1..26: note = 5th region of engineered crRNA scaffold, MF
  source 1..26: mol_type = other RNA
cagaacccgaatagacgaatgaagga

SEQ ID NO: 194 - RNA, 27 nt, synthetic construct
  misc_feature 1..27: note = 5th region of engineered crRNA scaffold, MF
  source 1..27: mol_type = other RNA
gcagaacccgaatagacgaatgaagga

SEQ ID NO: 195 - RNA, 28 nt, synthetic construct
  misc_feature 1..28: note = 5th region of engineered crRNA scaffold, MF
  source 1..28: mol_type = other RNA
tgcagaacccgaatagacgaatgaagga

SEQ ID NO: 196 - RNA, 29 nt, synthetic construct
  misc_feature 1..29: note = 5th region of engineered crRNA scaffold, MF
  source 1..29: mol_type = other RNA
ttgcagaacccgaatagacgaatgaagga

SEQ ID NO: 197 - RNA, 182 nt, synthetic construct
  misc_feature 1..182: note = SgRNA scaffold of ge3.0
  source 1..182: mol_type = other RNA
accgcttcaccaaaagctgtcccttaggggattagaacttgagtgaaggtgggctgcttgcatcagcctaatgtcgagaagtgctttcttcggaaagtaaccctcgaaacaaattcagtgctcctctccaattctgcacaagaaagttgcagaacccgaatagagcaatgaaggaatgcaac

SEQ ID NO: 198 - RNA, 127 nt, synthetic construct
  misc_feature 1..127: note = SgRNA scaffold of ge4.0
  source 1..127: mol_type = other RNA
accgcttcaccaaaagctgtcccttaggggattagaacttgagtgaaggtgggctgcttgcatcagcctaatgtcgagaagtgctttcttcggaaagtaaccctcgaaacaaagaaaggaatgcaac

SEQ ID NO: 199 - RNA, 100 nt, synthetic construct
  misc_feature 1..100: note = SgRNA scaffold of ge4.1
  source 1..100: mol_type = other RNA
accgcttcacttagagtgaaggtgggctgcttgcatcagcctaatgtcgagaagtgctttcttcggaaagtaaccctcgaaacaaagaaaggaatgcaac

SEQ ID NO: 200 - protein, 7 aa, simian virus 40
PKKKRKV

SEQ ID NO: 201 - protein, 16 aa, mus musculus
KRPAATKKAGQAKKKK

SEQ ID NO: 202 - protein, 9 aa, homo sapiens
PAAKRVKLD

SEQ ID NO: 203 - protein, 11 aa, Homo sapiens
RQRRNELKRSP

SEQ ID NO: 204 - protein, 38 aa, mus musculus
NQSSNFGPMKGGNFGGRSSGPYGGGGQYFAKPRNQGGY

SEQ ID NO: 205 - protein, 42 aa, Homo sapiens
RMRIZFKNKGKDTAELRRRRVEVSVELRKAKKDEQILKRRNV

SEQ ID NO: 206 - protein, 8 aa, Homo sapiens
VSRKRPRP

SEQ ID NO: 207 - protein, 8 aa, Homo sapiens
PPKKARED

SEQ ID NO: 208 - protein, 8 aa, Homo sapiens
PQPKKKPL

SEQ ID NO: 209 - protein, 12 aa, mus musculus
SALIKKKKKMAP

SEQ ID NO: 210 - protein, 5 aa, Influenza virus
DRLRR

SEQ ID NO: 211 - protein, 7 aa, Influenza virus
PKQKKRK

SEQ ID NO: 212 - protein, 10 aa, Hepatitis D virus
RKLKKKIKKL

SEQ ID NO: 213 - protein, 10 aa, mus musculus
REKKKFLKRR

SEQ ID NO: 214 - protein, 20 aa, homo sapiens
KRKGDEVDGVDEVAKKKSKK

SEQ ID NO: 215 - protein, 17 aa, homo sapiens
RKCLQAGMNLEARKTKK

SEQ ID NO: 216 - skipped

SEQ ID NO: 217 - RNA, 11 nt, synthetic construct
  misc_feature 1..11: note = U-rich tail sequence
  source 1..11: mol_type = other RNA
tttrtttrttt

SEQ ID NO: 218-221 - skipped (4 entries)

SEQ ID NO: 222 - RNA, 10 nt, synthetic construct
  misc_feature 1..10: note = U-rich tail sequence
  source 1..10: mol_type = other RNA
ttttrttttt

SEQ ID NO: 223 - RNA, 11 nt, synthetic construct
  misc_feature 1..11: note = U-rich tail sequence
  source 1..11: mol_type = other RNA
ttttrtttttt

SEQ ID NO: 224 - skipped

SEQ ID NO: 225 - RNA, 11 nt, synthetic construct
  misc_feature 1..11: note = U-rich tail sequence
  source 1..11: mol_type = other RNA
tttatttattt

SEQ ID NO: 226-229 - skipped (4 entries)

SEQ ID NO: 230 - RNA, 10 nt, synthetic construct
  misc_feature 1..10: note = U-rich tail sequence
  source 1..10: mol_type = other RNA
ttttattttt

SEQ ID NO: 231 - RNA, 11 nt, synthetic construct
  misc_feature 1..11: note = U-rich tail sequence
  source 1..11: mol_type = other RNA
ttttatttttt

SEQ ID NO: 232 - skipped

SEQ ID NO: 233 - RNA, 11 nt, synthetic construct
  misc_feature 1..11: note = U-rich tail sequence
  source 1..11: mol_type = other RNA
tttgtttgttt

SEQ ID NO: 234-237 - skipped (4 entries)

SEQ ID NO: 238 - RNA, 10 nt, synthetic construct
  misc_feature 1..10: note = U-rich tail sequence
  source 1..10: mol_type = other RNA
ttttgttttt

SEQ ID NO: 239 - RNA, 11 nt, synthetic construct
  misc_feature 1..11: note = U-rich tail sequence
  source 1..11: mol_type = other RNA
ttttgtttttt

SEQ ID NO: 240 - skipped

SEQ ID NO: 241 - protein, 167 aa, synthetic construct
  REGION 1..167: note = TadA
MSEVEFSHEYWMRHALTLAKRAWDEREVPVGAVLVHNNRVIGEGWNRPIGRHDPTAHAEIMALRQGGLVMQNYRLIDATLYVTLEPCVMCAGAMIHSRIGRVVFGARDAKTGAAGSLMDVLHHPGMNHRVEITEGILADECAALLSDFFRMRRQEIKAQKKAQSSTD

SEQ ID NO: 242 - protein, 167 aa, synthetic construct
  REGION 1..167: note = eTadA1(Tad*)
MSEVEFSHEYWMRHALTLAKRARDEREVPVGAVLVLNNRVIGEGWNRAIGLHDPTAHAEIMALRQGGLVMQNYRLIDATLYVTFEPCVMCAGAMIHSRIGRVVFGVRNAKTGAAGSLMDVLHYPGMNHRVEITEGILADECAALLCYFFRMPRQVFNAQKKAQSSTD

SEQ ID NO: 243 - protein, 167 aa, synthetic construct
  REGION 1..167: note = dTadA(E59A)
MSEVEFSHEYWMRHALTLAKRAWDEREVPVGAVLVHNNRVIGEGWNRPIGRHDPTAHAAIMALRQGGLVMQNYRLIDATLYVTLEPCVMCAGAMIHSRIGRVVFGARDAKTGAAGSLMDVLHHPGMNHRVEITEGILADECAALLSDFFRMRRQEIKAQKKAQSSTD

SEQ ID NO: 244 - protein, 167 aa, synthetic construct
  REGION 1..167: note = deTadA1(E59A)
MSEVEFSHEYWMRHALTLAKRARDEREVPVGAVLVLNNRVIGEGWNRAIGLHDPTAHAAIMALRQGGLVMQNYRLIDATLYVTFEPCVMCAGAMIHSRIGRVVFGVRNAKTGAAGSLMDVLHYPGMNHRVEITEGILADECAALLCYFFRMPRQVFNAQKKAQSSTD

SEQ ID NO: 245 - protein, 167 aa, synthetic construct
  REGION 1..167: note = eTadA2
MSEVEFSHEYWMRHALTLAKRARDEREVPVGAVLVLNNRVIGEGWNRAIGLHDPTAHAEIMALRQGGLVMQNYRLIDATLYVTFEPCVMCAGAMIHSRIGRVVFGWRNSKRGAAGSLMNVLNYPGMNHRVEITEGILADECAALLCDFYRMPRQVFNAQKKAQSSIN

SEQ ID NO: 246 - protein, 167 aa, synthetic construct
  REGION 1..167: note = eTadA3
MSEVEFSHEYWMRHALTLAKRARDEREVPVGAVLVLNNRVIGEGWNRAIGLHDPTAHAEIMALRQGGLVMQNYRLIDATLYVTFEPCVMCAGAMIHSRIGRVVFGWRQSKRGAAGSLMNVLNYPGMNHRVEITEGILADECAALLCDFYRMPRQVFNAQKKAQSSIN

SEQ ID NO: 247 - protein, 159 aa, synthetic construct
  REGION 1..159: note = eTadA4
MVEFSDEYWMRHALTLAKRARDEGEVPVGAVLVLNNRVIGEGWNRAIGLHDPTAHAEIMALRQGGQVLQNYRLIDATLYVTFEPCVMCAGAMIHSRIKRVVFGWRNSKRGAAGSLMNVLNHPGMNHRVEITEGVLADECAALLSDFFRMRRQQKKAQKK

SEQ ID NO: 248 - protein, 159 aa, synthetic construct
  REGION 1..159: note = eTadA5
MVEFSDEYWMRHALTLAKRARDEGEVPVGAVLVLNNQVIGEGWNRSISLHDPTAHAEIMALRQGGQVLQNYRLIDCTLYVTFEPCVMCAGAMIHSRIKRVVFGWRNPKRGAAGSLMNVLNHPGMNHRIEITEGVLADECAAMLSDFFRMRRQQKKAQKK

SEQ ID NO: 249 - protein, 159 aa, synthetic construct
  REGION 1..159: note = eTadA6
MVEFSDEYWMRHALTLAKRARDEGEVPVGAVLVLNNQVIGEGWNRSITHHDPTAHAEIMALRQGGQVLQNYRLIDCTLYVTFEPCVMCAGAMIHARIKRVVFGWRNPKRGAAGSVMNVLNHPGMNHRIEITEGVLADECAAMLSDFFRMRRQQKKAQKK

SEQ ID NO: 250 - protein, 167 aa, synthetic construct
  REGION 1..167: note = eTadA7
MSEVEFSHEYWMRHALTLAKRARDEREVPVGAVLVLNNRVIGEGWNRAIGLHDPTAHAEIMALRQGGLVMQNYRLIDATLYVTFEPCVMCAGAMIHSRIGRVVFGVRNSKRGAAGSLMNVLNYPGMNHRVEITEGILADECAALLCDFYRMPRQVFNAQKKAQSSIN

SEQ ID NO: 251 - protein, 167 aa, synthetic construct
  REGION 1..167: note = eTadA8(V106W)
MSEVEFSHEYWMRHALTLAKRARDEREVPVGAVLVLNNRVIGEGWNRAIGLHDPTAHAEIMALRQGGLVMQNYRLIDATLYVTFEPCVMCAGAMIHSRIGRVVFGWRNAKTGAAGSLMDVLHYPGMNHRVEITEGILADECAALLCYFFRMPRQVFNAQKKAQSSTD

SEQ ID NO: 252 - protein, 167 aa, synthetic construct
  REGION 1..167: note = eTadA9(V106W/D108Q)
MSEVEFSHEYWMRHALTLAKRARDEREVPVGAVLVLNNRVIGEGWNRAIGLHDPTAHAEIMALRQGGLVMQNYRLIDATLYVTFEPCVMCAGAMIHSRIGRVVFGWRQAKTGAAGSLMDVLHYPGMNHRVEITEGILADECAALLCYFFRMPRQVFNAQKKAQSSTD

SEQ ID NO: 253 - protein, 167 aa, synthetic construct
  REGION 1..167: note = eTadA10
MSEVEFSHEYWMRHALTLAKRARDEREVPVGAVLVLNNRVIGEGWNRAIGLHDPTAHAEIMALRQGGLVMQNYRLYDATLYSTFEPCVMCAGAMIHSRIGRVVFGVRNAKTGAAGSLMDVLHHPGMNHRVEITEGILADECAALLCRFFRMPRRVFNAQKKAQSSTD

SEQ ID NO: 254 - protein, 167 aa, synthetic construct
  REGION 1..167: note = eTadA11(D108Q)
MSEVEFSHEYWMRHALTLAKRARDEREVPVGAVLVLNNRVIGEGWNRAIGLHDPTAHAEIMALRQGGLVMQNYRLIDATLYVTFEPCVMCAGAMIHSRIGRVVFGVRQAKTGAAGSLMDVLHYPGMNHRVEITEGILADECAALLCYFFRMPRQVFNAQKKAQSSTD

SEQ ID NO: 255 - protein, 167 aa, synthetic construct; identical to SEQ ID NO: 241
  REGION 1..167: note = Tad

SEQ ID NO: 256 - protein, 167 aa, synthetic construct; identical to SEQ ID NO: 242
  REGION 1..167: note = eTad

SEQ ID NO: 257 - protein, 229 aa, synthetic construct [sequence omitted]

SEQ ID NO: 258 - protein, 199 aa, synthetic construct
  REGION 1..199: note = APOBEC3A
MEASPASGPRHLMDPHIFTSNFNNGIGRHKTYLCYEVERLDNGTSVKMDQHRGFLHNQAKNLLCGFYGRHAELRFLDLVPSLQLDPAQIYRVTWFISWSPCFSWGCAGEVRAFLQENTHVRLRIFAARIYDYDPLYKEALQMLRDAGAQVSIMTYDEFKHCWDTFVDHQGCPFQPWDGLDEHSQALSGRLRAILQNQGN

SEQ ID NO: 259 - protein, 382 aa, synthetic construct [sequence omitted]

SEQ ID NO: 260 - protein, 10 aa, synthetic construct
  REGION 1..10: note = Linker used to link between Tad and dTnpB, 10aa
SGGSSGGSSG

SEQ ID NO: 261 - protein, 14 aa, synthetic construct
  REGION 1..14: note = Linker used to link between Tad and dTnpB, 14aa
SGGSSGGSSGSETP

SEQ ID NO: 262 - protein, 16 aa, synthetic construct
  REGION 1..16: note = Linker used to link between Tad and dTnpB, 16aa
SGGSSGGSSGSETPGT

SEQ ID NO: 263 - protein, 20 aa, synthetic construct
  REGION 1..20: note = Linker used to link between Tad and dTnpB, 20aa
SGGSSGGSSGSETPGTSESA

SEQ ID NO: 264 - protein, 24 aa, synthetic construct
  REGION 1..24: note = Linker used to link between Tad and dTnpB, 24aa
SGGSSGGSSGSETPGTSESATPES

SEQ ID NO: 265 - protein, 28 aa, synthetic construct
  REGION 1..28: note = Linker used to link between Tad and dTnpB, 28aa
SGGSSGGSSGSETPGTSESATPESSGGS

SEQ ID NO: 266 - protein, 32 aa, synthetic construct
  REGION 1..32: note = Linker used to link between Tad and dTnpB, 32aa
SGGSSGGSSGSETPGTSESATPESSGGSSGGS

SEQ ID NO: 267 - protein, 36 aa, synthetic construct
  REGION 1..36: note = Linker used to link between Tad and dTnpB, 36aa
SGGSSGGSSGSETPGTSESATPESSGGSSGGSSGSE

SEQ ID NO: 268 - protein, 40 aa, synthetic construct
  REGION 1..40: note = Linker used to link between Tad and dTnpB, 40aa
SGGSSGGSSGSETPGTSESATPESSGGSSGGSSGSETPGT

SEQ ID NO: 269 - protein, 5 aa, synthetic construct
  REGION 1..5: note = Linker
GGGGS

SEQ ID NO: 270 - protein, 5 aa, synthetic construct
  REGION 1..5: note = Linker
EAAAK

SEQ ID NO: 271 - protein, 16 aa, synthetic construct
  REGION 1..16: note = Linker
SGSETPGTSESATPES

SEQ ID NO: 272 - protein, 4 aa, synthetic construct
  REGION 1..4: note = Linker
SGGS

SEQ ID NO: 273 - protein, 14 aa, synthetic construct
  REGION 1..14: note = Linker
SGGSKRTADGSEFE

SEQ ID NO: 274 - protein, 366 aa, synthetic construct
  REGION 1..366: note = TadA-32aaLinker-eTadA1
MSEVEFSHEYWMRHALTLAKRAWDEREVPVGAVLVHNNRVIGEGWNRPIGRHDPTAHAEIMALRQGGLVMQNYRLIDATLYVTLEPCVMCAGAMIHSRIGRVVFGARDAKTGAAGSLMDVLHHPGMNHRVEITEGILADECAALLSDFFRMRRQEIKAQKKAQSSTDSGGSSGGSSGSETPGTSESATPESSGGSSGGSMSEVEFSHEYWMRHALTLAKRARDEREVPVGAVLVLNNRVIGEGWNRAIGLHDPTAHAEIMALRQGGLVMQNYRLIDATLYVTFEPCVMCAGAMIHSRIGRVVFGVRNAKTGAAGSLMDVLHYPGMNHRVEITEGILADECAALLCYFFRMPRQVFNAQKKAQSSTD

SEQ ID NO: 275 - protein, 366 aa, synthetic construct
  REGION 1..366: note = eTadA1-32aaLinker-TadA
MSEVEFSHEYWMRHALTLAKRARDEREVPVGAVLVLNNRVIGEGWNRAIGLHDPTAHAEIMALRQGGLVMQNYRLIDATLYVTFEPCVMCAGAMIHSRIGRVVFGVRNAKTGAAGSLMDVLHYPGMNHRVEITEGILADECAALLCYFFRMPRQVFNAQKKAQSSTDSGGSSGGSSGSETPGTSESATPESSGGSSGGSMSEVEFSHEYWMRHALTLAKRAWDEREVPVGAVLVHNNRVIGEGWNRPIGRHDPTAHAEIMALRQGGLVMQNYRLIDATLYVTLEPCVMCAGAMIHSRIGRVVFGARDAKTGAAGSLMDVLHHPGMNHRVEITEGILADECAALLSDFFRMRRQEIKAQKKAQSSTD

SEQ ID NO: 276 - protein, 366 aa, synthetic construct
  REGION 1..366: note = TadA-32aaLinker-eTadA3
MSEVEFSHEYWMRHALTLAKRAWDEREVPVGAVLVHNNRVIGEGWNRPIGRHDPTAHAEIMALRQGGLVMQNYRLIDATLYVTLEPCVMCAGAMIHSRIGRVVFGARDAKTGAAGSLMDVLHHPGMNHRVEITEGILADECAALLSDFFRMRRQEIKAQKKAQSSTDSGGSSGGSSGSETPGTSESATPESSGGSSGGSMSEVEFSHEYWMRHALTLAKRARDEREVPVGAVLVLNNRVIGEGWNRAIGLHDPTAHAEIMALRQGGLVMQNYRLIDATLYVTFEPCVMCAGAMIHSRIGRVVFGWRQSKRGAAGSLMNVLNYPGMNHRVEITEGILADECAALLCDFYRMPRQVFNAQKKAQSSIN

SEQ ID NO: 277 - protein, 366 aa, synthetic construct
  REGION 1..366: note = TadA-32aaLinker-eTadA2
MSEVEFSHEYWMRHALTLAKRAWDEREVPVGAVLVHNNRVIGEGWNRPIGRHDPTAHAEIMALRQGGLVMQNYRLIDATLYVTLEPCVMCAGAMIHSRIGRVVFGARDAKTGAAGSLMDVLHHPGMNHRVEITEGILADECAALLSDFFRMRRQEIKAQKKAQSSTDSGGSSGGSSGSETPGTSESATPESSGGSSGGSMSEVEFSHEYWMRHALTLAKRARDEREVPVGAVLVLNNRVIGEGWNRAIGLHDPTAHAEIMALRQGGLVMQNYRLIDATLYVTFEPCVMCAGAMIHSRIGRVVFGWRNSKRGAAGSLMNVLNYPGMNHRVEITEGILADECAALLCDFYRMPRQVFNAQKKAQSSIN

SEQ ID NO: 278 - protein, 366 aa, synthetic construct
  REGION 1..366: note = dTadA-32aaLinker-eTadA1
MSEVEFSHEYWMRHALTLAKRAWDEREVPVGAVLVHNNRVIGEGWNRPIGRHDPTAHAAIMALRQGGLVMQNYRLIDATLYVTLEPCVMCAGAMIHSRIGRVVFGARDAKTGAAGSLMDVLHHPGMNHRVEITEGILADECAALLSDFFRMRRQEIKAQKKAQSSTDSGGSSGGSSGSETPGTSESATPESSGGSSGGSMSEVEFSHEYWMRHALTLAKRARDEREVPVGAVLVLNNRVIGEGWNRAIGLHDPTAHAEIMALRQGGLVMQNYRLIDATLYVTFEPCVMCAGAMIHSRIGRVVFGVRNAKTGAAGSLMDVLHYPGMNHRVEITEGILADECAALLCYFFRMPRQVFNAQKKAQSSTD

SEQ ID NO: 279 - protein, 366 aa, synthetic construct
  REGION 1..366: note = TadA-32aaLinker-deTadA1
MSEVEFSHEYWMRHALTLAKRAWDEREVPVGAVLVHNNRVIGEGWNRPIGRHDPTAHAEIMALRQGGLVMQNYRLIDATLYVTLEPCVMCAGAMIHSRIGRVVFGARDAKTGAAGSLMDVLHHPGMNHRVEITEGILADECAALLSDFFRMRRQEIKAQKKAQSSTDSGGSSGGSSGSETPGTSESATPESSGGSSGGSMSEVEFSHEYWMRHALTLAKRARDEREVPVGAVLVLNNRVIGEGWNRAIGLHDPTAHAAIMALRQGGLVMQNYRLIDATLYVTFEPCVMCAGAMIHSRIGRVVFGVRNAKTGAAGSLMDVLHYPGMNHRVEITEGILADECAALLCYFFRMPRQVFNAQKKAQSSTD

SEQ ID NO: 280 - protein, 428 aa, synthetic construct
  REGION 1..428: note = Ntype, APOBEC1-32aaLinker-TadA
MSSETGPVAVDPTLRRRIEPHEFEVFFDPRELRKETCLLYEINWGGRHSIWRHTSQNTNKHVEVNFIEKFTTERYFCPNTRCSITWFLSWSPCGECSRAITEFLSRYPHVTLFIYIARLYHHADPRNRQGLRDLISSGVTIQIMTEQESGYCWRNFVNYSPSNEAHWPRYPHLWVRLYVLELYCIILGLPPCLNILRRKQPQLTFFTIALQSCHYQRLPPHILWATGLKSGGSSGGSSGSETPGTSESATPESSGGSSGGSMSEVEFSHEYWMRHALTLAKRAWDEREVPVGAVLVHNNRVIGEGWNRPIGRHDPTAHAEIMALRQGGLVMQNYRLIDATLYVTLEPCVMCAGAMIHSRIGRVVFGARDAKTGAAGSLMDVLHHPGMNHRVEITEGILADECAALLSDFFRMRRQEIKAQKKAQSSTD

SEQ ID NO: 281 - protein, 460 aa, synthetic construct
  REGION 1..460: note = Ntype, APOBEC1-32aaLinker-eTadA
MSSETGPVAVDPTLRRRIEPHEFEVFFDPRELRKETCLLYEINWGGRHSIWRHTSQNTNKHVEVNFIEKFTTERYFCPNTRCSITWFLSWSPCGECSRAITEFLSRYPHVTLFIYIARLYHHADPRNRQGLRDLISSGVTIQIMTEQESGYCWRNFVNYSPSNEAHWPRYPHLWVRLYVLELYCIILGLPPCLNILRRKQPQLTFFTIALQSCHYQRLPPHILWATGLKSGGSSGGSSGSETPGTSESATPESSGGSSGGSMSEVEFSHEYWMRHALTLAKRARDEREVPVGAVLVLNNRVIGEGWNRAIGLHDPTAHAEIMALRQGGLVMQNYRLIDATLYVTFEPCVMCAGAMIHSRIGRVVFGVRNAKTGAAGSLMDVLHYPGMNHRVEITEGILADECAALLCYFFRMPRQVFNAQKKAQSSTDSGGSSGGSSGSETPGTSESATPESSGGSSGGS

SEQ ID NO: 282 - protein, 428 aa, synthetic construct
  REGION 1..428: note = Ctype, TadA-32aaLinker-APOBEC1
MSEVEFSHEYWMRHALTLAKRAWDEREVPVGAVLVHNNRVIGEGWNRPIGRHDPTAHAEIMALRQGGLVMQNYRLIDATLYVTLEPCVMCAGAMIHSRIGRVVFGARDAKTGAAGSLMDVLHHPGMNHRVEITEGILADECAALLSDFFRMRRQEIKAQKKAQSSTDSGGSSGGSSGSETPGTSESATPESSGGSSGGSMSSETGPVAVDPTLRRRIEPHEFEVFFDPRELRKETCLLYEINWGGRHSIWRHTSQNTNKHVEVNFIEKFTTERYFCPNTRCSITWFLSWSPCGECSRAITEFLSRYPHVTLFIYIARLYHHADPRNRQGLRDLISSGVTIQIMTEQESGYCWRNFVNYSPSNEAHWPRYPHLWVRLYVLELYCIILGLPPCLNILRRKQPQLTFFTIALQSCHYQRLPPHILWATGLK

SEQ ID NO: 283 - protein, 428 aa, synthetic construct
  REGION 1..428: note = Ctype, eTadA-32aaLinker-APOBEC1
MSEVEFSHEYWMRHALTLAKRARDEREVPVGAVLVLNNRVIGEGWNRAIGLHDPTAHAEIMALRQGGLVMQNYRLIDATLYVTFEPCVMCAGAMIHSRIGRVVFGVRNAKTGAAGSLMDVLHYPGMNHRVEITEGILADECAALLCYFFRMPRQVFNAQKKAQSSTDSGGSSGGSSGSETPGTSESATPESSGGSSGGSMSSETGPVAVDPTLRRRIEPHEFEVFFDPRELRKETCLLYEINWGGRHSIWRHTSQNTNKHVEVNFIEKFTTERYFCPNTRCSITWFLSWSPCGECSRAITEFLSRYPHVTLFIYIARLYHHADPRNRQGLRDLISSGVTIQIMTEQESGYCWRNFVNYSPSNEAHWPRYPHLWVRLYVLELYCIILGLPPCLNILRRKQPQLTFFTIALQSCHYQRLPPHILWATGLK

SEQ ID NO: 284 - protein, 943 aa, synthetic construct
  REGION 1..943: note = dCas12f1(D326A)-ABE-N1
MSEVEFSHEYWMRHALTLAKRAWDEREVPVGAVLVHNNRVIGEGWNRPIGRHDPTAHAEIMALRQGGLVMQNYRLIDATLYVTLEPCVMCAGAMIHSRIGRVVFGARDAKTGAAGSLMDVLHHPGMNHRVEITEGILADECAALLSDFFRMRRQEIKAQKKAQSSTDSGGSSGGSSGSETPGTSESATPESSGGSSGGSMSEVEFSHEYWMRHALTLAKRARDEREVPVGAVLVLNNRVIGEGWNRAIGLHDPTAHAEIMALRQGGLVMQNYRLIDATLYVTFEPCVMCAGAMIHSRIGRVVFGVRNAKTGAAGSLMDVLHYPGMNHRVEITEGILADECAALLCYFFRMPRQVFNAQKKAQSSTDSGGSSGGSSGSETPGTSESATPESSGGSSGGSMAKNTITKTLKLRIVRPYNSAEVEKIVADEKNNREKIALEKNKDKVKEACSKHLKVAAYCTTQVERNACLFCKARKLDDKFYQKLRGQFPDAVFWQEISEIFRQLQKQAAEIYNQSLIELYYEIFIKGKGIANASSVEHYLSDVCYTRAAELFKNAAIASGLRSKIKSNFRLKELKNMKSGLPTTKSDNFPIPLVKQKGGQYTGFEISNHNSDFIIKIPFGRWQVKKEIDKYRPWEKFDFEQVQKSPKPISLLLSTQRRKRNKGWSKDEGTEAEIKKVMNGDYQTSYIEVKRGSKIGEKSAWMLNLSIDVPKIDKGVDPSIIGGIAVGVKSPLVCAINNAFSRYSISDNDLFHFNKKMFARRRILLKKNRHKRAGHGAKNKLKPITILTEKSERFRKKLIERWACEIADFFIKNKVGTVQMENLESMKRKEDSYFNIRLRGFWPYAEMQNKIEFKLKQYGIEIRKVAPNNTSKTCSKCGHLNNYFNFEYRKKNKFPHFKCEKCNFKENADYNAALNISNPKLKSTKEEPKRPAATKKAGQAKKKK

SEQ ID NO: 285 - protein, 943 aa, synthetic construct
  REGION 1..943: note = dCas12f1(D326A)-ABE-N2
MSEVEFSHEYWMRHALTLAKRARDEREVPVGAVLVLNNRVIGEGWNRAIGLHDPTAHAEIMALRQGGLVMQNYRLIDATLYVTFEPCVMCAGAMIHSRIGRVVFGVRNAKTGAAGSLMDVLHYPGMNHRVEITEGILADECAALLCYFFRMPRQVFNAQKKAQSSTDSGGSSGGSSGSETPGTSESATPESSGGSSGGSMSEVEFSHEYWMRHALTLAKRAWDEREVPVGAVLVHNNRVIGEGWNRPIGRHDPTAHAEIMALRQGGLVMQNYRLIDATLYVTLEPCVMCAGAMIHSRIGRVVFGARDAKTGAAGSLMDVLHHPGMNHRVEITEGILADECAALLSDFFRMRRQEIKAQKKAQSSTDSGGSSGGSSGSETPGTSESATPESSGGSSGGSMAKNTITKTLKLRIVRPYNSAEVEKIVADEKNNREKIALEKNKDKVKEACSKHLKVAAYCTTQVERNACLFCKARKLDDKFYQKLRGQFPDAVFWQEISEIFRQLQKQAAEIYNQSLIELYYEIFIKGKGIANASSVEHYLSDVCYTRAAELFKNAAIASGLRSKIKSNFRLKELKNMKSGLPTTKSDNFPIPLVKQKGGQYTGFEISNHNSDFIIKIPFGRWQVKKEIDKYRPWEKFDFEQVQKSPKPISLLLSTQRRKRNKGWSKDEGTEAEIKKVMNGDYQTSYIEVKRGSKIGEKSAWMLNLSIDVPKIDKGVDPSIIGGIAVGVKSPLVCAINNAFSRYSISDNDLFHFNKKMFARRRILLKKNRHKRAGHGAKNKLKPITILTEKSERFRKKLIERWACEIADFFIKNKVGTVQMENLESMKRKEDSYFNIRLRGFWPYAEMQNKIEFKLKQYGIEIRKVAPNNTSKTCSKCGHLNNYFNFEYRKKNKFPHFKCEKCNFKENADYNAALNISNPKLKSTKEEPKRPAATKKAGQAKKKK

SEQ ID NO: 286 - protein, 943 aa, synthetic construct
  REGION 1..943: note = dCas12f1(D326A)-ABE-C1
MAKNTITKTLKLRIVRPYNSAEVEKIVADEKNNREKIALEKNKDKVKEACSKHLKVAAYCTTQVERNACLFCKARKLDDKFYQKLRGQFPDAVFWQEISEIFRQLQKQAAEIYNQSLIELYYEIFIKGKGIANASSVEHYLSDVCYTRAAELFKNAAIASGLRSKIKSNFRLKELKNMKSGLPTTKSDNFPIPLVKQKGGQYTGFEISNHNSDFIIKIPFGRWQVKKEIDKYRPWEKFDFEQVQKSPKPISLLLSTQRRKRNKGWSKDEGTEAEIKKVMNGDYQTSYIEVKRGSKIGEKSAWMLNLSIDVPKIDKGVDPSIIGGIAVGVKSPLVCAINNAFSRYSISDNDLFHFNKKMFARRRILLKKNRHKRAGHGAKNKLKPITILTEKSERFRKKLIERWACEIADFFIKNKVGTVQMENLESMKRKEDSYFNIRLRGFWPYAEMQNKIEFKLKQYGIEIRKVAPNNTSKTCSKCGHLNNYFNFEYRKKNKFPHFKCEKCNFKENADYNAALNISNPKLKSTKEEPSGGSSGGSSGSETPGTSESATPESSGGSSGGSMSEVEFSHEYWMRHALTLAKRARDEREVPVGAVLVLNNRVIGEGWNRAIGLHDPTAHAEIMALRQGGLVMQNYRLIDATLYVTFEPCVMCAGAMIHSRIGRVVFGVRNAKTGAAGSLMDVLHYPGMNHRVEITEGILADECAALLCYFFRMPRQVFNAQKKAQSSTDSGGSSGGSSGSETPGTSESATPESSGGSSGGSMSEVEFSHEYWMRHALTLAKRAWDEREVPVGAVLVHNNRVIGEGWNRPIGRHDPTAHAEIMALRQGGLVMQNYRLIDATLYVTLEPCVMCAGAMIHSRIGRVVFGARDAKTGAAGSLMDVLHHPGMNHRVEITEGILADECAALLSDFFRMRRQEIKAQKKAQSSTDKRPAATKKAGQAKKKK

SEQ ID NO: 287 - protein, 943 aa, synthetic construct
  REGION 1..943: note = dCas12f1(D326A)-ABE-C2
MAKNTITKTLKLRIVRPYNSAEVEKIVADEKNNREKIALEKNKDKVKEACSKHLKVAAYCTTQVERNACLFCKARKLDDKFYQKLRGQFPDAVFWQEISEIFRQLQKQAAEIYNQSLIELYYEIFIKGKGIANASSVEHYLSDVCYTRAAELFKNAAIASGLRSKIKSNFRLKELKNMKSGLPTTKSDNFPIPLVKQKGGQYTGFEISNHNSDFIIKIPFGRWQVKKEIDKYRPWEKFDFEQVQKSPKPISLLLSTQRRKRNKGWSKDEGTEAEIKKVMNGDYQTSYIEVKRGSKIGEKSAWMLNLSIDVPKIDKGVDPSIIGGIAVGVKSPLVCAINNAFSRYSISDNDLFHFNKKMFARRRILLKKNRHKRAGHGAKNKLKPITILTEKSERFRKKLIERWACEIADFFIKNKVGTVQMENLESMKRKEDSYFNIRLRGFWPYAEMQNKIEFKLKQYGIEIRKVAPNNTSKTCSKCGHLNNYFNFEYRKKNKFPHFKCEKCNFKENADYNAALNISNPKLKSTKEEPSGGSSGGSSGSETPGTSESATPESSGGSSGGSMSEVEFSHEYWMRHALTLAKRAWDEREVPVGAVLVHNNRVIGEGWNRPIGRHDPTAHAEIMALRQGGLVMQNYRLIDATLYVTLEPCVMCAGAMIHSRIGRVVFGARDAKTGAAGSLMDVLHHPGMNHRVEITEGILADECAALLSDFFRMRRQEIKAQKKAQSSTDSGGSSGGSSGSETPGTSESATPESSGGSSGGSMSEVEFSHEYWMRHALTLAKRARDEREVPVGAVLVLNNRVIGEGWNRAIGLHDPTAHAEIMALRQGGLVMQNYRLIDATLYVTFEPCVMCAGAMIHSRIGRVVFGVRNAKTGAAGSLMDVLHYPGMNHRVEITEGILADECAALLCYFFRMPRQVFNAQKKAQSSTDKRPAATKKAGQAKKKK

SEQ ID NO: 288 - protein, 971 aa, synthetic construct
  REGION 1..971: note = dTnpB(D354A)-ABE-N1
MSEVEFSHEYWMRHALTLAKRAWDEREVPVGAVLVHNNRVIGEGWNRPIGRHDPTAHAEIMALRQGGLVMQNYRLIDATLYVTLEPCVMCAGAMIHSRIGRVVFGARDAKTGAAGSLMDVLHHPGMNHRVEITEGILADECAALLSDFFRMRRQEIKAQKKAQSSTDSGGSSGGSSGSETPGTSESATPESSGGSSGGSMSEVEFSHEYWMRHALTLAKRARDEREVPVGAVLVLNNRVIGEGWNRAIGLHDPTAHAEIMALRQGGLVMQNYRLIDATLYVTFEPCVMCAGAMIHSRIGRVVFGVRNAKTGAAGSLMDVLHYPGMNHRVEITEGILADECAALLCYFFRMPRQVFNAQKKAQSSTDSGGSSGGSSGSETPGTSESATPESSGGSSGGSMGEKSSRRRRNGKSGAWTAAITSCVGGKMAKNTITKTLKLRIVRPYNSAEVEKIVADEKNNREKIALEKNKDKVKEACSKHLKVAAYCTTQVERNACLFCKARKLDDKFYQKLRGQFPDAVFWQEISEIFRQLQKQAAEIYNQSLIELYYEIFIKGKGIANASSVEHYLSDVCYTRAAELFKNAAIASGLRSKIKSNFRLKELKNMKSGLPTTKSDNFPIPLVKQKGGQYTGFEISNHNSDFIIKIPFGRWQVKKEIDKYRPWEKFDFEQVQKSPKPISLLLSTQRRKRNKGWSKDEGTEAEIKKVMNGDYQTSYIEVKRGSKIGEKSAWMLNLSIDVPKIDKGVDPSIIGGIAVGVKSPLVCAINNAFSRYSISDNDLFHFNKKMFARRRILLKKNRHKRAGHGAKNKLKPITILTEKSERFRKKLIERWACEIADFFIKNKVGTVQMENLESMKRKEDSYFNIRLRGFWPYAEMQNKIEFKLKQYGIEIRKVAPNNTSKTCSKCGHLNNYFNFEYRKKNKFPHFKCEKCNFKENADYNAALNISNPKLKSTKEEPKRPAATKKAGQAKKKK

SEQ ID NO: 289 - protein, 971 aa, synthetic construct
  REGION 1..971: note = dTnpB(D354A)-ABE-N2
MSEVEFSHEYWMRHALTLAKRARDEREVPVGAVLVLNNRVIGEGWNRAIGLHDPTAHAEIMALRQGGLVMQNYRLIDATLYVTFEPCVMCAGAMIHSRIGRVVFGVRNAKTGAAGSLMDVLHYPGMNHRVEITEGILADECAALLCYFFRMPRQVFNAQKKAQSSTDSGGSSGGSSGSETPGTSESATPESSGGSSGGSMSEVEFSHEYWMRHALTLAKRAWDEREVPVGAVLVHNNRVIGEGWNRPIGRHDPTAHAEIMALRQGGLVMQNYRLIDATLYVTLEPCVMCAGAMIHSRIGRVVFGARDAKTGAAGSLMDVLHHPGMNHRVEITEGILADECAALLSDFFRMRRQEIKAQKKAQSSTDSGGSSGGSSGSETPGTSESATPESSGGSSGGSMGEKSSRRRRNGKSGAWTAAITSCVGGKMAKNTITKTLKLRIVRPYNSAEVEKIVADEKNNREKIALEKNKDKVKEACSKHLKVAAYCTTQVERNACLFCKARKLDDKFYQKLRGQFPDAVFWQEISEIFRQLQKQAAEIYNQSLIELYYEIFIKGKGIANASSVEHYLSDVCYTRAAELFKNAAIASGLRSKIKSNFRLKELKNMKSGLPTTKSDNFPIPLVKQKGGQYTGFEISNHNSDFIIKIPFGRWQVKKEIDKYRPWEKFDFEQVQKSPKPISLLLSTQRRKRNKGWSKDEGTEAEIKKVMNGDYQTSYIEVKRGSKIGEKSAWMLNLSIDVPKIDKGVDPSIIGGIAVGVKSPLVCAINNAFSRYSISDNDLFHFNKKMFARRRILLKKNRHKRAGHGAKNKLKPITILTEKSERFRKKLIERWACEIADFFIKNKVGTVQMENLESMKRKEDSYFNIRLRGFWPYAEMQNKIEFKLKQYGIEIRKVAPNNTSKTCSKCGHLNNYFNFEYRKKNKFPHFKCEKCNFKENADYNAALNISNPKLKSTKEEPKRPAATKKAGQAKKKK

SEQ ID NO: 290 - protein, 971 aa, synthetic construct
  REGION 1..971: note = dTnpB(D354A)-ABE-C1
MGEKSSRRRRNGKSGAWTAAITSCVGGKMAKNTITKTLKLRIVRPYNSAEVEKIVADEKNNREKIALEKNKDKVKEACSKHLKVAAYCTTQVERNACLFCKARKLDDKFYQKLRGQFPDAVFWQEISEIFRQLQKQAAEIYNQSLIELYYEIFIKGKGIANASSVEHYLSDVCYTRAAELFKNAAIASGLRSKIKSNFRLKELKNMKSGLPTTKSDNFPIPLVKQKGGQYTGFEISNHNSDFIIKIPFGRWQVKKEIDKYRPWEKFDFEQVQKSPKPISLLLSTQRRKRNKGWSKDEGTEAEIKKVMNGDYQTSYIEVKRGSKIGEKSAWMLNLSIDVPKIDKGVDPSIIGGIAVGVKSPLVCAINNAFSRYSISDNDLFHFNKKMFARRRILLKKNRHKRAGHGAKNKLKPITILTEKSERFRKKLIERWACEIADFFIKNKVGTVQMENLESMKRKEDSYFNIRLRGFWPYAEMQNKIEFKLKQYGIEIRKVAPNNTSKTCSKCGHLNNYFNFEYRKKNKFPHFKCEKCNFKENADYNAALNISNPKLKSTKEEPSGGSSGGSSGSETPGTSESATPESSGGSSGGSMSEVEFSHEYWMRHALTLAKRARDEREVPVGAVLVLNNRVIGEGWNRAIGLHDPTAHAEIMALRQGGLVMQNYRLIDATLYVTFEPCVMCAGAMIHSRIGRVVFGVRNAKTGAAGSLMDVLHYPGMNHRVEITEGILADECAALLCYFFRMPRQVFNAQKKAQSSTDSGGSSGGSSGSETPGTSESATPESSGGSSGGSMSEVEFSHEYWMRHALTLAKRAWDEREVPVGAVLVHNNRVIGEGWNRPIGRHDPTAHAEIMALRQGGLVMQNYRLIDATLYVTLEPCVMCAGAMIHSRIGRVVFGARDAKTGAAGSLMDVLHHPGMNHRVEITEGILADECAALLSDFFRMRRQEIKAQKKAQSSTDKRPAATKKAGQAKKKK

SEQ ID NO: 291 - protein, 971 aa, synthetic construct
  REGION 1..971: note = dTnpB(D354A)-ABE-C2
MGEKSSRRRRNGKSGAWTAAITSCVGGKMAKNTITKTLKLRIVRPYNSAEVEKIVADEKNNREKIALEKNKDKVKEACSKHLKVAAYCTTQVERNACLFCKARKLDDKFYQKLRGQFPDAVFWQEISEIFRQLQKQAAEIYNQSLIELYYEIFIKGKGIANASSVEHYLSDVCYTRAAELFKNAAIASGLRSKIKSNFRLKELKNMKSGLPTTKSDNFPIPLVKQKGGQYTGFEISNHNSDFIIKIPFGRWQVKKEIDKYRPWEKFDFEQVQKSPKPISLLLSTQRRKRNKGWSKDEGTEAEIKKVMNGDYQTSYIEVKRGSKIGEKSAWMLNLSIDVPKIDKGVDPSIIGGIAVGVKSPLVCAINNAFSRYSISDNDLFHFNKKMFARRRILLKKNRHKRAGHGAKNKLKPITILTEKSERFRKKLIERWACEIADFFIKNKVGTVQMENLESMKRKEDSYFNIRLRGFWPYAEMQNKIEFKLKQYGIEIRKVAPNNTSKTCSKCGHLNNYFNFEYRKKNKFPHFKCEKCNFKENADYNAALNISNPKLKSTKEEPSGGSSGGSSGSETPGTSESATPESSGGSSGGSMSEVEFSHEYWMRHALTLAKRAWDEREVPVGAVLVHNNRVIGEGWNRPIGRHDPTAHAEIMALRQGGLVMQNYRLIDATLYVTLEPCVMCAGAMIHSRIGRVVFGARDAKTGAAGSLMDVLHHPGMNHRVEITEGILADECAALLSDFFRMRRQEIKAQKKAQSSTDSGGSSGGSSGSETPGTSESATPESSGGSSGGSMSEVEFSHEYWMRHALTLAKRARDEREVPVGAVLVLNNRVIGEGWNRAIGLHDPTAHAEIMALRQGGLVMQNYRLIDATLYVTFEPCVMCAGAMIHSRIGRVVFGVRNAKTGAAGSLMDVLHYPGMNHRVEITEGILADECAALLCYFFRMPRQVFNAQKKAQSSTDKRPAATKKAGQAKKKK

SEQ ID NO: 292 - protein, 943 aa, synthetic construct
  REGION 1..943: note = dCas12f1(E422A)-ABE-C2
MAKNTITKTLKLRIVRPYNSAEVEKIVADEKNNREKIALEKNKDKVKEACSKHLKVAAYCTTQVERNACLFCKARKLDDKFYQKLRGQFPDAVFWQEISEIFRQLQKQAAEIYNQSLIELYYEIFIKGKGIANASSVEHYLSDVCYTRAAELFKNAAIASGLRSKIKSNFRLKELKNMKSGLPTTKSDNFPIPLVKQKGGQYTGFEISNHNSDFIIKIPFGRWQVKKEIDKYRPWEKFDFEQVQKSPKPISLLLSTQRRKRNKGWSKDEGTEAEIKKVMNGDYQTSYIEVKRGSKIGEKSAWMLNLSIDVPKIDKGVDPSIIGGIDVGVKSPLVCAINNAFSRYSISDNDLFHFNKKMFARRRILLKKNRHKRAGHGAKNKLKPITILTEKSERFRKKLIERWACEIADFFIKNKVGTVQMANLESMKRKEDSYFNIRLRGFWPYAEMQNKIEFKLKQYGIEIRKVAPNNTSKTCSKCGHLNNYFNFEYRKKNKFPHFKCEKCNFKENADYNAALNISNPKLKSTKEEPSGGSSGGSSGSETPGTSESATPESSGGSSGGSMSEVEFSHEYWMRHALTLAKRAWDEREVPVGAVLVHNNRVIGEGWNRPIGRHDPTAHAEIMALRQGGLVMQNYRLIDATLYVTLEPCVMCAGAMIHSRIGRVVFGARDAKTGAAGSLMDVLHHPGMNHRVEITEGILADECAALLSDFFRMRRQEIKAQKKAQSSTDSGGSSGGSSGSETPGTSESATPESSGGSSGGSMSEVEFSHEYWMRHALTLAKRARDEREVPVGAVLVLNNRVIGEGWNRAIGLHDPTAHAEIMALRQGGLVMQNYRLIDATLYVTFEPCVMCAGAMIHSRIGRVVFGVRNAKTGAAGSLMDVLHYPGMNHRVEITEGILADECAALLCYFFRMPRQVFNAQKKAQSSTDKRPAATKKAGQAKKKK

SEQ ID NO: 293 - protein, 943 aa, synthetic construct
  REGION 1..943: note = dCas12f1(R490A)-ABE-C2
MAKNTITKTLKLRIVRPYNSAEVEKIVADEKNNREKIALEKNKDKVKEACSKHLKVAAYCTTQVERNACLFCKARKLDDKFYQKLRGQFPDAVFWQEISEIFRQLQKQAAEIYNQSLIELYYEIFIKGKGIANASSVEHYLSDVCYTRAAELFKNAAIASGLRSKIKSNFRLKELKNMKSGLPTTKSDNFPIPLVKQKGGQYTGFEISNHNSDFIIKIPFGRWQVKKEIDKYRPWEKFDFEQVQKSPKPISLLLSTQRRKRNKGWSKDEGTEAEIKKVMNGDYQTSYIEVKRGSKIGEKSAWMLNLSIDVPKIDKGVDPSIIGGIDVGVKSPLVCAINNAFSRYSISDNDLFHFNKKMFARRRILLKKNRHKRAGHGAKNKLKPITILTEKSERFRKKLIERWACEIADFFIKNKVGTVQMENLESMKRKEDSYFNIRLRGFWPYAEMQNKIEFKLKQYGIEIRKVAPNNTSKTCSKCGHLNNYFNFEYAKKNKFPHFKCEKCNFKENADYNAALNISNPKLKSTKEEPSGGSSGGSSGSETPGTSESATPESSGGSSGGSMSEVEFSHEYWMRHALTLAKRAWDEREVPVGAVLVHNNRVIGEGWNRPIGRHDPTAHAEIMALRQGGLVMQNYRLIDATLYVTLEPCVMCAGAMIHSRIGRVVFGARDAKTGAAGSLMDVLHHPGMNHRVEITEGILADECAALLSDFFRMRRQEIKAQKKAQSSTDSGGSSGGSSGSETPGTSESATPESSGGSSGGSMSEVEFSHEYWMRHALTLAKRARDEREVPVGAVLVLNNRVIGEGWNRAIGLHDPTAHAEIMALRQGGLVMQNYRLIDATLYVTFEPCVMCAGAMIHSRIGRVVFGVRNAKTGAAGSLMDVLHYPGMNHRVEITEGILADECAALLCYFFRMPRQVFNAQKKAQSSTDKRPAATKKAGQAKKKK

SEQ ID NO: 294 - protein, 943 aa, synthetic construct
  REGION 1..943: note = dCas12f1(D510A)-ABE-C2
MAKNTITKTLKLRIVRPYNSAEVEKIVADEKNNREKIALEKNKDKVKEACSKHLKVAAYCTTQVERNACLFCKARKLDDKFYQKLRGQFPDAVFWQEISEIFRQLQKQAAEIYNQSLIELYYEIFIKGKGIANASSVEHYLSDVCYTRAAELFKNAAIASGLRSKIKSNFRLKELKNMKSGLPTTKSDNFPIPLVKQKGGQYTGFEISNHNSDFIIKIPFGRWQVKKEIDKYRPWEKFDFEQVQKSPKPISLLLSTQRRKRNKGWSKDEGTEAEIKKVMNGDYQTSYIEVKRGSKIGEKSAWMLNLSIDVPKIDKGVDPSIIGGIDVGVKSPLVCAINNAFSRYSISDNDLFHFNKKMFARRRILLKKNRHKRAGHGAKNKLKPITILTEKSERFRKKLIERWACEIADFFIKNKVGTVQMENLESMKRKEDSYFNIRLRGFWPYAEMQNKIEFKLKQYGIEIRKVAPNNTSKTCSKCGHLNNYFNFEYRKKNKFPHFKCEKCNFKENAAYNAALNISNPKLKSTKEEPSGGSSGGSSGSETPGTSESATPESSGGSSGGSMSEVEFSHEYWMRHALTLAKRAWDEREVPVGAVLVHNNRVIGEGWNRPIGRHDPTAHAEIMALRQGGLVMQNYRLIDATLYVTLEPCVMCAGAMIHSRIGRVVFGARDAKTGAAGSLMDVLHHPGMNHRVEITEGILADECAALLSDFFRMRRQEIKAQKKAQSSTDSGGSSGGSSGSETPGTSESATPESSGGSSGGSMSEVEFSHEYWMRHALTLAKRARDEREVPVGAVLVLNNRVIGEGWNRAIGLHDPTAHAEIMALRQGGLVMQNYRLIDATLYVTFEPCVMCAGAMIHSRIGRVVFGVRNAKTGAAGSLMDVLHYPGMNHRVEITEGILADECAALLCYFFRMPRQVFNAQKKAQSSTDKRPAATKKAGQAKKKK

SEQ ID NO: 295 - protein, 971 aa, synthetic construct
  REGION 1..971: note = dTnpb(E450A)-ABE-C2
MGEKSSRRRRNGKSGAWTAAITSCVGGKMAKNTITKTLKLRIVRPYNSAEVEKIVADEKNNREKIALEKNKDKVKEACSKHLKVAAYCTTQVERNACLFCKARKLDDKFYQKLRGQFPDAVFWQEISEIFRQLQKQAAEIYNQSLIELYYEIFIKGKGIANASSVEHYLSDVCYTRAAELFKNAAIASGLRSKIKSNFRLKELKNMKSGLPTTKSDNFPIPLVKQKGGQYTGFEISNHNSDFIIKIPFGRWQVKKEIDKYRPWEKFDFEQVQKSPKPISLLLSTQRRKRNKGWSKDEGTEAEIKKVMNGDYQTSYIEVKRGSKIGEKSAWMLNLSIDVPKIDKGVDPSIIGGIDVGVKSPLVCAINNAFSRYSISDNDLFHFNKKMFARRRILLKKNRHKRAGHGAKNKLKPITILTEKSERFRKKLIERWACEIADFFIKNKVGTVQMANLESMKRKEDSYFNIRLRGFWPYAEMQNKIEFKLKQYGIEIRKVAPNNTSKTCSKCGHLNNYFNFEYRKKNKFPHFKCEKCNFKENADYNAALNISNPKLKSTKEEPSGGSSGGSSGSETPGTSESATPESSGGSSGGSMSEVEFSHEYWMRHALTLAKRAWDEREVPVGAVLVHNNRVIGEGWNRPIGRHDPTAHAEIMALRQGGLVMQNYRLIDATLYVTLEPCVMCAGAMIHSRIGRVVFGARDAKTGAAGSLMDVLHHPGMNHRVEITEGILADECAALLSDFFRMRRQEIKAQKKAQSSTDSGGSSGGSSGSETPGTSESATPESSGGSSGGSMSEVEFSHEYWMRHALTLAKRARDEREVPVGAVLVLNNRVIGEGWNRAIGLHDPTAHAEIMALRQGGLVMQNYRLIDATLYVTFEPCVMCAGAMIHSRIGRVVFGVRNAKTGAAGSLMDVLHYPGMNHRVEITEGILADECAALLCYFFRMPRQVFNAQKKAQSSTDKRPAATKKAGQAKKKK

SEQ ID NO: 296 - protein, 971 aa, synthetic construct
  REGION 1..971: note = dTnpb(R518A)-ABE-C2
MGEKSSRRRRNGKSGAWTAAITSCVGGKMAKNTITKTLKLRIVRPYNSAEVEKIVADEKNNREKIALEKNKDKVKEACSKHLKVAAYCTTQVERNACLFCKARKLDDKFYQKLRGQFPDAVFWQEISEIFRQLQKQAAEIYNQSLIELYYEIFIKGKGIANASSVEHYLSDVCYTRAAELFKNAAIASGLRSKIKSNFRLKELKNMKSGLPTTKSDNFPIPLVKQKGGQYTGFEISNHNSDFIIKIPFGRWQVKKEIDKYRPWEKFDFEQVQKSPKPISLLLSTQRRKRNKGWSKDEGTEAEIKKVMNGDYQTSYIEVKRGSKIGEKSAWMLNLSIDVPKIDKGVDPSIIGGIDVGVKSPLVCAINNAFSRYSISDNDLFHFNKKMFARRRILLKKNRHKRAGHGAKNKLKPITILTEKSERFRKKLIERWACEIADFFIKNKVGTVQMENLESMKRKEDSYFNIRLRGFWPYAEMQNKIEFKLKQYGIEIRKVAPNNTSKTCSKCGHLNNYFNFEYAKKNKFPHFKCEKCNFKENADYNAALNISNPKLKSTKEEPSGGSSGGSSGSETPGTSESATPESSGGSSGGSMSEVEFSHEYWMRHALTLAKRAWDEREVPVGAVLVHNNRVIGEGWNRPIGRHDPTAHAEIMALRQGGLVMQNYRLIDATLYVTLEPCVMCAGAMIHSRIGRVVFGARDAKTGAAGSLMDVLHHPGMNHRVEITEGILADECAALLSDFFRMRRQEIKAQKKAQSSTDSGGSSGGSSGSETPGTSESATPESSGGSSGGSMSEVEFSHEYWMRHALTLAKRARDEREVPVGAVLVLNNRVIGEGWNRAIGLHDPTAHAEIMALRQGGLVMQNYRLIDATLYVTFEPCVMCAGAMIHSRIGRVVFGVRNAKTGAAGSLMDVLHYPGMNHRVEITEGILADECAALLCYFFRMPRQVFNAQKKAQSSTDKRPAATKKAGQAKKKK

SEQ ID NO: 297 - protein, 971 aa, synthetic construct
  REGION 1..971: note = dTnpb(D538A)-ABE-C2
MGEKSSRRRRNGKSGAWTAAITSCVGGKMAKNTITKTLKLRIVRPYNSAEVEKIVADEKNNREKIALEKNKDKVKEACSKHLKVAAYCTTQVERNACLFCKARKLDDKFYQKLRGQFPDAVFWQEISEIFRQLQKQAAEIYNQSLIELYYEIFIKGKGIANASSVEHYLSDVCYTRAAELFKNAAIASGLRSKIKSNFRLKELKNMKSGLPTTKSDNFPIPLVKQKGGQYTGFEISNHNSDFIIKIPFGRWQVKKEIDKYRPWEKFDFEQVQKSPKPISLLLSTQRRKRNKGWSKDEGTEAEIKKVMNGDYQTSYIEVKRGSKIGEKSAWMLNLSIDVPKIDKGVDPSIIGGIDVGVKSPLVCAINNAFSRYSISDNDLFHFNKKMFARRRILLKKNRHKRAGHGAKNKLKPITILTEKSERFRKKLIERWACEIADFFIKNKVGTVQMENLESMKRKEDSYFNIRLRGFWPYAEMQNKIEFKLKQYGIEIRKVAPNNTSKTCSKCGHLNNYFNFEYRKKNKFPHFKCEKCNFKENAAYNAALNISNPKLKSTKEEPSGGSSGGSSGSETPGTSESATPESSGGSSGGSMSEVEFSHEYWMRHALTLAKRAWDEREVPVGAVLVHNNRVIGEGWNRPIGRHDPTAHAEIMALRQGGLVMQNYRLIDATLYVTLEPCVMCAGAMIHSRIGRVVFGARDAKTGAAGSLMDVLHHPGMNHRVEITEGILADECAALLSDFFRMRRQEIKAQKKAQSSTDSGGSSGGSSGSETPGTSESATPESSGGSSGGSMSEVEFSHEYWMRHALTLAKRARDEREVPVGAVLVLNNRVIGEGWNRAIGLHDPTAHAEIMALRQGGLVMQNYRLIDATLYVTFEPCVMCAGAMIHSRIGRVVFGVRNAKTGAAGSLMDVLHYPGMNHRVEITEGILADECAALLCYFFRMPRQVFNAQKKAQSSTDKRPAATKKAGQAKKKK

SEQ ID NO: 298 - protein, 971 aa, synthetic construct
  REGION 1..971: note = dTnpB(D538A)-ABE-C3.1(TadA-eTadA3)
MGEKSSRRRRNGKSGAWTAAITSCVGGKMAKNTITKTLKLRIVRPYNSAEVEKIVADEKNNREKIALEKNKDKVKEACSKHLKVAAYCTTQVERNACLFCKARKLDDKFYQKLRGQFPDAVFWQEISEIFRQLQKQAAEIYNQSLIELYYEIFIKGKGIANASSVEHYLSDVCYTRAAELFKNAAIASGLRSKIKSNFRLKELKNMKSGLPTTKSDNFPIPLVKQKGGQYTGFEISNHNSDFIIKIPFGRWQVKKEIDKYRPWEKFDFEQVQKSPKPISLLLSTQRRKRNKGWSKDEGTEAEIKKVMNGDYQTSYIEVKRGSKIGEKSAWMLNLSIDVPKIDKGVDPSIIGGIDVGVKSPLVCAINNAFSRYSISDNDLFHFNKKMFARRRILLKKNRHKRAGHGAKNKLKPITILTEKSERFRKKLIERWACEIADFFIKNKVGTVQMENLESMKRKEDSYFNIRLRGFWPYAEMQNKIEFKLKQYGIEIRKVAPNNTSKTCSKCGHLNNYFNFEYRKKNKFPHFKCEKCNFKENAAYNAALNISNPKLKSTKEEPSGGSSGGSSGSETPGTSESATPESSGGSSGGSMSEVEFSHEYWMRHALTLAKRAWDEREVPVGAVLVHNNRVIGEGWNRPIGRHDPTAHAEIMALRQGGLVMQNYRLIDATLYVTLEPCVMCAGAMIHSRIGRVVFGARDAKTGAAGSLMDVLHHPGMNHRVEITEGILADECAALLSDFFRMRRQEIKAQKKAQSSTDSGGSSGGSSGSETPGTSESATPESSGGSSGGSMSEVEFSHEYWMRHALTLAKRARDEREVPVGAVLVLNNRVIGEGWNRAIGLHDPTAHAEIMALRQGGLVMQNYRLIDATLYVTFEPCVMCAGAMIHSRIGRVVFGWRQSKRGAAGSLMNVLNYPGMNHRVEITEGILADECAALLCDFYRMPRQVFNAQKKAQSSINKRPAATKKAGQAKKKK

SEQ ID NO: 299 - protein, 971 aa, synthetic construct
  REGION 1..971: note = dTnpB(D354A)-ABE-C3.1(TadA-eTadA3)
MGEKSSRRRRNGKSGAWTAAITSCVGGKMAKNTITKTLKLRIVRPYNSAEVEKIVADEKNNREKIALEKNKDKVKEACSKHLKVAAYCTTQVERNACLFCKARKLDDKFYQKLRGQFPDAVFWQEISEIFRQLQKQAAEIYNQSLIELYYEIFIKGKGIANASSVEHYLSDVCYTRAAELFKNAAIASGLRSKIKSNFRLKELKNMKSGLPTTKSDNFPIPLVKQKGGQYTGFEISNHNSDFIIKIPFGRWQVKKEIDKYRPWEKFDFEQVQKSPKPISLLLSTQRRKRNKGWSKDEGTEAEIKKVMNGDYQTSYIEVKRGSKIGEKSAWMLNLSIDVPKIDKGVDPSIIGGIAVGVKSPLVCAINNAFSRYSISDNDLFHFNKKMFARRRILLKKNRHKRAGHGAKNKLKPITILTEKSERFRKKLIERWACEIADFFIKNKVGTVQMENLESMKRKEDSYFNIRLRGFWPYAEMQNKIEFKLKQYGIEIRKVAPNNTSKTCSKCGHLNNYFNFEYRKKNKFPHFKCEKCNFKENADYNAALNISNPKLKSTKEEPSGGSSGGSSGSETPGTSESATPESSGGSSGGSMSEVEFSHEYWMRHALTLAKRAWDEREVPVGAVLVHNNRVIGEGWNRPIGRHDPTAHAEIMALRQGGLVMQNYRLIDATLYVTLEPCVMCAGAMIHSRIGRVVFGARDAKTGAAGSLMDVLHHPGMNHRVEITEGILADECAALLSDFFRMRRQEIKAQKKAQSSTDSGGSSGGSSGSETPGTSESATPESSGGSSGGSMSEVEFSHEYWMRHALTLAKRARDEREVPVGAVLVLNNRVIGEGWNRAIGLHDPTAHAEIMALRQGGLVMQNYRLIDATLYVTFEPCVMCAGAMIHSRIGRVVFGWRQSKRGAAGSLMNVLNYPGMNHRVEITEGILADECAALLCDFYRMPRQVFNAQKKAQSSINKRPAATKKAGQAKKKK

SEQ ID NO: 300 - protein, 943 aa, synthetic construct
  REGION 1..943: note = d12f1_05(D510A, I131W)-ABE-C2
MAKNTITKTLKLRIVRPYNSAEVEKIVADEKNNREKIALEKNKDKVKEACSKHLKVAAYCTTQVERNACLFCKARKLDDKFYQKLRGQFPDAVFWQEISEIFRQLQKQAAEIYNQSLIELYYEIFIKGKGWANASSVEHYLSDVCYTRAAELFKNAAIASGLRSKIKSNFRLKELKNMKSGLPTTKSDNFPIPLVKQKGGQYTGFEISNHNSDFIIKIPFGRWQVKKEIDKYRPWEKFDFEQVQKSPKPISLLLSTQRRKRNKGWSKDEGTEAEIKKVMNGDYQTSYIEVKRGSKIGEKSAWMLNLSIDVPKIDKGVDPSIIGGIDVGVKSPLVCAINNAFSRYSISDNDLFHFNKKMFARRRILLKKNRHKRAGHGAKNKLKPITILTEKSERFRKKLIERWACEIADFFIKNKVGTVQMENLESMKRKEDSYFNIRLRGFWPYAEMQNKIEFKLKQYGIEIRKVAPNNTSKTCSKCGHLNNYFNFEYRKKNKFPHFKCEKCNFKENAAYNAALNISNPKLKSTKEEPSGGSSGGSSGSETPGTSESATPESSGGSSGGSMSEVEFSHEYWMRHALTLAKRAWDEREVPVGAVLVHNNRVIGEGWNRPIGRHDPTAHAEIMALRQGGLVMQNYRLIDATLYVTLEPCVMCAGAMIHSRIGRVVFGARDAKTGAAGSLMDVLHHPGMNHRVEITEGILADECAALLSDFFRMRRQEIKAQKKAQSSTDSGGSSGGSSGSETPGTSESATPESSGGSSGGSMSEVEFSHEYWMRHALTLAKRARDEREVPVGAVLVLNNRVIGEGWNRAIGLHDPTAHAEIMALRQGGLVMQNYRLIDATLYVTFEPCVMCAGAMIHSRIGRVVFGVRNAKTGAAGSLMDVLHYPGMNHRVEITEGILADECAALLCYFFRMPRQVFNAQKKAQSSTDKRPAATKKAGQAKKKK

SEQ ID NO: 301 - protein, 943 aa, synthetic construct
  REGION 1..943: note = d12f1_06(D510A, S136Y)-ABE-C2
MAKNTITKTLKLRIVRPYNSAEVEKIVADEKNNREKIALEKNKDKVKEACSKHLKVAAYCTTQVERNACLFCKARKLDDKFYQKLRGQFPDAVFWQEISEIFRQLQKQAAEIYNQSLIELYYEIFIKGKGIANASYVEHYLSDVCYTRAAELFKNAAIASGLRSKIKSNFRLKELKNMKSGLPTTKSDNFPIPLVKQKGGQYTGFEISNHNSDFIIKIPFGRWQVKKEIDKYRPWEKFDFEQVQKSPKPISLLLSTQRRKRNKGWSKDEGTEAEIKKVMNGDYQTSYIEVKRGSKIGEKSAWMLNLSIDVPKIDKGVDPSIIGGIDVGVKSPLVCAINNAFSRYSISDNDLFHFNKKMFARRRILLKKNRHKRAGHGAKNKLKPITILTEKSERFRKKLIERWACEIADFFIKNKVGTVQMENLESMKRKEDSYFNIRLRGFWPYAEMQNKIEFKLKQYGIEIRKVAPNNTSKTCSKCGHLNNYFNFEYRKKNKFPHFKCEKCNFKENAAYNAALNISNPKLKSTKEEPSGGSSGGSSGSETPGTSESATPESSGGSSGGSMSEVEFSHEYWMRHALTLAKRAWDEREVPVGAVLVHNNRVIGEGWNRPIGRHDPTAHAEIMALRQGGLVMQNYRLIDATLYVTLEPCVMCAGAMIHSRIGRVVFGARDAKTGAAGSLMDVLHHPGMNHRVEITEGILADECAALLSDFFRMRRQEIKAQKKAQSSTDSGGSSGGSSGSETPGTSESATPESSGGSSGGSMSEVEFSHEYWMRHALTLAKRARDEREVPVGAVLVLNNRVIGEGWNRAIGLHDPTAHAEIMALRQGGLVMQNYRLIDATLYVTFEPCVMCAGAMIHSRIGRVVFGVRNAKTGAAGSLMDVLHYPGMNHRVEITEGILADECAALLCYFFRMPRQVFNAQKKAQSSTDKRPAATKKAGQAKKKK

SEQ ID NO: 302 - protein, 943 aa, synthetic construct
  REGION 1..943: note = d12f1_07(D510A, I131W/S136Y)-ABE-C2
MAKNTITKTLKLRIVRPYNSAEVEKIVADEKNNREKIALEKNKDKVKEACSKHLKVAAYCTTQVERNACLFCKARKLDDKFYQKLRGQFPDAVFWQEISEIFRQLQKQAAEIYNQSLIELYYEIFIKGKGWANASYVEHYLSDVCYTRAAELFKNAAIASGLRSKIKSNFRLKELKNMKSGLPTTKSDNFPIPLVKQKGGQYTGFEISNHNSDFIIKIPFGRWQVKKEIDKYRPWEKFDFEQVQKSPKPISLLLSTQRRKRNKGWSKDEGTEAEIKKVMNGDYQTSYIEVKRGSKIGEKSAWMLNLSIDVPKIDKGVDPSIIGGIDVGVKSPLVCAINNAFSRYSISDNDLFHFNKKMFARRRILLKKNRHKRAGHGAKNKLKPITILTEKSERFRKKLIERWACEIADFFIKNKVGTVQMENLESMKRKEDSYFNIRLRGFWPYAEMQNKIEFKLKQYGIEIRKVAPNNTSKTCSKCGHLNNYFNFEYRKKNKFPHFKCEKCNFKENAAYNAALNISNPKLKSTKEEPSGGSSGGSSGSETPGTSESATPESSGGSSGGSMSEVEFSHEYWMRHALTLAKRAWDEREVPVGAVLVHNNRVIGEGWNRPIGRHDPTAHAEIMALRQGGLVMQNYRLIDATLYVTLEPCVMCAGAMIHSRIGRVVFGARDAKTGAAGSLMDVLHHPGMNHRVEITEGILADECAALLSDFFRMRRQEIKAQKKAQSSTDSGGSSGGSSGSETPGTSESATPESSGGSSGGSMSEVEFSHEYWMRHALTLAKRARDEREVPVGAVLVLNNRVIGEGWNRAIGLHDPTAHAEIMALRQGGLVMQNYRLIDATLYVTFEPCVMCAGAMIHSRIGRVVFGVRNAKTGAAGSLMDVLHYPGMNHRVEITEGILADECAALLCYFFRMPRQVFNAQKKAQSSTDKRPAATKKAGQAKKKK

SEQ ID NO: 303 - protein, 971 aa, synthetic construct
  REGION 1..971: note = dtnpb_05(D538, I159W)-ABE-C2
MGEKSSRRRRNGKSGAWTAAITSCVGGKMAKNTITKTLKLRIVRPYNSAEVEKIVADEKNNREKIALEKNKDKVKEACSKHLKVAAYCTTQVERNACLFCKARKLDDKFYQKLRGQFPDAVFWQEISEIFRQLQKQAAEIYNQSLIELYYEIFIKGKGWANASSVEHYLSDVCYTRAAELFKNAAIASGLRSKIKSNFRLKELKNMKSGLPTTKSDNFPIPLVKQKGGQYTGFEISNHNSDFIIKIPFGRWQVKKEIDKYRPWEKFDFEQVQKSPKPISLLLSTQRRKRNKGWSKDEGTEAEIKKVMNGDYQTSYIEVKRGSKIGEKSAWMLNLSIDVPKIDKGVDPSIIGGIDVGVKSPLVCAINNAFSRYSISDNDLFHFNKKMFARRRILLKKNRHKRAGHGAKNKLKPITILTEKSERFRKKLIERWACEIADFFIKNKVGTVQMENLESMKRKEDSYFNIRLRGFWPYAEMQNKIEFKLKQYGIEIRKVAPNNTSKTCSKCGHLNNYFNFEYRKKNKFPHFKCEKCNFKENAAYNAALNISNPKLKSTKEEPSGGSSGGSSGSETPGTSESATPESSGGSSGGSMSEVEFSHEYWMRHALTLAKRAWDEREVPVGAVLVHNNRVIGEGWNRPIGRHDPTAHAEIMALRQGGLVMQNYRLIDATLYVTLEPCVMCAGAMIHSRIGRVVFGARDAKTGAAGSLMDVLHHPGMNHRVEITEGILADECAALLSDFFRMRRQEIKAQKKAQSSTDSGGSSGGSSGSETPGTSESATPESSGGSSGGSMSEVEFSHEYWMRHALTLAKRARDEREVPVGAVLVLNNRVIGEGWNRAIGLHDPTAHAEIMALRQGGLVMQNYRLIDATLYVTFEPCVMCAGAMIHSRIGRVVFGVRNAKTGAAGSLMDVLHYPGMNHRVEITEGILADECAALLCYFFRMPRQVFNAQKKAQSSTDKRPAATKKAGQAKKKK

SEQ ID NO: 304 - protein, 971 aa, synthetic construct
  REGION 1..971: note = dtnpb_06(D538, S164Y)-ABE-C2
MGEKSSRRRRNGKSGAWTAAITSCVGGKMAKNTITKTLKLRIVRPYNSAEVEKIVADEKNNREKIALEKNKDKVKEACSKHLKVAAYCTTQVERNACLFCKARKLDDKFYQKLRGQFPDAVFWQEISEIFRQLQKQAAEIYNQSLIELYYEIFIKGKGIANASYVEHYLSDVCYTRAAELFKNAAIASGLRSKIKSNFRLKELKNMKSGLPTTKSDNFPIPLVKQKGGQYTGFEISNHNSDFIIKIPFGRWQVKKEIDKYRPWEKFDFEQVQKSPKPISLLLSTQRRKRNKGWSKDEGTEAEIKKVMNGDYQTSYIEVKRGSKIGEKSAWMLNLSIDVPKIDKGVDPSIIGGIDVGVKSPLVCAINNAFSRYSISDNDLFHFNKKMFARRRILLKKNRHKRAGHGAKNKLKPITILTEKSERFRKKLIERWACEIADFFIKNKVGTVQMENLESMKRKEDSYFNIRLRGFWPYAEMQNKIEFKLKQYGIEIRKVAPNNTSKTCSKCGHLNNYFNFEYRKKNKFPHFKCEKCNFKENAAYNAALNISNPKLKSTKEEPSGGSSGGSSGSETPGTSESATPESSGGSSGGSMSEVEFSHEYWMRHALTLAKRAWDEREVPVGAVLVHNNRVIGEGWNRPIGRHDPTAHAEIMALRQGGLVMQNYRLIDATLYVTLEPCVMCAGAMIHSRIGRVVFGARDAKTGAAGSLMDVLHHPGMNHRVEITEGILADECAALLSDFFRMRRQEIKAQKKAQSSTDSGGSSGGSSGSETPGTSESATPESSGGSSGGSMSEVEFSHEYWMRHALTLAKRARDEREVPVGAVLVLNNRVIGEGWNRAIGLHDPTAHAEIMALRQGGLVMQNYRLIDATLYVTFEPCVMCAGAMIHSRIGRVVFGVRNAKTGAAGSLMDVLHYPGMNHRVEITEGILADECAALLCYFFRMPRQVFNAQKKAQSSTDKRPAATKKAGQAKKKK

SEQ ID NO: 305 - protein, 971 aa, synthetic construct
  REGION 1..971: note = dtnpb_07(D538, I159W/S164Y)-ABE-C2
MGEKSSRRRRNGKSGAWTAAITSCVGGKMAKNTITKTLKLRIVRPYNSAEVEKIVADEKNNREKIALEKNKDKVKEACSKHLKVAAYCTTQVERNACLFCKARKLDDKFYQKLRGQFPDAVFWQEISEIFRQLQKQAAEIYNQSLIELYYEIFIKGKGWANASYVEHYLSDVCYTRAAELFKNAAIASGLRSKIKSNFRLKELKNMKSGLPTTKSDNFPIPLVKQKGGQYTGFEISNHNSDFIIKIPFGRWQVKKEIDKYRPWEKFDFEQVQKSPKPISLLLSTQRRKRNKGWSKDEGTEAEIKKVMNGDYQTSYIEVKRGSKIGEKSAWMLNLSIDVPKIDKGVDPSIIGGIDVGVKSPLVCAINNAFSRYSISDNDLFHFNKKMFARRRILLKKNRHKRAGHGAKNKLKPITILTEKSERFRKKLIERWACEIADFFIKNKVGTVQMENLESMKRKEDSYFNIRLRGFWPYAEMQNKIEFKLKQYGIEIRKVAPNNTSKTCSKCGHLNNYFNFEYRKKNKFPHFKCEKCNFKENAAYNAALNISNPKLKSTKEEPSGGSSGGSSGSETPGTSESATPESSGGSSGGSMSEVEFSHEYWMRHALTLAKRAWDEREVPVGAVLVHNNRVIGEGWNRPIGRHDPTAHAEIMALRQGGLVMQNYRLIDATLYVTLEPCVMCAGAMIHSRIGRVVFGARDAKTGAAGSLMDVLHHPGMNHRVEITEGILADECAALLSDFFRMRRQEIKAQKKAQSSTDSGGSSGGSSGSETPGTSESATPESSGGSSGGSMSEVEFSHEYWMRHALTLAKRARDEREVPVGAVLVLNNRVIGEGWNRAIGLHDPTAHAEIMALRQGGLVMQNYRLIDATLYVTFEPCVMCAGAMIHSRIGRVVFGVRNAKTGAAGSLMDVLHYPGMNHRVEITEGILADECAALLCYFFRMPRQVFNAQKKAQSSTDKRPAATKKAGQAKKKK

SEQ ID NO: 306 - protein, 943 aa, synthetic construct
  REGION 1..943: note = d12f1(D326A)-dTadA-eTadA1
MAKNTITKTLKLRIVRPYNSAEVEKIVADEKNNREKIALEKNKDKVKEACSKHLKVAAYCTTQVERNACLFCKARKLDDKFYQKLRGQFPDAVFWQEISEIFRQLQKQAAEIYNQSLIELYYEIFIKGKGIANASSVEHYLSDVCYTRAAELFKNAAIASGLRSKIKSNFRLKELKNMKSGLPTTKSDNFPIPLVKQKGGQYTGFEISNHNSDFIIKIPFGRWQVKKEIDKYRPWEKFDFEQVQKSPKPISLLLSTQRRKRNKGWSKDEGTEAEIKKVMNGDYQTSYIEVKRGSKIGEKSAWMLNLSIDVPKIDKGVDPSIIGGIAVGVKSPLVCAINNAFSRYSISDNDLFHFNKKMFARRRILLKKNRHKRAGHGAKNKLKPITILTEKSERFRKKLIERWACEIADFFIKNKVGTVQMENLESMKRKEDSYFNIRLRGFWPYAEMQNKIEFKLKQYGIEIRKVAPNNTSKTCSKCGHLNNYFNFEYRKKNKFPHFKCEKCNFKENADYNAALNISNPKLKSTKEEPSGGSSGGSSGSETPGTSESATPESSGGSSGGSMSEVEFSHEYWMRHALTLAKRAWDEREVPVGAVLVHNNRVIGEGWNRPIGRHDPTAHAAIMALRQGGLVMQNYRLIDATLYVTLEPCVMCAGAMIHSRIGRVVFGARDAKTGAAGSLMDVLHHPGMNHRVEITEGILADECAALLSDFFRMRRQEIKAQKKAQSSTDSGGSSGGSSGSETPGTSESATPESSGGSSGGSMSEVEFSHEYWMRHALTLAKRARDEREVPVGAVLVLNNRVIGEGWNRAIGLHDPTAHAEIMALRQGGLVMQNYRLIDATLYVTFEPCVMCAGAMIHSRIGRVVFGVRNAKTGAAGSLMDVLHYPGMNHRVEITEGILADECAALLCYFFRMPRQVFNAQKKAQSSTDKRPAATKKAGQAKKKK

SEQ ID NO: 307 - protein, 943 aa, synthetic construct
  REGION 1..943: note = d12f1(D326A)-TadA-deTadA1
MAKNTITKTLKLRIVRPYNSAEVEKIVADEKNNREKIALEKNKDKVKEACSKHLKVAAYCTTQVERNACLFCKARKLDDKFYQKLRGQFPDAVFWQEISEIFRQLQKQAAEIYNQSLIELYYEIFIKGKGIANASSVEHYLSDVCYTRAAELFKNAAIASGLRSKIKSNFRLKELKNMKSGLPTTKSDNFPIPLVKQKGGQYTGFEISNHNSDFIIKIPFGRWQVKKEIDKYRPWEKFDFEQVQKSPKPISLLLSTQRRKRNKGWSKDEGTEAEIKKVMNGDYQTSYIEVKRGSKIGEKSAWMLNLSIDVPKIDKGVDPSIIGGIAVGVKSPLVCAINNAFSRYSISDNDLFHFNKKMFARRRILLKKNRHKRAGHGAKNKLKPITILTEKSERFRKKLIERWACEIADFFIKNKVGTVQMENLESMKRKEDSYFNIRLRGFWPYAEMQNKIEFKLKQYGIEIRKVAPNNTSKTCSKCGHLNNYFNFEYRKKNKFPHFKCEKCNFKENADYNAALNISNPKLKSTKEEPSGGSSGGSSGSETPGTSESATPESSGGSSGGSMSEVEFSHEYWMRHALTLAKRAWDEREVPVGAVLVHNNRVIGEGWNRPIGRHDPTAHAEIMALRQGGLVMQNYRLIDATLYVTLEPCVMCAGAMIHSRIGRVVFGARDAKTGAAGSLMDVLHHPGMNHRVEITEGILADECAALLSDFFRMRRQEIKAQKKAQSSTDSGGSSGGSSGSETPGTSESATPESSGGSSGGSMSEVEFSHEYWMRHALTLAKRARDEREVPVGAVLVLNNRVIGEGWNRAIGLHDPTAHAAIMALRQGGLVMQNYRLIDATLYVTFEPCVMCAGAMIHSRIGRVVFGVRNAKTGAAGSLMDVLHYPGMNHRVEITEGILADECAALLCYFFRMPRQVFNAQKKAQSSTDKRPAATKKAGQAKKKK

SEQ ID NO: 308 - protein, 943 aa, synthetic construct
  REGION 1..943: note = d12f1(D326A)-TadA-eTadA2
MAKNTITKTLKLRIVRPYNSAEVEKIVADEKNNREKIALEKNKDKVKEACSKHLKVAAYCTTQVERNACLFCKARKLDDKFYQKLRGQFPDAVFWQEISEIFRQLQKQAAEIYNQSLIELYYEIFIKGKGIANASSVEHYLSDVCYTRAAELFKNAAIASGLRSKIKSNFRLKELKNMKSGLPTTKSDNFPIPLVKQKGGQYTGFEISNHNSDFIIKIPFGRWQVKKEIDKYRPWEKFDFEQVQKSPKPISLLLSTQRRKRNKGWSKDEGTEAEIKKVMNGDYQTSYIEVKRGSKIGEKSAWMLNLSIDVPKIDKGVDPSIIGGIAVGVKSPLVCAINNAFSRYSISDNDLFHFNKKMFARRRILLKKNRHKRAGHGAKNKLKPITILTEKSERFRKKLIERWACEIADFFIKNKVGTVQMENLESMKRKEDSYFNIRLRGFWPYAEMQNKIEFKLKQYGIEIRKVAPNNTSKTCSKCGHLNNYFNFEYRKKNKFPHFKCEKCNFKENADYNAALNISNPKLKSTKEEPSGGSSGGSSGSETPGTSESATPESSGGSSGGSMSEVEFSHEYWMRHALTLAKRAWDEREVPVGAVLVHNNRVIGEGWNRPIGRHDPTAHAEIMALRQGGLVMQNYRLIDATLYVTLEPCVMCAGAMIHSRIGRVVFGARDAKTGAAGSLMDVLHHPGMNHRVEITEGILADECAALLSDFFRMRRQEIKAQKKAQSSTDSGGSSGGSSGSETPGTSESATPESSGGSSGGSMSEVEFSHEYWMRHALTLAKRARDEREVPVGAVLVLNNRVIGEGWNRAIGLHDPTAHAEIMALRQGGLVMQNYRLIDATLYVTFEPCVMCAGAMIHSRIGRVVFGWRNSKRGAAGSLMNVLNYPGMNHRVEITEGILADECAALLCDFYRMPRQVFNAQKKAQSSINKRPAATKKAGQAKKKK

SEQ ID NO: 309 - protein, 744 aa, synthetic construct
  REGION 1..744: note = d12f1(D326A)-eTadA2
MAKNTITKTLKLRIVRPYNSAEVEKIVADEKNNREKIALEKNKDKVKEACSKHLKVAAYCTTQVERNACLFCKARKLDDKFYQKLRGQFPDAVFWQEISEIFRQLQKQAAEIYNQSLIELYYEIFIKGKGIANASSVEHYLSDVCYTRAAELFKNAAIASGLRSKIKSNFRLKELKNMKSGLPTTKSDNFPIPLVKQKGGQYTGFEISNHNSDFIIKIPFGRWQVKKEIDKYRPWEKFDFEQVQKSPKPISLLLSTQRRKRNKGWSKDEGTEAEIKKVMNGDYQTSYIEVKRGSKIGEKSAWMLNLSIDVPKIDKGVDPSIIGGIAVGVKSPLVCAINNAFSRYSISDNDLFHFNKKMFARRRILLKKNRHKRAGHGAKNKLKPITILTEKSERFRKKLIERWACEIADFFIKNKVGTVQMENLESMKRKEDSYFNIRLRGFWPYAEMQNKIEFKLKQYGIEIRKVAPNNTSKTCSKCGHLNNYFNFEYRKKNKFPHFKCEKCNFKENADYNAALNISNPKLKSTKEEPSGGSSGGSSGSETPGTSESATPESSGGSSGGSMSEVEFSHEYWMRHALTLAKRARDEREVPVGAVLVLNNRVIGEGWNRAIGLHDPTAHAEIMALRQGGLVMQNYRLIDATLYVTFEPCVMCAGAMIHSRIGRVVFGWRNSKRGAAGSLMNVLNYPGMNHRVEITEGILADECAALLCDFYRMPRQVFNAQKKAQSSINKRPAATKKAGQAKKKK

SEQ ID NO: 310 - protein, 736 aa, synthetic construct
  REGION 1..736: note = d12f1(D326A)-eTadA4
MAKNTITKTLKLRIVRPYNSAEVEKIVADEKNNREKIALEKNKDKVKEACSKHLKVAAYCTTQVERNACLFCKARKLDDKFYQKLRGQFPDAVFWQEISEIFRQLQKQAAEIYNQSLIELYYEIFIKGKGIANASSVEHYLSDVCYTRAAELFKNAAIASGLRSKIKSNFRLKELKNMKSGLPTTKSDNFPIPLVKQKGGQYTGFEISNHNSDFIIKIPFGRWQVKKEIDKYRPWEKFDFEQVQKSPKPISLLLSTQRRKRNKGWSKDEGTEAEIKKVMNGDYQTSYIEVKRGSKIGEKSAWMLNLSIDVPKIDKGVDPSIIGGIAVGVKSPLVCAINNAFSRYSISDNDLFHFNKKMFARRRILLKKNRHKRAGHGAKNKLKPITILTEKSERFRKKLIERWACEIADFFIKNKVGTVQMENLESMKRKEDSYFNIRLRGFWPYAEMQNKIEFKLKQYGIEIRKVAPNNTSKTCSKCGHLNNYFNFEYRKKNKFPHFKCEKCNFKENADYNAALNISNPKLKSTKEEPSGGSSGGSSGSETPGTSESATPESSGGSSGGSMVEFSDEYWMRHALTLAKRARDEGEVPVGAVLVLNNRVIGEGWNRAIGLHDPTAHAEIMALRQGGQVLQNYRLIDATLYVTFEPCVMCAGAMIHSRIKRVVFGWRNSKRGAAGSLMNVLNHPGMNHRVEITEGVLADECAALLSDFFRMRRQQKKAQKKKRPAATKKAGQAKKKK

SEQ ID NO: 311 - protein, 736 aa, synthetic construct
  REGION 1..736: note = d12f1(D326A)-eTadA5
MAKNTITKTLKLRIVRPYNSAEVEKIVADEKNNREKIALEKNKDKVKEACSKHLKVAAYCTTQVERNACLFCKARKLDDKFYQKLRGQFPDAVFWQEISEIFRQLQKQAAEIYNQSLIELYYEIFIKGKGIANASSVEHYLSDVCYTRAAELFKNAAIASGLRSKIKSNFRLKELKNMKSGLPTTKSDNFPIPLVKQKGGQYTGFEISNHNSDFIIKIPFGRWQVKKEIDKYRPWEKFDFEQVQKSPKPISLLLSTQRRKRNKGWSKDEGTEAEIKKVMNGDYQTSYIEVKRGSKIGEKSAWMLNLSIDVPKIDKGVDPSIIGGIAVGVKSPLVCAINNAFSRYSISDNDLFHFNKKMFARRRILLKKNRHKRAGHGAKNKLKPITILTEKSERFRKKLIERWACEIADFFIKNKVGTVQMENLESMKRKEDSYFNIRLRGFWPYAEMQNKIEFKLKQYGIEIRKVAPNNTSKTCSKCGHLNNYFNFEYRKKNKFPHFKCEKCNFKENADYNAALNISNPKLKSTKEEPSGGSSGGSSGSETPGTSESATPESSGGSSGGSMVEFSDEYWMRHALTLAKRARDEGEVPVGAVLVLNNQVIGEGWNRSISLHDPTAHAEIMALRQGGQVLQNYRLIDCTLYVTFEPCVMCAGAMIHSRIKRVVFGWRNPKRGAAGSLMNVLNHPGMNHRIEITEGVLADECAAMLSDFFRMRRQQKKAQKKKRPAATKKAGQAKKKK

SEQ ID NO: 312 - protein, 736 aa, synthetic construct
  REGION 1..736: note = d12f1(D326A)-eTadA6
MAKNTITKTLKLRIVRPYNSAEVEKIVADEKNNREKIALEKNKDKVKEACSKHLKVAAYCTTQVERNACLFCKARKLDDKFYQKLRGQFPDAVFWQEISEIFRQLQKQAAEIYNQSLIELYYEIFIKGKGIANASSVEHYLSDVCYTRAAELFKNAAIASGLRSKIKSNFRLKELKNMKSGLPTTKSDNFPIPLVKQKGGQYTGFEISNHNSDFIIKIPFGRWQVKKEIDKYRPWEKFDFEQVQKSPKPISLLLSTQRRKRNKGWSKDEGTEAEIKKVMNGDYQTSYIEVKRGSKIGEKSAWMLNLSIDVPKIDKGVDPSIIGGIAVGVKSPLVCAINNAFSRYSISDNDLFHFNKKMFARRRILLKKNRHKRAGHGAKNKLKPITILTEKSERFRKKLIERWACEIADFFIKNKVGTVQMENLESMKRKEDSYFNIRLRGFWPYAEMQNKIEFKLKQYGIEIRKVAPNNTSKTCSKCGHLNNYFNFEYRKKNKFPHFKCEKCNFKENADYNAALNISNPKLKSTKEEPSGGSSGGSSGSETPGTSESATPESSGGSSGGSMVEFSDEYWMRHALTLAKRARDEGEVPVGAVLVLNNQVIGEGWNRSITHHDPTAHAEIMALRQGGQVLQNYRLIDCTLYVTFEPCVMCAGAMIHARIKRVVFGWRNPKRGAAGSVMNVLNHPGMNHRIEITEGVLADECAAMLSDFFRMRRQQKKAQKKKRPAATKKAGQAKKKK

SEQ ID NO: 313 - protein, 943 aa, synthetic construct
  REGION 1..943: note = d12f1(D326A)-TadA-eTadA3
MAKNTITKTLKLRIVRPYNSAEVEKIVADEKNNREKIALEKNKDKVKEACSKHLKVAAYCTTQVERNACLFCKARKLDDKFYQKLRGQFPDAVFWQEISEIFRQLQKQAAEIYNQSLIELYYEIFIKGKGIANASSVEHYLSDVCYTRAAELFKNAAIASGLRSKIKSNFRLKELKNMKSGLPTTKSDNFPIPLVKQKGGQYTGFEISNHNSDFIIKIPFGRWQVKKEIDKYRPWEKFDFEQVQKSPKPISLLLSTQRRKRNKGWSKDEGTEAEIKKVMNGDYQTSYIEVKRGSKIGEKSAWMLNLSIDVPKIDKGVDPSIIGGIAVGVKSPLVCAINNAFSRYSISDNDLFHFNKKMFARRRILLKKNRHKRAGHGAKNKLKPITILTEKSERFRKKLIERWACEIADFFIKNKVGTVQMENLESMKRKEDSYFNIRLRGFWPYAEMQNKIEFKLKQYGIEIRKVAPNNTSKTCSKCGHLNNYFNFEYRKKNKFPHFKCEKCNFKENADYNAALNISNPKLKSTKEEPSGGSSGGSSGSETPGTSESATPESSGGSSGGSMSEVEFSHEYWMRHALTLAKRAWDEREVPVGAVLVHNNRVIGEGWNRPIGRHDPTAHAEIMALRQGGLVMQNYRLIDATLYVTLEPCVMCAGAMIHSRIGRVVFGARDAKTGAAGSLMDVLHHPGMNHRVEITEGILADECAALLSDFFRMRRQEIKAQKKAQSSTDSGGSSGGSSGSETPGTSESATPESSGGSSGGSMSEVEFSHEYWMRHALTLAKRARDEREVPVGAVLVLNNRVIGEGWNRAIGLHDPTAHAEIMALRQGGLVMQNYRLIDATLYVTFEPCVMCAGAMIHSRIGRVVFGWRQSKRGAAGSLMNVLNYPGMNHRVEITEGILADECAALLCDFYRMPRQVFNAQKKAQSSINKRPAATKKAGQAKKKK

SEQ ID NO: 314 - protein, 971 aa, synthetic construct
  REGION 1..971: note = dtnpb(D354)-dTadA-eTadA1
MGEKSSRRRRNGKSGAWTAAITSCVGGKMAKNTITKTLKLRIVRPYNSAEVEKIVADEKNNREKIALEKNKDKVKEACSKHLKVAAYCTTQVERNACLFCKARKLDDKFYQKLRGQFPDAVFWQEISEIFRQLQKQAAEIYNQSLIELYYEIFIKGKGIANASSVEHYLSDVCYTRAAELFKNAAIASGLRSKIKSNFRLKELKNMKSGLPTTKSDNFPIPLVKQKGGQYTGFEISNHNSDFIIKIPFGRWQVKKEIDKYRPWEKFDFEQVQKSPKPISLLLSTQRRKRNKGWSKDEGTEAEIKKVMNGDYQTSYIEVKRGSKIGEKSAWMLNLSIDVPKIDKGVDPSIIGGIAVGVKSPLVCAINNAFSRYSISDNDLFHFNKKMFARRRILLKKNRHKRAGHGAKNKLKPITILTEKSERFRKKLIERWACEIADFFIKNKVGTVQMENLESMKRKEDSYFNIRLRGFWPYAEMQNKIEFKLKQYGIEIRKVAPNNTSKTCSKCGHLNNYFNFEYRKKNKFPHFKCEKCNFKENADYNAALNISNPKLKSTKEEPSGGSSGGSSGSETPGTSESATPESSGGSSGGSMSEVEFSHEYWMRHALTLAKRAWDEREVPVGAVLVHNNRVIGEGWNRPIGRHDPTAHAAIMALRQGGLVMQNYRLIDATLYVTLEPCVMCAGAMIHSRIGRVVFGARDAKTGAAGSLMDVLHHPGMNHRVEITEGILADECAALLSDFFRMRRQEIKAQKKAQSSTDSGGSSGGSSGSETPGTSESATPESSGGSSGGSMSEVEFSHEYWMRHALTLAKRARDEREVPVGAVLVLNNRVIGEGWNRAIGLHDPTAHAEIMALRQGGLVMQNYRLIDATLYVTFEPCVMCAGAMIHSRIGRVVFGVRNAKTGAAGSLMDVLHYPGMNHRVEITEGILADECAALLCYFFRMPRQVFNAQKKAQSSTDKRPAATKKAGQAKKKK

SEQ ID NO: 315 - protein, 971 aa, synthetic construct
  REGION 1..971: note = dtnpb(D354)-TadA-deTadA1
MGEKSSRRRRNGKSGAWTAAITSCVGGKMAKNTITKTLKLRIVRPYNSAEVEKIVADEKNNREKIALEKNKDKVKEACSKHLKVAAYCTTQVERNACLFCKARKLDDKFYQKLRGQFPDAVFWQEISEIFRQLQKQAAEIYNQSLIELYYEIFIKGKGIANASSVEHYLSDVCYTRAAELFKNAAIASGLRSKIKSNFRLKELKNMKSGLPTTKSDNFPIPLVKQKGGQYTGFEISNHNSDFIIKIPFGRWQVKKEIDKYRPWEKFDFEQVQKSPKPISLLLSTQRRKRNKGWSKDEGTEAEIKKVMNGDYQTSYIEVKRGSKIGEKSAWMLNLSIDVPKIDKGVDPSIIGGIAVGVKSPLVCAINNAFSRYSISDNDLFHFNKKMFARRRILLKKNRHKRAGHGAKNKLKPITILTEKSERFRKKLIERWACEIADFFIKNKVGTVQMENLESMKRKEDSYFNIRLRGFWPYAEMQNKIEFKLKQYGIEIRKVAPNNTSKTCSKCGHLNNYFNFEYRKKNKFPHFKCEKCNFKENADYNAALNISNPKLKSTKEEPSGGSSGGSSGSETPGTSESATPESSGGSSGGSMSEVEFSHEYWMRHALTLAKRAWDEREVPVGAVLVHNNRVIGEGWNRPIGRHDPTAHAEIMALRQGGLVMQNYRLIDATLYVTLEPCVMCAGAMIHSRIGRVVFGARDAKTGAAGSLMDVLHHPGMNHRVEITEGILADECAALLSDFFRMRRQEIKAQKKAQSSTDSGGSSGGSSGSETPGTSESATPESSGGSSGGSMSEVEFSHEYWMRHALTLAKRARDEREVPVGAVLVLNNRVIGEGWNRAIGLHDPTAHAAIMALRQGGLVMQNYRLIDATLYVTFEPCVMCAGAMIHSRIGRVVFGVRNAKTGAAGSLMDVLHYPGMNHRVEITEGILADECAALLCYFFRMPRQVFNAQKKAQSSTDKRPAATKKAGQAKKKK

SEQ ID NO: 316 - protein, 971 aa, synthetic construct
  REGION 1..971: note = dtnpb(D354)-TadA-eTadA2
MGEKSSRRRRNGKSGAWTAAITSCVGGKMAKNTITKTLKLRIVRPYNSAEVEKIVADEKNNREKIALEKNKDKVKEACSKHLKVAAYCTTQVERNACLFCKARKLDDKFYQKLRGQFPDAVFWQEISEIFRQLQKQAAEIYNQSLIELYYEIFIKGKGIANASSVEHYLSDVCYTRAAELFKNAAIASGLRSKIKSNFRLKELKNMKSGLPTTKSDNFPIPLVKQKGGQYTGFEISNHNSDFIIKIPFGRWQVKKEIDKYRPWEKFDFEQVQKSPKPISLLLSTQRRKRNKGWSKDEGTEAEIKKVMNGDYQTSYIEVKRGSKIGEKSAWMLNLSIDVPKIDKGVDPSIIGGIAVGVKSPLVCAINNAFSRYSISDNDLFHFNKKMFARRRILLKKNRHKRAGHGAKNKLKPITILTEKSERFRKKLIERWACEIADFFIKNKVGTVQMENLESMKRKEDSYFNIRLRGFWPYAEMQNKIEFKLKQYGIEIRKVAPNNTSKTCSKCGHLNNYFNFEYRKKNKFPHFKCEKCNFKENADYNAALNISNPKLKSTKEEPSGGSSGGSSGSETPGTSESATPESSGGSSGGSMSEVEFSHEYWMRHALTLAKRAWDEREVPVGAVLVHNNRVIGEGWNRPIGRHDPTAHAEIMALRQGGLVMQNYRLIDATLYVTLEPCVMCAGAMIHSRIGRVVFGARDAKTGAAGSLMDVLHHPGMNHRVEITEGILADECAALLSDFFRMRRQEIKAQKKAQSSTDSGGSSGGSSGSETPGTSESATPESSGGSSGGSMSEVEFSHEYWMRHALTLAKRARDEREVPVGAVLVLNNRVIGEGWNRAIGLHDPTAHAEIMALRQGGLVMQNYRLIDATLYVTFEPCVMCAGAMIHSRIGRVVFGWRNSKRGAAGSLMNVLNYPGMNHRVEITEGILADECAALLCDFYRMPRQVFNAQKKAQSSINKRPAATKKAGQAKKKK

SEQ ID NO: 317 - protein, 772 aa, synthetic construct
  REGION 1..772: note = dtnpb(D354)-eTadA2
MGEKSSRRRRNGKSGAWTAAITSCVGGKMAKNTITKTLKLRIVRPYNSAEVEKIVADEKNNREKIALEKNKDKVKEACSKHLKVAAYCTTQVERNACLFCKARKLDDKFYQKLRGQFPDAVFWQEISEIFRQLQKQAAEIYNQSLIELYYEIFIKGKGIANASSVEHYLSDVCYTRAAELFKNAAIASGLRSKIKSNFRLKELKNMKSGLPTTKSDNFPIPLVKQKGGQYTGFEISNHNSDFIIKIPFGRWQVKKEIDKYRPWEKFDFEQVQKSPKPISLLLSTQRRKRNKGWSKDEGTEAEIKKVMNGDYQTSYIEVKRGSKIGEKSAWMLNLSIDVPKIDKGVDPSIIGGIAVGVKSPLVCAINNAFSRYSISDNDLFHFNKKMFARRRILLKKNRHKRAGHGAKNKLKPITILTEKSERFRKKLIERWACEIADFFIKNKVGTVQMENLESMKRKEDSYFNIRLRGFWPYAEMQNKIEFKLKQYGIEIRKVAPNNTSKTCSKCGHLNNYFNFEYRKKNKFPHFKCEKCNFKENADYNAALNISNPKLKSTKEEPSGGSSGGSSGSETPGTSESATPESSGGSSGGSMSEVEFSHEYWMRHALTLAKRARDEREVPVGAVLVLNNRVIGEGWNRAIGLHDPTAHAEIMALRQGGLVMQNYRLIDATLYVTFEPCVMCAGAMIHSRIGRVVFGWRNSKRGAAGSLMNVLNYPGMNHRVEITEGILADECAALLCDFYRMPRQVFNAQKKAQSSINKRPAATKKAGQAKKKK

SEQ ID NO: 318 - protein, 764 aa, synthetic construct
  REGION 1..764: note = dtnpb(D354)-eTadA4
MGEKSSRRRRNGKSGAWTAAITSCVGGKMAKNTITKTLKLRIVRPYNSAEVEKIVADEKNNREKIALEKNKDKVKEACSKHLKVAAYCTTQVERNACLFCKARKLDDKFYQKLRGQFPDAVFWQEISEIFRQLQKQAAEIYNQSLIELYYEIFIKGKGIANASSVEHYLSDVCYTRAAELFKNAAIASGLRSKIKSNFRLKELKNMKSGLPTTKSDNFPIPLVKQKGGQYTGFEISNHNSDFIIKIPFGRWQVKKEIDKYRPWEKFDFEQVQKSPKPISLLLSTQRRKRNKGWSKDEGTEAEIKKVMNGDYQTSYIEVKRGSKIGEKSAWMLNLSIDVPKIDKGVDPSIIGGIAVGVKSPLVCAINNAFSRYSISDNDLFHFNKKMFARRRILLKKNRHKRAGHGAKNKLKPITILTEKSERFRKKLIERWACEIADFFIKNKVGTVQMENLESMKRKEDSYFNIRLRGFWPYAEMQNKIEFKLKQYGIEIRKVAPNNTSKTCSKCGHLNNYFNFEYRKKNKFPHFKCEKCNFKENADYNAALNISNPKLKSTKEEPSGGSSGGSSGSETPGTSESATPESSGGSSGGSMVEFSDEYWMRHALTLAKRARDEGEVPVGAVLVLNNRVIGEGWNRAIGLHDPTAHAEIMALRQGGQVLQNYRLIDATLYVTFEPCVMCAGAMIHSRIKRVVFGWRNSKRGAAGSLMNVLNHPGMNHRVEITEGVLADECAALLSDFFRMRRQQKKAQKKKRPAATKKAGQAKKKK

SEQ ID NO: 319 - protein, 764 aa, synthetic construct; identical to SEQ ID NO: 318
  REGION 1..764: note = dtnpb(D354)-eTadA5

SEQ ID NO: 320 - protein, 764 aa, synthetic construct
  REGION 1..764: note = dtnpb(D354)-eTadA6
MGEKSSRRRRNGKSGAWTAAITSCVGGKMAKNTITKTLKLRIVRPYNSAEVEKIVADEKNNREKIALEKNKDKVKEACSKHLKVAAYCTTQVERNACLFCKARKLDDKFYQKLRGQFPDAVFWQEISEIFRQLQKQAAEIYNQSLIELYYEIFIKGKGIANASSVEHYLSDVCYTRAAELFKNAAIASGLRSKIKSNFRLKELKNMKSGLPTTKSDNFPIPLVKQKGGQYTGFEISNHNSDFIIKIPFGRWQVKKEIDKYRPWEKFDFEQVQKSPKPISLLLSTQRRKRNKGWSKDEGTEAEIKKVMNGDYQTSYIEVKRGSKIGEKSAWMLNLSIDVPKIDKGVDPSIIGGIAVGVKSPLVCAINNAFSRYSISDNDLFHFNKKMFARRRILLKKNRHKRAGHGAKNKLKPITILTEKSERFRKKLIERWACEIADFFIKNKVGTVQMENLESMKRKEDSYFNIRLRGFWPYAEMQNKIEFKLKQYGIEIRKVAPNNTSKTCSKCGHLNNYFNFEYRKKNKFPHFKCEKCNFKENADYNAALNISNPKLKSTKEEPSGGSSGGSSGSETPGTSESATPESSGGSSGGSMVEFSDEYWMRHALTLAKRARDEGEVPVGAVLVLNNQVIGEGWNRSITHHDPTAHAEIMALRQGGQVLQNYRLIDCTLYVTFEPCVMCAGAMIHARIKRVVFGWRNPKRGAAGSVMNVLNHPGMNHRIEITEGVLADECAAMLSDFFRMRRQQKKAQKKKRPAATKKAGQAKKKK

SEQ ID NO: 321 - protein, 971 aa, synthetic construct; identical to SEQ ID NO: 291
  REGION 1..971: note = dtnpb(D354A)-TadA-eTadA1

SEQ ID NO: 322 - protein, 971 aa, synthetic construct
  REGION 1..971: note = d28ext(D354A)-TadA-eTadA1
MAGGPGAGSAAPVSSTSSLPLAALNMRVMAKNTITKTLKLRIVRPYNSAEVEKIVADEKNNREKIALEKNKDKVKEACSKHLKVAAYCTTQVERNACLFCKARKLDDKFYQKLRGQFPDAVFWQEISEIFRQLQKQAAEIYNQSLIELYYEIFIKGKGIANASSVEHYLSDVCYTRAAELFKNAAIASGLRSKIKSNFRLKELKNMKSGLPTTKSDNFPIPLVKQKGGQYTGFEISNHNSDFIIKIPFGRWQVKKEIDKYRPWEKFDFEQVQKSPKPISLLLSTQRRKRNKGWSKDEGTEAEIKKVMNGDYQTSYIEVKRGSKIGEKSAWMLNLSIDVPKIDKGVDPSIIGGIAVGVKSPLVCAINNAFSRYSISDNDLFHFNKKMFARRRILLKKNRHKRAGHGAKNKLKPITILTEKSERFRKKLIERWACEIADFFIKNKVGTVQMENLESMKRKEDSYFNIRLRGFWPYAEMQNKIEFKLKQYGIEIRKVAPNNTSKTCSKCGHLNNYFNFEYRKKNKFPHFKCEKCNFKENADYNAALNISNPKLKSTKEEPSGGSSGGSSGSETPGTSESATPESSGGSSGGSMSEVEFSHEYWMRHALTLAKRAWDEREVPVGAVLVHNNRVIGEGWNRPIGRHDPTAHAEIMALRQGGLVMQNYRLIDATLYVTLEPCVMCAGAMIHSRIGRVVFGARDAKTGAAGSLMDVLHHPGMNHRVEITEGILADECAALLSDFFRMRRQEIKAQKKAQSSTDSGGSSGGSSGSETPGTSESATPESSGGSSGGSMSEVEFSHEYWMRHALTLAKRARDEREVPVGAVLVLNNRVIGEGWNRAIGLHDPTAHAEIMALRQGGLVMQNYRLIDATLYVTFEPCVMCAGAMIHSRIGRVVFGVRNAKTGAAGSLMDVLHYPGMNHRVEITEGILADECAALLCYFFRMPRQVFNAQKKAQSSTDKRPAATKKAGQAKKKK

SEQ ID NO: 323 - protein, 971 aa, synthetic construct; identical to SEQ ID NO: 322
  REGION 1..971: note = d26ext(D352A)-TadA-eTadA1

SEQ ID NO: 324 - protein, 969 aa, synthetic construct
  REGION 1..969: note = dx(D352A)-TadA-eTadA1
MEKRINKIRKKLSADNATKPVSRSGPMAKNTITKTLKLRIVRPYNSAEVEKIVADEKNNREKIALEKNKDKVKEACSKHLKVAAYCTTQVERNACLFCKARKLDDKFYQKLRGQFPDAVFWQEISEIFRQLQKQAAEIYNQSLIELYYEIFIKGKGIANASSVEHYLSDVCYTRAAELFKNAAIASGLRSKIKSNFRLKELKNMKSGLPTTKSDNFPIPLVKQKGGQYTGFEISNHNSDFIIKIPFGRWQVKKEIDKYRPWEKFDFEQVQKSPKPISLLLSTQRRKRNKGWSKDEGTEAEIKKVMNGDYQTSYIEVKRGSKIGEKSAWMLNLSIDVPKIDKGVDPSIIGGIAVGVKSPLVCAINNAFSRYSISDNDLFHFNKKMFARRRILLKKNRHKRAGHGAKNKLKPITILTEKSERFRKKLIERWACEIADFFIKNKVGTVQMENLESMKRKEDSYFNIRLRGFWPYAEMQNKIEFKLKQYGIEIRKVAPNNTSKTCSKCGHLNNYFNFEYRKKNKFPHFKCEKCNFKENADYNAALNISNPKLKSTKEEPSGGSSGGSSGSETPGTSESATPESSGGSSGGSMSEVEFSHEYWMRHALTLAKRAWDEREVPVGAVLVHNNRVIGEGWNRPIGRHDPTAHAEIMALRQGGLVMQNYRLIDATLYVTLEPCVMCAGAMIHSRIGRVVFGARDAKTGAAGSLMDVLHHPGMNHRVEITEGILADECAALLSDFFRMRRQEIKAQKKAQSSTDSGGSSGGSSGSETPGTSESATPESSGGSSGGSMSEVEFSHEYWMRHALTLAKRARDEREVPVGAVLVLNNRVIGEGWNRAIGLHDPTAHAEIMALRQGGLVMQNYRLIDATLYVTFEPCVMCAGAMIHSRIGRVVFGVRNAKTGAAGSLMDVLHYPGMNHRVEITEGILADECAALLCYFFRMPRQVFNAQKKAQSSTDKRPAATKKAGQAKKKK

SEQ ID NO: 325 - protein, 1235 aa, synthetic construct
  REGION 1..1235: note = APOBEC1-TadA-d12f1(D326A)-UGI
MSSETGPVAVDPTLRRRIEPHEFEVFFDPRELRKETCLLYEINWGGRHSIWRHTSQNTNKHVEVNFIEKFTTERYFCPNTRCSITWFLSWSPCGECSRAITEFLSRYPHVTLFIYIARLYHHADPRNRQGLRDLISSGVTIQIMTEQESGYCWRNFVNYSPSNEAHWPRYPHLWVRLYVLELYCIILGLPPCLNILRRKQPQLTFFTIALQSCHYQRLPPHILWATGLKSGGSSGGSSGSETPGTSESATPESSGGSSGGSMSEVEFSHEYWMRHALTLAKRAWDEREVPVGAVLVHNNRVIGEGWNRPIGRHDPTAHAEIMALRQGGLVMQNYRLIDATLYVTLEPCVMCAGAMIHSRIGRVVFGARDAKTGAAGSLMDVLHHPGMNHRVEITEGILADECAALLSDFFRMRRQEIKAQKKAQSSTDSGGSSGGSSGSETPGTSESATPESSGGSSGGSMAKNTITKTLKLRIVRPYNSAEVEKIVADEKNNREKIALEKNKDKVKEACSKHLKVAAYCTTQVERNACLFCKARKLDDKFYQKLRGQFPDAVFWQEISEIFRQLQKQAAEIYNQSLIELYYEIFIKGKGIANASSVEHYLSDVCYTRAAELFKNAAIASGLRSKIKSNFRLKELKNMKSGLPTTKSDNFPIPLVKQKGGQYTGFEISNHNSDFIIKIPFGRWQVKKEIDKYRPWEKFDFEQVQKSPKPISLLLSTQRRKRNKGWSKDEGTEAEIKKVMNGDYQTSYIEVKRGSKIGEKSAWMLNLSIDVPKIDKGVDPSIIGGIAVGVKSPLVCAINNAFSRYSISDNDLFHFNKKMFARRRILLKKNRHKRAGHGAKNKLKPITILTEKSERFRKKLIERWACEIADFFIKNKVGTVQMENLESMKRKEDSYFNIRLRGFWPYAEMQNKIEFKLKQYGIEIRKVAPNNTSKTCSKCGHLNNYFNFEYRKKNKFPHFKCEKCNFKENADYNAALNISNPKLKSTKEEPSGGSSGGSSGSETPGTSESATPESSGGSSGGSTNLSDIIEKETGKQLVIQESILMLPEEVEEVIGNKPESDILVHTAYDESTDENVMLLTSDAPEYKPWALVIQDSNGENKIKMLSGGSSGGSSGSETPGTSESATPESSGGSSGGSTNLSDIIEKETGKQLVIQESILMLPEEVEEVIGNKPESDILVHTAYDESTDENVMLLTSDAPEYKPWALVIQDSNGENKIKMLKRPAATKKAGQAKKKK

SEQ ID NO: 326 - protein, 1235 aa, synthetic construct
  REGION 1..1235: note = APOBEC1-eTadA-d12f1(D326A)-UGI
MSSETGPVAVDPTLRRRIEPHEFEVFFDPRELRKETCLLYEINWGGRHSIWRHTSQNTNKHVEVNFIEKFTTERYFCPNTRCSITWFLSWSPCGECSRAITEFLSRYPHVTLFIYIARLYHHADPRNRQGLRDLISSGVTIQIMTEQESGYCWRNFVNYSPSNEAHWPRYPHLWVRLYVLELYCIILGLPPCLNILRRKQPQLTFFTIALQSCHYQRLPPHILWATGLKSGGSSGGSSGSETPGTSESATPESSGGSSGGSMSEVEFSHEYWMRHALTLAKRARDEREVPVGAVLVLNNRVIGEGWNRAIGLHDPTAHAEIMALRQGGLVMQNYRLIDATLYVTFEPCVMCAGAMIHSRIGRVVFGVRNAKTGAAGSLMDVLHYPGMNHRVEITEGILADECAALLCYFFRMPRQVFNAQKKAQSSTDSGGSSGGSSGSETPGTSESATPESSGGSSGGSMAKNTITKTLKLRIVRPYNSAEVEKIVADEKNNREKIALEKNKDKVKEACSKHLKVAAYCTTQVERNACLFCKARKLDDKFYQKLRGQFPDAVFWQEISEIFRQLQKQAAEIYNQSLIELYYEIFIKGKGIANASSVEHYLSDVCYTRAAELFKNAAIASGLRSKIKSNFRLKELKNMKSGLPTTKSDNFPIPLVKQKGGQYTGFEISNHNSDFIIKIPFGRWQVKKEIDKYRPWEKFDFEQVQKSPKPISLLLSTQRRKRNKGWSKDEGTEAEIKKVMNGDYQTSYIEVKRGSKIGEKSAWMLNLSIDVPKIDKGVDPSIIGGIAVGVKSPLVCAINNAFSRYSISDNDLFHFNKKMFARRRILLKKNRHKRAGHGAKNKLKPITILTEKSERFRKKLIERWACEIADFFIKNKVGTVQMENLESMKRKEDSYFNIRLRGFWPYAEMQNKIEFKLKQYGIEIRKVAPNNTSKTCSKCGHLNNYFNFEYRKKNKFPHFKCEKCNFKENADYNAALNISNPKLKSTKEEPSGGSSGGSSGSETPGTSESATPESSGGSSGGSTNLSDIIEKETGKQLVIQESILMLPEEVEEVIGNKPESDILVHTAYDESTDENVMLLTSDAPEYKPWALVIQDSNGENKIKMLSGGSSGGSSGSETPGTSESATPESSGGSSGGSTNLSDIIEKETGKQLVIQESILMLPEEVEEVIGNKPESDILVHTAYDESTDENVMLLTSDAPEYKPWALVIQDSNGENKIKMLKRPAATKKAGQAKKKK

SEQ ID NO: 327 - protein, 1187 aa, synthetic construct
  REGION 1..1187: note = UGI-d12f1(D326A)-eTadA-APOBEC1
TNLSDIIEKETGKQLVIQESILMLPEEVEEVIGNKPESDILVHTAYDESTDENVMLLTSDAPEYKPWALVIQDSNGENKIKMLSGGSSGGSSGSETPGTSESATPESSGGSSGGSTNLSDIIEKETGKQLVIQESILMLPEEVEEVIGNKPESDILVHTAYDESTDENVMLLTSDAPEYKPWALVIQDSNGENKIKMLSGGSSGGSSGSETPGTSESATPESSGGSSGGSMAKNTITKTLKLRIVRPYNSAEVEKIVADEKNNREKIALEKNKDKVKEACSKHLKVAAYCTTQVERNACLFCKARKLDDKFYQKLRGQFPDAVFWQEISEIFRQLQKQAAEIYNQSLIELYYEIFIKGKGIANASSVEHYLSDVCYTRAAELFKNAAIASGLRSKIKSNFRLKELKNMKSGLPTTKSDNFPIPLVKQKGGQYTGFEISNHNSDFIIKIPFGRWQVKKEIDKYRPWEKFDFEQVQKSPKPISLLLSTQRRKRNKGWSKDEGTEAEIKKVMNGDYQTSYIEVKRGSKIGEKSAWMLNLSIDVPKIDKGVDPSIIGGIAVGVKSPLVCAINNAFSRYSISDNDLFHFNKKMFARRRILLKKNRHKRAGHGAKNKLKPITILTEKSERFRKKLIERWACEIADFFIKNKVGTVQMENLESMKRKEDSYFNIRLRGFWPYAEMQNKIEFKLKQYGIEIRKVAPNNTSKTCSKCGHLNNYFNFEYRKKNKFPHFKCEKCNFKENADYNAALNISNPKLKSTKEEPSGGSSGGSSGSETPGTSESATPESSGGSSGGSMSEVEFSHEYWMRHALTLAKRARDEREVPVGAVLVLNNRVIGEGWNRAIGLHDPTAHAEIMALRQGGLVMQNYRLIDATLYVTFEPCVMCAGAMIHSRIGRVVFGVRNAKTGAAGSLMDVLHYPGMNHRVEITEGILADECAALLCYFFRMPRQVFNAQKKAQSSTDMSSETGPVAVDPTLRRRIEPHEFEVFFDPRELRKETCLLYEINWGGRHSIWRHTSQNTNKHVEVNFIEKFTTERYFCPNTRCSITWFLSWSPCGECSRAITEFLSRYPHVTLFIYIARLYHHADPRNRQGLRDLISSGVTIQIMTEQESGYCWRNFVNYSPSNEAHWPRYPHLWVRLYVLELYCIILGLPPCLNILRRKQPQLTFFTIALQSCHYQRLPPHILWATGLK

SEQ ID NO: 328 - protein, 1219 aa, synthetic construct
  REGION 1..1219: note = UGI-d12f1(D326A)-TadA-APOBEC1
TNLSDIIEKETGKQLVIQESILMLPEEVEEVIGNKPESDILVHTAYDESTDENVMLLTSDAPEYKPWALVIQDSNGENKIKMLSGGSSGGSSGSETPGTSESATPESSGGSSGGSTNLSDIIEKETGKQLVIQESILMLPEEVEEVIGNKPESDILVHTAYDESTDENVMLLTSDAPEYKPWALVIQDSNGENKIKMLSGGSSGGSSGSETPGTSESATPESSGGSSGGSMAKNTITKTLKLRIVRPYNSAEVEKIVADEKNNREKIALEKNKDKVKEACSKHLKVAAYCTTQVERNACLFCKARKLDDKFYQKLRGQFPDAVFWQEISEIFRQLQKQAAEIYNQSLIELYYEIFIKGKGIANASSVEHYLSDVCYTRAAELFKNAAIASGLRSKIKSNFRLKELKNMKSGLPTTKSDNFPIPLVKQKGGQYTGFEISNHNSDFIIKIPFGRWQVKKEIDKYRPWEKFDFEQVQKSPKPISLLLSTQRRKRNKGWSKDEGTEAEIKKVMNGDYQTSYIEVKRGSKIGEKSAWMLNLSIDVPKIDKGVDPSIIGGIAVGVKSPLVCAINNAFSRYSISDNDLFHFNKKMFARRRILLKKNRHKRAGHGAKNKLKPITILTEKSERFRKKLIERWACEIADFFIKNKVGTVQMENLESMKRKEDSYFNIRLRGFWPYAEMQNKIEFKLKQYGIEIRKVAPNNTSKTCSKCGHLNNYFNFEYRKKNKFPHFKCEKCNFKENADYNAALNISNPKLKSTKEEPSGGSSGGSSGSETPGTSESATPESSGGSSGGSMSEVEFSHEYWMRHALTLAKRAWDEREVPVGAVLVHNNRVIGEGWNRPIGRHDPTAHAEIMALRQGGLVMQNYRLIDATLYVTLEPCVMCAGAMIHSRIGRVVFGARDAKTGAAGSLMDVLHHPGMNHRVEITEGILADECAALLSDFFRMRRQEIKAQKKAQSSTDSGGSSGGSSGSETPGTSESATPESSGGSSGGSMSSETGPVAVDPTLRRRIEPHEFEVFFDPRELRKETCLLYEINWGGRHSIWRHTSQNTNKHVEVNFIEKFTTERYFCPNTRCSITWFLSWSPCGECSRAITEFLSRYPHVTLFIYIARLYHHADPRNRQGLRDLISSGVTIQIMTEQESGYCWRNFVNYSPSNEAHWPRYPHLWVRLYVLELYCIILGLPPCLNILRRKQPQLTFFTIALQSCHYQRLPPHILWATGLK

SEQ ID NO: 329 - protein, 51 aa, Homo sapiens
MDALDDFDLDMLGSDALDDFDLDMLGSDALDDFDLDMLGSDALDDFDLDML

SEQ ID NO: 330 - protein, 65 aa, Homo sapiens
RTLVTFKDVFVDFTREEWKLLDTAQQIVYRNVMLENYKNLVSLGYQLTKPDVILRLEKGEEPWLV

SEQ ID NO: 331 - protein, 286 aa, Homo sapiens
VQVKRVLEKSPGKLLVKMPFQASPGGKGEGGGATTSAQVMVIKRPGRKRKAEADPQAIPKKRGRKPGSVVAAAAAEAKKKAVKESSIRSVQETVLPIKKRKTRETVSIEVKEVVKPLLVSTLGEKSGKGLKTCKSPGRKSKESSPKGRSSSASSPPKKEHHHHHHHAESPKAPMPLLPPPPPPEPQSSEDPISPPEPQDLSSSICKEEKMPRAGSLESDGCPKEPAKTQPMVAAAATTTTTTTTTVAEKYKHRGEGERKDIVSSSMPRPNREEPVDSRTPVTERVS

SEQ ID NO: 332 - protein, 311 aa, Homo sapiens
PSRLQMFFANNHDQEFDPPKVYPPVPAEKRKPIRVLSLFDGIATGLLVLKDLGIQVDRYIASEVCEDSITVGMVRHQGKIMYVGDVRSVTQKHIQEWGPFDLVIGGSPCNDLSIVNPARKGLYEGTGRLFFEFYRLLHDARPKEGDDRPFFWLFENVVAMGVSDKRDISRFLESNPVMIDAKEVSAAHRARYFWGNLPGMNRPLASTVNDKLELQECLEHGRIAKFSKVRTITTRSNSIKQGKDQHFPVFMNEKEDILWCTEMERVFGFPVHYTDVSNMSRLARQRLLGRSWSVPVIRHLFAPLKEYFACV

SEQ ID NO: 333 - protein, 428 aa, Homo sapiens
MAKTVAYFYDPDVGNFHYGAGHPMKPHRLALTHSLVLHYGLYKKMIVFKPYQASQHDMCRFHSEDYIDFLQRVSPTNMQGFTKSLNAFNVGDDCPVFPGLFEFCSRYTGASLQGATQLNNKICDIAINWAGGLHHAKKFEASGFCYVNDIVIGILELLKYHPRVLYIDIDIHHGDGVQEAFYLTDRVMTVSFHKYGNYFFPGTGDMYEVGAESGRYYCLNVPLRDGIDDQSYKHLFQPVINQVVDFYQPTCIVLQCGADSLGCDRLGCFNLSIRGHGECVEYVKSFNIPLLVLGGGGYTVRNVARCWTYETSLLVEEAISEELPYSEYFEYFAPDFTLHPDVSTRIENQNSRQYLDQIRQTIFENLKMLNHAPSVQIHDVPADLLTYDRTDEADAEERGPEENYSRPEAPNEFYDGDHDNDKESDVEI

SEQ ID NO: 334 - DNA, 20 bp, synthetic construct
  misc_feature 1..20: note = target gene's protospacer sequence
  source 1..20: mol_type = other DNA
cacacacacagtgggctacc

SEQ ID NO: 335 - DNA, 20 bp, synthetic construct
  misc_feature 1..20: note = target gene's protospacer sequence
  source 1..20: mol_type = other DNA
catccccaggacacacacac

SEQ ID NO: 336 - DNA, 20 bp, synthetic construct
  misc_feature 1..20: note = target gene's protospacer sequence
  source 1..20: mol_type = other DNA
caaagacactcaccctgttg

SEQ ID NO: 337 - DNA, 20 bp, synthetic construct
  misc_feature 1..20: note = target gene's protospacer sequence
  source 1..20: mol_type = other DNA
aagaaagctacaggaaagca

SEQ ID NO: 338 - DNA, 20 bp, synthetic construct
  misc_feature 1..20: note = target gene's protospacer sequence
  source 1..20: mol_type = other DNA
caaaacccaactgattcacc

SEQ ID NO: 339 - DNA, 20 bp, synthetic construct
  misc_feature 1..20: note = target gene's protospacer sequence
  source 1..20: mol_type = other DNA
caaaagctaccacacatagc

SEQ ID NO: 340 - DNA, 20 bp, synthetic construct
  misc_feature 1..20: note = target gene's protospacer sequence
  source 1..20: mol_type = other DNA
caaaactgtggccaatacag

SEQ ID NO: 341 - DNA, 20 bp, synthetic construct
  misc_feature 1..20: note = target gene's protospacer sequence
  source 1..20: mol_type = other DNA
gaaaactgcaggcaagattc

SEQ ID NO: 342 - DNA, 20 bp, synthetic construct
  misc_feature 1..20: note = target gene's protospacer sequence
  source 1..20: mol_type = other DNA
caaaactgtacacgtgggcc

SEQ ID NO: 343 - DNA, 20 bp, synthetic construct
  misc_feature 1..20: note = target gene's protospacer sequence
  source 1..20: mol_type = other DNA
caaaacgtgcacaatgtgca

SEQ ID NO: 344 - DNA, 20 bp, synthetic construct
  misc_feature 1..20: note = target gene's protospacer sequence
  source 1..20: mol_type = other DNA
cccccacaggattgtaataa

SEQ ID NO: 345 - DNA, 20 bp, synthetic construct
  misc_feature 1..20: note = target gene's protospacer sequence
  source 1..20: mol_type = other DNA
ggccaagtgcgaagtcagag

SEQ ID NO: 346 - DNA, 20 bp, synthetic construct
  misc_feature 1..20: note = target gene's protospacer sequence
  source 1..20: mol_type = other DNA
ctaggacactcaccctgttg

SEQ ID NO: 347 - DNA, 20 bp, synthetic construct
  misc_feature 1..20: note = target gene's protospacer sequence
  source 1..20: mol_type = other DNA
ctagcacacagtgggcagag

SEQ ID NO: 348 - DNA, 20 bp, synthetic construct
  misc_feature 1..20: note = target gene's protospacer sequence
  source 1..20: mol_type = other DNA
ctaggacactcaccctggag

SEQ ID NO: 349 - DNA, 20 bp, synthetic construct
  misc_feature 1..20: note = target gene's protospacer sequence
  source 1..20: mol_type = other DNA
ctagtcggccattcagagag

SEQ ID NO: 350 - DNA, 20 bp, synthetic construct
  misc_feature 1..20: note = target gene's protospacer sequence
  source 1..20: mol_type = other DNA
gcagtcggaatggcggatgg

SEQ ID NO: 351 - DNA, 20 bp, synthetic construct
  misc_feature 1..20: note = target gene's protospacer sequence
  source 1..20: mol_type = other DNA
agaacacatacccctgggcc

SEQ ID NO: 352 - DNA, 20 bp, synthetic construct
  misc_feature 1..20: note = target gene's protospacer sequence
  source 1..20: mol_type = other DNA
cagtgtgtgcaggaacggag

SEQ ID NO: 353 - DNA, 20 bp, synthetic construct
  misc_feature 1..20: note = target gene's protospacer sequence
  source 1..20: mol_type = other DNA
atacagaaatcctaaatggt

SEQ ID NO: 354 - DNA, 20 bp, synthetic construct
  misc_feature 1..20: note = target gene's protospacer sequence
  source 1..20: mol_type = other DNA
aagaaagctacaggaaagca

SEQ ID NO: 355 - DNA, 20 bp, synthetic construct
  misc_feature 1..20: note = target gene's protospacer sequence
  source 1..20: mol_type = other DNA
aataagtcttaccacgtgtc

SEQ ID NO: 356 - DNA, 20 bp, synthetic construct
  misc_feature 1..20: note = target gene's protospacer sequence
  source 1..20: mol_type = other DNA
acaaagaaaccagcagtggc

SEQ ID NO: 357 - DNA, 20 bp, synthetic construct
  misc_feature 1..20: note = target gene's protospacer sequence
  source 1..20: mol_type = other DNA
acaagttcagaatcacctta

SEQ ID NO: 358 - DNA, 20 bp, synthetic construct
  misc_feature 1..20: note = target gene's protospacer sequence
  source 1..20: mol_type = other DNA
aggactatgtgtggccagtg

SEQ ID NO: 359 - DNA, 20 bp, synthetic construct
  misc_feature 1..20: note = target gene's protospacer sequence
  source 1..20: mol_type = other DNA
caaagaaatgtactgcctta

SEQ ID NO: 360 - DNA, 20 bp, synthetic construct
  misc_feature 1..20: note = target gene's protospacer sequence
  source 1..20: mol_type = other DNA
caacagcctcaccaggaaca

SEQ ID NO: 361 - DNA, 20 bp, synthetic construct
  misc_feature 1..20: note = target gene's protospacer sequence
  source 1..20: mol_type = other DNA
cacaagggatctgagacttg

SEQ ID NO: 362 - DNA, 20 bp, synthetic construct
  misc_feature 1..20: note = target gene's protospacer sequence
  source 1..20: mol_type = other DNA
cacataggccattcagaaac

SEQ ID NO: 363 - DNA, 20 bp, synthetic construct
  misc_feature 1..20: note = target gene's protospacer sequence
  source 1..20: mol_type = other DNA
cagagtcccgggaacaagcc

SEQ ID NO: 364 - DNA, 20 bp, synthetic construct
  misc_feature 1..20: note = target gene's protospacer sequence
  source 1..20: mol_type = other DNA
catacagggctctgtaccca

SEQ ID NO: 365 - DNA, 20 bp, synthetic construct
  misc_feature 1..20: note = target gene's protospacer sequence
  source 1..20: mol_type = other DNA
ctgagatttgcgaagagtta

SEQ ID NO: 366 - DNA, 20 bp, synthetic construct
  misc_feature 1..20: note = target gene's protospacer sequence
  source 1..20: mol_type = other DNA
cttagtagtctcagaaccaa

SEQ ID NO: 367 - DNA, 20 bp, synthetic construct
  misc_feature 1..20: note = target gene's protospacer sequence
  source 1..20: mol_type = other DNA
gaaatatgactggaagtaaa

SEQ ID NO: 368 - DNA, 20 bp, synthetic construct
  misc_feature 1..20: note = target gene's protospacer sequence
  source 1..20: mol_type = other DNA
gagagaccgctcaggctgga

SEQ ID NO: 369 - DNA, 20 bp, synthetic construct
  misc_feature 1..20: note = target gene's protospacer sequence
  source 1..20: mol_type = other DNA
gcagtacacctgagggaaca

SEQ ID NO: 370 - DNA, 20 bp, synthetic construct
  misc_feature 1..20: note = target gene's protospacer sequence
  source 1..20: mol_type = other DNA
gcattaaggccagcgctggg

SEQ ID NO: 371 - DNA, 20 bp, synthetic construct
  misc_feature 1..20: note = target gene's protospacer sequence
  source 1..20: mol_type = other DNA
gccatggtgaaggtgaaatc

SEQ ID NO: 372 - DNA, 20 bp, synthetic construct
  misc_feature 1..20: note = target gene's protospacer sequence
  source 1..20: mol_type = other DNA
ggcaagggtcttgatgcatc

SEQ ID NO: 373 - DNA, 20 bp, synthetic construct
  misc_feature 1..20: note = target gene's protospacer sequence
  source 1..20: mol_type = other DNA
gtaggctgctgttggacaga

SEQ ID NO: 374 - DNA, 20 bp, synthetic construct
  misc_feature 1..20: note = target gene's protospacer sequence
  source 1..20: mol_type = other DNA
gtcaaataaagaaaaatacg

SEQ ID NO: 375 - DNA, 20 bp, synthetic construct
  misc_feature 1..20: note = target gene's protospacer sequence
  source 1..20: mol_type = other DNA
agagcagcgattgtaaggag

SEQ ID NO: 376 - DNA, 24 bp, synthetic construct
  misc_feature 1..24: note = target gene's protospacer sequence with PAM in 5'
  source 1..24: mol_type = other DNA
tttgcacacacacagtgggctacc

SEQ ID NO: 377 - DNA, 24 bp, synthetic construct
  misc_feature 1..24: note = target gene's protospacer sequence with PAM in 5'
  source 1..24: mol_type = other DNA
tttgcatccccaggacacacacac

SEQ ID NO: 378 - DNA, 24 bp, synthetic construct
  misc_feature 1..24: note = target gene's protospacer sequence with PAM in 5'
  source 1..24: mol_type = other DNA
tttacaaagacactcaccctgttg

SEQ ID NO: 379 - DNA, 24 bp, synthetic construct
  misc_feature 1..24: note = target gene's protospacer sequence with PAM in 5'
  source 1..24: mol_type = other DNA
tttaaagaaagctacaggaaagca

SEQ ID NO: 380 - DNA, 24 bp, synthetic construct
  misc_feature 1..24: note = target gene's protospacer sequence with PAM in 5'
  source 1..24: mol_type = other DNA
tttacaaaacccaactgattcacc

SEQ ID NO: 381 - DNA, 24 bp, synthetic construct
  misc_feature 1..24: note = target gene's protospacer sequence with PAM in 5'
  source 1..24: mol_type = other DNA
tttacaaaagctaccacacatagc

SEQ ID NO: 382 - DNA, 24 bp, synthetic construct
  misc_feature 1..24: note = target gene's protospacer sequence with PAM in 5'
  source 1..24: mol_type = other DNA
tttacaaaactgtggccaatacag

SEQ ID NO: 383 - DNA, 24 bp, synthetic construct
  misc_feature 1..24: note = target gene's protospacer sequence with PAM in 5'
  source 1..24: mol_type = other DNA
tttggaaaactgcaggcaagattc

SEQ ID NO: 384 - DNA, 24 bp, synthetic construct
  misc_feature 1..24: note = target gene's protospacer sequence with PAM in 5'
  source 1..24: mol_type = other DNA
tttgcaaaactgtacacgtgggcc

SEQ ID NO: 385 - DNA, 24 bp, synthetic construct
  misc_feature 1..24: note = target gene's protospacer sequence with PAM in 5'
  source 1..24: mol_type = other DNA
tttgcaaaacgtgcacaatgtgca

SEQ ID NO: 386 - DNA, 24 bp, synthetic construct
  misc_feature 1..24: note = target gene's protospacer sequence with PAM in 5'
  source 1..24: mol_type = other DNA
tttacccccacaggattgtaataa

SEQ ID NO: 387 - DNA, 24 bp, synthetic construct
  misc_feature 1..24: note = target gene's protospacer sequence with PAM in 5'
  source 1..24: mol_type = other DNA
tttaggccaagtgcgaagtcagag

SEQ ID NO: 388 - DNA, 24 bp, synthetic construct
  misc_feature 1..24: note = target gene's protospacer sequence with PAM in 5'
  source 1..24: mol_type = other DNA
tttactaggacactcaccctgttg

SEQ ID NO: 389 - DNA, 24 bp, synthetic construct
  misc_feature 1..24: note = target gene's protospacer sequence with PAM in 5'
  source 1..24: mol_type = other DNA
tttgctagcacacagtgggcagag

SEQ ID NO: 390 - DNA, 24 bp, synthetic construct
  misc_feature 1..24: note = target gene's protospacer sequence with PAM in 5'
  source 1..24: mol_type = other DNA
tttactaggacactcaccctggag

SEQ ID NO: 391 - DNA, 24 bp, synthetic construct
  misc_feature 1..24: note = target gene's protospacer sequence with PAM in 5'
  source 1..24: mol_type = other DNA
tttactagtcggccattcagagag

SEQ ID NO: 392 - DNA, 24 bp, synthetic construct
  misc_feature 1..24: note = target gene's protospacer sequence with PAM in 5'
  source 1..24: mol_type = other DNA
tttagcagtcggaatggcggatgg

SEQ ID NO: 393 - DNA, 24 bp, synthetic construct
  misc_feature 1..24: note = target gene's protospacer sequence with PAM in 5'
  source 1..24: mol_type = other DNA
tttaagaacacatacccctgggcc

SEQ ID NO: 394 - DNA, 24 bp, synthetic construct
  misc_feature 1..24: note = target gene's protospacer sequence with PAM in 5'
  source 1..24: mol_type = other DNA
tttgcagtgtgtgcaggaacggag

SEQ ID NO: 395 - DNA, 24 bp, synthetic construct
  misc_feature 1..24: note = target gene's protospacer sequence with PAM in 5'
  source 1..24: mol_type = other DNA
tttaatacagaaatcctaaatggt

SEQ ID NO: 396 - DNA, 24 bp, synthetic construct
  misc_feature 1..24: note = target gene's protospacer sequence with PAM in 5'
  source 1..24: mol_type = other DNA
tttaaagaaagctacaggaaagca

SEQ ID NO: 397 - DNA, 24 bp, synthetic construct
  misc_feature 1..24: note = target gene's protospacer sequence with PAM in 5'
  source 1..24: mol_type = other DNA
tttaaataagtcttaccacgtgtc

SEQ ID NO: 398 - DNA, 24 bp, synthetic construct
  misc_feature 1..24: note = target gene's protospacer sequence with PAM in 5'
  source 1..24: mol_type = other DNA
tttaacaaagaaaccagcagtggc

SEQ ID NO: 399 - DNA, 24 bp, synthetic construct
  misc_feature 1..24: note = target gene's protospacer sequence with PAM in 5'
  source 1..24: mol_type = other DNA
tttaacaagttcagaatcacctta

SEQ ID NO: 400 - DNA, 24 bp, synthetic construct
  misc_feature 1..24: note = target gene's protospacer sequence with PAM in 5'
  source 1..24: mol_type = other DNA
tttaaggactatgtgtggccagtg

SEQ ID NO: 401 - DNA, 24 bp, synthetic construct
  misc_feature 1..24: note = target gene's protospacer sequence with PAM in 5'
  source 1..24: mol_type = other DNA
tttacaaagaaatgtactgcctta

SEQ ID NO: 402 - DNA, 24 bp, synthetic construct
  misc_feature 1..24: note = target gene's protospacer sequence with PAM in 5'
  source 1..24: mol_type = other DNA
tttacaacagcctcaccaggaaca

SEQ ID NO: 403 - DNA, 24 bp, synthetic construct
  misc_feature 1..24: note = target gene's protospacer sequence with PAM in 5'
  source 1..24: mol_type = other DNA
tttacacaagggatctgagacttg

SEQ ID NO: 404 - DNA, 24 bp, synthetic construct
  misc_feature 1..24: note = target gene's protospacer sequence with PAM in 5'
  source 1..24: mol_type = other DNA
tttacacataggccattcagaaac

SEQ ID NO: 405 - DNA, 24 bp, synthetic construct
  misc_feature 1..24: note = target gene's protospacer sequence with PAM in 5'
  source 1..24: mol_type = other DNA
tttacagagtcccgggaacaagcc

SEQ ID NO: 406 - DNA, 24 bp, synthetic construct
  misc_feature 1..24: note = target gene's protospacer sequence with PAM in 5'
  source 1..24: mol_type = other DNA
tttacatacagggctctgtaccca

SEQ ID NO: 407 - DNA, 24 bp, synthetic construct
  misc_feature 1..24: note = target gene's protospacer sequence with PAM in 5'
  source 1..24: mol_type = other DNA
tttactgagatttgcgaagagtta

SEQ ID NO: 408 - DNA, 24 bp, synthetic construct
  misc_feature 1..24: note = target gene's protospacer sequence with PAM in 5'
  source 1..24: mol_type = other DNA
tttacttagtagtctcagaaccaa

SEQ ID NO: 409 - DNA, 24 bp, synthetic construct
  misc_feature 1..24: note = target gene's protospacer sequence with PAM in 5'
  source 1..24: mol_type = other DNA
tttagaaatatgactggaagtaaa

SEQ ID NO: 410 - DNA, 24 bp, synthetic construct
  misc_feature 1..24: note = target gene's protospacer sequence with PAM in 5'
  source 1..24: mol_type = other DNA
tttagagagaccgctcaggctgga

SEQ ID NO: 411 - DNA, 24 bp, synthetic construct
  misc_feature 1..24: note = target gene's protospacer sequence with PAM in 5'
  source 1..24: mol_type = other DNA
tttagcagtacacctgagggaaca

SEQ ID NO: 412 - DNA, 24 bp, synthetic construct
  misc_feature 1..24: note = target gene's protospacer sequence with PAM in 5'
  source 1..24: mol_type = other DNA
tttagcattaaggccagcgctggg

SEQ ID NO: 413 - DNA, 24 bp, synthetic construct
  misc_feature 1..24: note = target gene's protospacer sequence with PAM in 5'
  source 1..24: mol_type = other DNA
tttagccatggtgaaggtgaaatc

SEQ ID NO: 414 - DNA, 24 bp, synthetic construct
  misc_feature 1..24: note = target gene's protospacer sequence with PAM in 5'
  source 1..24: mol_type = other DNA
tttaggcaagggtcttgatgcatc

SEQ ID NO: 415 - DNA, 24 bp, synthetic construct
  misc_feature 1..24: note = target gene's protospacer sequence with PAM in 5'
  source 1..24: mol_type = other DNA
tttagtaggctgctgttggacaga

SEQ ID NO: 416 - DNA, 24 bp, synthetic construct
  misc_feature 1..24: note = target gene's protospacer sequence with PAM in 5'
  source 1..24: mol_type = other DNA
tttagtcaaataaagaaaaatacg

SEQ ID NO: 417 - DNA, 24 bp, synthetic construct
  misc_feature 1..24: note = target gene's protospacer sequence with PAM in 5'
  source 1..24: mol_type = other DNA
tttaagagcagcgattgtaaggag

SEQ ID NO: 418 - protein, 949 aa, synthetic construct
  REGION 1..949: note = dTnpB(D354A)-10aa-ABE-C2
MGEKSSRRRRNGKSGAWTAAITSCVGGKMAKNTITKTLKLRIVRPYNSAEVEKIVADEKNNREKIALEKNKDKVKEACSKHLKVAAYCTTQVERNACLFCKARKLDDKFYQKLRGQFPDAVFWQEISEIFRQLQKQAAEIYNQSLIELYYEIFIKGKGIANASSVEHYLSDVCYTRAAELFKNAAIASGLRSKIKSNFRLKELKNMKSGLPTTKSDNFPIPLVKQKGGQYTGFEISNHNSDFIIKIPFGRWQVKKEIDKYRPWEKFDFEQVQKSPKPISLLLSTQRRKRNKGWSKDEGTEAEIKKVMNGDYQTSYIEVKRGSKIGEKSAWMLNLSIDVPKIDKGVDPSIIGGIAVGVKSPLVCAINNAFSRYSISDNDLFHFNKKMFARRRILLKKNRHKRAGHGAKNKLKPITILTEKSERFRKKLIERWACEIADFFIKNKVGTVQMENLESMKRKEDSYFNIRLRGFWPYAEMQNKIEFKLKQYGIEIRKVAPNNTSKTCSKCGHLNNYFNFEYRKKNKFPHFKCEKCNFKENADYNAALNISNPKLKSTKEEPSGGSSGGSSGMSEVEFSHEYWMRHALTLAKRAWDEREVPVGAVLVHNNRVIGEGWNRPIGRHDPTAHAEIMALRQGGLVMQNYRLIDATLYVTLEPCVMCAGAMIHSRIGRVVFGARDAKTGAAGSLMDVLHHPGMNHRVEITEGILADECAALLSDFFRMRRQEIKAQKKAQSSTDSGGSSGGSSGSETPGTSESATPESSGGSSGGSMSEVEFSHEYWMRHALTLAKRARDEREVPVGAVLVLNNRVIGEGWNRAIGLHDPTAHAEIMALRQGGLVMQNYRLIDATLYVTFEPCVMCAGAMIHSRIGRVVFGVRNAKTGAAGSLMDVLHYPGMNHRVEITEGILADECAALLCYFFRMPRQVFNAQKKAQSSTDKRPAATKKAGQAKKKK

SEQ ID NO: 419 - protein, 953 aa, synthetic construct
  REGION 1..953: note = dTnpB(D354A)-14aa-ABE-C2
MGEKSSRRRRNGKSGAWTAAITSCVGGKMAKNTITKTLKLRIVRPYNSAEVEKIVADEKNNREKIALEKNKDKVKEACSKHLKVAAYCTTQVERNACLFCKARKLDDKFYQKLRGQFPDAVFWQEISEIFRQLQKQAAEIYNQSLIELYYEIFIKGKGIANASSVEHYLSDVCYTRAAELFKNAAIASGLRSKIKSNFRLKELKNMKSGLPTTKSDNFPIPLVKQKGGQYTGFEISNHNSDFIIKIPFGRWQVKKEIDKYRPWEKFDFEQVQKSPKPISLLLSTQRRKRNKGWSKDEGTEAEIKKVMNGDYQTSYIEVKRGSKIGEKSAWMLNLSIDVPKIDKGVDPSIIGGIAVGVKSPLVCAINNAFSRYSISDNDLFHFNKKMFARRRILLKKNRHKRAGHGAKNKLKPITILTEKSERFRKKLIERWACEIADFFIKNKVGTVQMENLESMKRKEDSYFNIRLRGFWPYAEMQNKIEFKLKQYGIEIRKVAPNNTSKTCSKCGHLNNYFNFEYRKKNKFPHFKCEKCNFKENADYNAALNISNPKLKSTKEEPSGGSSGGSSGSETPMSEVEFSHEYWMRHALTLAKRAWDEREVPVGAVLVHNNRVIGEGWNRPIGRHDPTAHAEIMALRQGGLVMQNYRLIDATLYVTLEPCVMCAGAMIHSRIGRVVFGARDAKTGAAGSLMDVLHHPGMNHRVEITEGILADECAALLSDFFRMRRQEIKAQKKAQSSTDSGGSSGGSSGSETPGTSESATPESSGGSSGGSMSEVEFSHEYWMRHALTLAKRARDEREVPVGAVLVLNNRVIGEGWNRAIGLHDPTAHAEIMALRQGGLVMQNYRLIDATLYVTFEPCVMCAGAMIHSRIGRVVFGVRNAKTGAAGSLMDVLHYPGMNHRVEITEGILADECAALLCYFFRMPRQVFNAQKKAQSSTDKRPAATKKAGQAKKKK

SEQ ID NO: 420 - protein, 955 aa, synthetic construct
  REGION 1..955: note = dTnpB(D354A)-16aa-ABE-C2
MGEKSSRRRRNGKSGAWTAAITSCVGGKMAKNTITKTLKLRIVRPYNSAEVEKIVADEKNNREKIALEKNKDKVKEACSKHLKVAAYCTTQVERNACLFCKARKLDDKFYQKLRGQFPDAVFWQEISEIFRQLQKQAAEIYNQSLIELYYEIFIKGKGIANASSVEHYLSDVCYTRAAELFKNAAIASGLRSKIKSNFRLKELKNMKSGLPTTKSDNFPIPLVKQKGGQYTGFEISNHNSDFIIKIPFGRWQVKKEIDKYRPWEKFDFEQVQKSPKPISLLLSTQRRKRNKGWSKDEGTEAEIKKVMNGDYQTSYIEVKRGSKIGEKSAWMLNLSIDVPKIDKGVDPSIIGGIAVGVKSPLVCAINNAFSRYSISDNDLFHFNKKMFARRRILLKKNRHKRAGHGAKNKLKPITILTEKSERFRKKLIERWACEIADFFIKNKVGTVQMENLESMKRKEDSYFNIRLRGFWPYAEMQNKIEFKLKQYGIEIRKVAPNNTSKTCSKCGHLNNYFNFEYRKKNKFPHFKCEKCNFKENADYNAALNISNPKLKSTKEEPSGGSSGGSSGSETPGTMSEVEFSHEYWMRHALTLAKRAWDEREVPVGAVLVHNNRVIGEGWNRPIGRHDPTAHAEIMALRQGGLVMQNYRLIDATLYVTLEPCVMCAGAMIHSRIGRVVFGARDAKTGAAGSLMDVLHHPGMNHRVEITEGILADECAALLSDFFRMRRQEIKAQKKAQSSTDSGGSSGGSSGSETPGTSESATPESSGGSSGGSMSEVEFSHEYWMRHALTLAKRARDEREVPVGAVLVLNNRVIGEGWNRAIGLHDPTAHAEIMALRQGGLVMQNYRLIDATLYVTFEPCVMCAGAMIHSRIGRVVFGVRNAKTGAAGSLMDVLHYPGMNHRVEITEGILADECAALLCYFFRMPRQVFNAQKKAQSSTDKRPAATKKAGQAKKKK

SEQ ID NO: 421 - protein, 959 aa, synthetic construct
  REGION 1..959: note = dTnpB(D354A)-20aa-ABE-C2
MGEKSSRRRRNGKSGAWTAAITSCVGGKMAKNTITKTLKLRIVRPYNSAEVEKIVADEKNNREKIALEKNKDKVKEACSKHLKVAAYCTTQVERNACLFCKARKLDDKFYQKLRGQFPDAVFWQEISEIFRQLQKQAAEIYNQSLIELYYEIFIKGKGIANASSVEHYLSDVCYTRAAELFKNAAIASGLRSKIKSNFRLKELKNMKSGLPTTKSDNFPIPLVKQKGGQYTGFEISNHNSDFIIKIPFGRWQVKKEIDKYRPWEKFDFEQVQKSPKPISLLLSTQRRKRNKGWSKDEGTEAEIKKVMNGDYQTSYIEVKRGSKIGEKSAWMLNLSIDVPKIDKGVDPSIIGGIAVGVKSPLVCAINNAFSRYSISDNDLFHFNKKMFARRRILLKKNRHKRAGHGAKNKLKPITILTEKSERFRKKLIERWACEIADFFIKNKVGTVQMENLESMKRKEDSYFNIRLRGFWPYAEMQNKIEFKLKQYGIEIRKVAPNNTSKTCSKCGHLNNYFNFEYRKKNKFPHFKCEKCNFKENADYNAALNISNPKLKSTKEEPSGGSSGGSSGSETPGTSESAMSEVEFSHEYWMRHALTLAKRAWDEREVPVGAVLVHNNRVIGEGWNRPIGRHDPTAHAEIMALRQGGLVMQNYRLIDATLYVTLEPCVMCAGAMIHSRIGRVVFGARDAKTGAAGSLMDVLHHPGMNHRVEITEGILADECAALLSDFFRMRRQEIKAQKKAQSSTDSGGSSGGSSGSETPGTSESATPESSGGSSGGSMSEVEFSHEYWMRHALTLAKRARDEREVPVGAVLVLNNRVIGEGWNRAIGLHDPTAHAEIMALRQGGLVMQNYRLIDATLYVTFEPCVMCAGAMIHSRIGRVVFGVRNAKTGAAGSLMDVLHYPGMNHRVEITEGILADECAALLCYFFRMPRQVFNAQKKAQSSTDKRPAATKKAGQAKKKK

SEQ ID NO: 422 - protein, 963 aa, synthetic construct
  REGION 1..963: note = dTnpB(D354A)-24aa-ABE-C2
MGEKSSRRRRNGKSGAWTAAITSCVGGKMAKNTITKTLKLRIVRPYNSAEVEKIVADEKNNREKIALEKNKDKVKEACSKHLKVAAYCTTQVERNACLFCKARKLDDKFYQKLRGQFPDAVFWQEISEIFRQLQKQAAEIYNQSLIELYYEIFIKGKGIANASSVEHYLSDVCYTRAAELFKNAAIASGLRSKIKSNFRLKELKNMKSGLPTTKSDNFPIPLVKQKGGQYTGFEISNHNSDFIIKIPFGRWQVKKEIDKYRPWEKFDFEQVQKSPKPISLLLSTQRRKRNKGWSKDEGTEAEIKKVMNGDYQTSYIEVKRGSKIGEKSAWMLNLSIDVPKIDKGVDPSIIGGIAVGVKSPLVCAINNAFSRYSISDNDLFHFNKKMFARRRILLKKNRHKRAGHGAKNKLKPITILTEKSERFRKKLIERWACEIADFFIKNKVGTVQMENLESMKRKEDSYFNIRLRGFWPYAEMQNKIEFKLKQYGIEIRKVAPNNTSKTCSKCGHLNNYFNFEYRKKNKFPHFKCEKCNFKENADYNAALNISNPKLKSTKEEPSGGSSGGSSGSETPGTSESATPESMSEVEFSHEYWMRHALTLAKRAWDEREVPVGAVLVHNNRVIGEGWNRPIGRHDPTAHAEIMALRQGGLVMQNYRLIDATLYVTLEPCVMCAGAMIHSRIGRVVFGARDAKTGAAGSLMDVLHHPGMNHRVEITEGILADECAALLSDFFRMRRQEIKAQKKAQSSTDSGGSSGGSSGSETPGTSESATPESSGGSSGGSMSEVEFSHEYWMRHALTLAKRARDEREVPVGAVLVLNNRVIGEGWNRAIGLHDPTAHAEIMALRQGGLVMQNYRLIDATLYVTFEPCVMCAGAMIHSRIGRVVFGVRNAKTGAAGSLMDVLHYPGMNHRVEITEGILADECAALLCYFFRMPRQVFNAQKKAQSSTDKRPAATKKAGQAKKKK

SEQ ID NO: 423 - protein, 967 aa, synthetic construct
  REGION 1..967: note = dTnpB(D354A)-28aa-ABE-C2
MGEKSSRRRRNGKSGAWTAAITSCVGGKMAKNTITKTLKLRIVRPYNSAEVEKIVADEKNNREKIALEKNKDKVKEACSKHLKVAAYCTTQVERNACLFCKARKLDDKFYQKLRGQFPDAVFWQEISEIFRQLQKQAAEIYNQSLIELYYEIFIKGKGIANASSVEHYLSDVCYTRAAELFKNAAIASGLRSKIKSNFRLKELKNMKSGLPTTKSDNFPIPLVKQKGGQYTGFEISNHNSDFIIKIPFGRWQVKKEIDKYRPWEKFDFEQVQKSPKPISLLLSTQRRKRNKGWSKDEGTEAEIKKVMNGDYQTSYIEVKRGSKIGEKSAWMLNLSIDVPKIDKGVDPSIIGGIAVGVKSPLVCAINNAFSRYSISDNDLFHFNKKMFARRRILLKKNRHKRAGHGAKNKLKPITILTEKSERFRKKLIERWACEIADFFIKNKVGTVQMENLESMKRKEDSYFNIRLRGFWPYAEMQNKIEFKLKQYGIEIRKVAPNNTSKTCSKCGHLNNYFNFEYRKKNKFPHFKCEKCNFKENADYNAALNISNPKLKSTKEEPSGGSSGGSSGSETPGTSESATPESSGGSMSEVEFSHEYWMRHALTLAKRAWDEREVPVGAVLVHNNRVIGEGWNRPIGRHDPTAHAEIMALRQGGLVMQNYRLIDATLYVTLEPCVMCAGAMIHSRIGRVVFGARDAKTGAAGSLMDVLHHPGMNHRVEITEGILADECAALLSDFFRMRRQEIKAQKKAQSSTDSGGSSGGSSGSETPGTSESATPESSGGSSGGSMSEVEFSHEYWMRHALTLAKRARDEREVPVGAVLVLNNRVIGEGWNRAIGLHDPTAHAEIMALRQGGLVMQNYRLIDATLYVTFEPCVMCAGAMIHSRIGRVVFGVRNAKTGAAGSLMDVLHYPGMNHRVEITEGILADECAALLCYFFRMPRQVFNAQKKAQSSTDKRPAATKKAGQAKKKK

SEQ ID NO: 424 - protein, 975 aa, synthetic construct
  REGION 1..975: note = dTnpB(D354A)-36aa-ABE-C2
MGEKSSRRRRNGKSGAWTAAITSCVGGKMAKNTITKTLKLRIVRPYNSAEVEKIVADEKNNREKIALEKNKDKVKEACSKHLKVAAYCTTQVERNACLFCKARKLDDKFYQKLRGQFPDAVFWQEISEIFRQLQKQAAEIYNQSLIELYYEIFIKGKGIANASSVEHYLSDVCYTRAAELFKNAAIASGLRSKIKSNFRLKELKNMKSGLPTTKSDNFPIPLVKQKGGQYTGFEISNHNSDFIIKIPFGRWQVKKEIDKYRPWEKFDFEQVQKSPKPISLLLSTQRRKRNKGWSKDEGTEAEIKKVMNGDYQTSYIEVKRGSKIGEKSAWMLNLSIDVPKIDKGVDPSIIGGIAVGVKSPLVCAINNAFSRYSISDNDLFHFNKKMFARRRILLKKNRHKRAGHGAKNKLKPITILTEKSERFRKKLIERWACEIADFFIKNKVGTVQMENLESMKRKEDSYFNIRLRGFWPYAEMQNKIEFKLKQYGIEIRKVAPNNTSKTCSKCGHLNNYFNFEYRKKNKFPHFKCEKCNFKENADYNAALNISNPKLKSTKEEPSGGSSGGSSGSETPGTSESATPESSGGSSGGSSGSEMSEVEFSHEYWMRHALTLAKRAWDEREVPVGAVLVHNNRVIGEGWNRPIGRHDPTAHAEIMALRQGGLVMQNYRLIDATLYVTLEPCVMCAGAMIHSRIGRVVFGARDAKTGAAGSLMDVLHHPGMNHRVEITEGILADECAALLSDFFRMRRQEIKAQKKAQSSTDSGGSSGGSSGSETPGTSESATPESSGGSSGGSMSEVEFSHEYWMRHALTLAKRARDEREVPVGAVLVLNNRVIGEGWNRAIGLHDPTAHAEIMALRQGGLVMQNYRLIDATLYVTFEPCVMCAGAMIHSRIGRVVFGVRNAKTGAAGSLMDVLHYPGMNHRVEITEGILADECAALLCYFFRMPRQVFNAQKKAQSSTDKRPAATKKAGQAKKKK

SEQ ID NO: 425 - protein, 979 aa, synthetic construct
  REGION 1..979: note = dTnpB(D354A)-40aa-ABE-C2
MGEKSSRRRRNGKSGAWTAAITSCVGGKMAKNTITKTLKLRIVRPYNSAEVEKIVADEKNNREKIALEKNKDKVKEACSKHLKVAAYCTTQVERNACLFCKARKLDDKFYQKLRGQFPDAVFWQEISEIFRQLQKQAAEIYNQSLIELYYEIFIKGKGIANASSVEHYLSDVCYTRAAELFKNAAIASGLRSKIKSNFRLKELKNMKSGLPTTKSDNFPIPLVKQKGGQYTGFEISNHNSDFIIKIPFGRWQVKKEIDKYRPWEKFDFEQVQKSPKPISLLLSTQRRKRNKGWSKDEGTEAEIKKVMNGDYQTSYIEVKRGSKIGEKSAWMLNLSIDVPKIDKGVDPSIIGGIAVGVKSPLVCAINNAFSRYSISDNDLFHFNKKMFARRRILLKKNRHKRAGHGAKNKLKPITILTEKSERFRKKLIERWACEIADFFIKNKVGTVQMENLESMKRKEDSYFNIRLRGFWPYAEMQNKIEFKLKQYGIEIRKVAPNNTSKTCSKCGHLNNYFNFEYRKKNKFPHFKCEKCNFKENADYNAALNISNPKLKSTKEEPSGGSSGGSSGSETPGTSESATPESSGGSSGGSSGSETPGTMSEVEFSHEYWMRHALTLAKRAWDEREVPVGAVLVHNNRVIGEGWNRPIGRHDPTAHAEIMALRQGGLVMQNYRLIDATLYVTLEPCVMCAGAMIHSRIGRVVFGARDAKTGAAGSLMDVLHHPGMNHRVEITEGILADECAALLSDFFRMRRQEIKAQKKAQSSTDSGGSSGGSSGSETPGTSESATPESSGGSSGGSMSEVEFSHEYWMRHALTLAKRARDEREVPVGAVLVLNNRVIGEGWNRAIGLHDPTAHAEIMALRQGGLVMQNYRLIDATLYVTFEPCVMCAGAMIHSRIGRVVFGVRNAKTGAAGSLMDVLHYPGMNHRVEITEGILADECAALLCYFFRMPRQVFNAQKKAQSSTDKRPAATKKAGQAKKKK

SEQ ID NO: 426 - protein, 949 aa, synthetic construct
  REGION 1..949: note = dTnpB(D354A)-10aa-ABE-C3.1
MGEKSSRRRRNGKSGAWTAAITSCVGGKMAKNTITKTLKLRIVRPYNSAEVEKIVADEKNNREKIALEKNKDKVKEACSKHLKVAAYCTTQVERNACLFCKARKLDDKFYQKLRGQFPDAVFWQEISEIFRQLQKQAAEIYNQSLIELYYEIFIKGKGIANASSVEHYLSDVCYTRAAELFKNAAIASGLRSKIKSNFRLKELKNMKSGLPTTKSDNFPIPLVKQKGGQYTGFEISNHNSDFIIKIPFGRWQVKKEIDKYRPWEKFDFEQVQKSPKPISLLLSTQRRKRNKGWSKDEGTEAEIKKVMNGDYQTSYIEVKRGSKIGEKSAWMLNLSIDVPKIDKGVDPSIIGGIAVGVKSPLVCAINNAFSRYSISDNDLFHFNKKMFARRRILLKKNRHKRAGHGAKNKLKPITILTEKSERFRKKLIERWACEIADFFIKNKVGTVQMENLESMKRKEDSYFNIRLRGFWPYAEMQNKIEFKLKQYGIEIRKVAPNNTSKTCSKCGHLNNYFNFEYRKKNKFPHFKCEKCNFKENADYNAALNISNPKLKSTKEEPSGGSSGGSSGMSEVEFSHEYWMRHALTLAKRAWDEREVPVGAVLVHNNRVIGEGWNRPIGRHDPTAHAEIMALRQGGLVMQNYRLIDATLYVTLEPCVMCAGAMIHSRIGRVVFGARDAKTGAAGSLMDVLHHPGMNHRVEITEGILADECAALLSDFFRMRRQEIKAQKKAQSSTDSGGSSGGSSGSETPGTSESATPESSGGSSGGSMSEVEFSHEYWMRHALTLAKRARDEREVPVGAVLVLNNRVIGEGWNRAIGLHDPTAHAEIMALRQGGLVMQNYRLIDATLYVTFEPCVMCAGAMIHSRIGRVVFGWRQSKRGAAGSLMNVLNYPGMNHRVEITEGILADECAALLCDFYRMPRQVFNAQKKAQSSINKRPAATKKAGQAKKKK

SEQ ID NO: 427 - protein, 953 aa, synthetic construct
  REGION 1..953: note = dTnpB(D354A)-14aa-ABE-C3.1
MGEKSSRRRRNGKSGAWTAAITSCVGGKMAKNTITKTLKLRIVRPYNSAEVEKIVADEKNNREKIALEKNKDKVKEACSKHLKVAAYCTTQVERNACLFCKARKLDDKFYQKLRGQFPDAVFWQEISEIFRQLQKQAAEIYNQSLIELYYEIFIKGKGIANASSVEHYLSDVCYTRAAELFKNAAIASGLRSKIKSNFRLKELKNMKSGLPTTKSDNFPIPLVKQKGGQYTGFEISNHNSDFIIKIPFGRWQVKKEIDKYRPWEKFDFEQVQKSPKPISLLLSTQRRKRNKGWSKDEGTEAEIKKVMNGDYQTSYIEVKRGSKIGEKSAWMLNLSIDVPKIDKGVDPSIIGGIAVGVKSPLVCAINNAFSRYSISDNDLFHFNKKMFARRRILLKKNRHKRAGHGAKNKLKPITILTEKSERFRKKLIERWACEIADFFIKNKVGTVQMENLESMKRKEDSYFNIRLRGFWPYAEMQNKIEFKLKQYGIEIRKVAPNNTSKTCSKCGHLNNYFNFEYRKKNKFPHFKCEKCNFKENADYNAALNISNPKLKSTKEEPSGGSSGGSSGSETPMSEVEFSHEYWMRHALTLAKRAWDEREVPVGAVLVHNNRVIGEGWNRPIGRHDPTAHAEIMALRQGGLVMQNYRLIDATLYVTLEPCVMCAGAMIHSRIGRVVFGARDAKTGAAGSLMDVLHHPGMNHRVEITEGILADECAALLSDFFRMRRQEIKAQKKAQSSTDSGGSSGGSSGSETPGTSESATPESSGGSSGGSMSEVEFSHEYWMRHALTLAKRARDEREVPVGAVLVLNNRVIGEGWNRAIGLHDPTAHAEIMALRQGGLVMQNYRLIDATLYVTFEPCVMCAGAMIHSRIGRVVFGWRQSKRGAAGSLMNVLNYPGMNHRVEITEGILADECAALLCDFYRMPRQVFNAQKKAQSSINKRPAATKKAGQAKKKK

SEQ ID NO: 428 - protein, 955 aa, synthetic construct
  REGION 1..955: note = dTnpB(D354A)-16aa-ABE-C3.1
MGEKSSRRRRNGKSGAWTAAITSCVGGKMAKNTITKTLKLRIVRPYNSAEVEKIVADEKNNREKIALEKNKDKVKEACSKHLKVAAYCTTQVERNACLFCKARKLDDKFYQKLRGQFPDAVFWQEISEIFRQLQKQAAEIYNQSLIELYYEIFIKGKGIANASSVEHYLSDVCYTRAAELFKNAAIASGLRSKIKSNFRLKELKNMKSGLPTTKSDNFPIPLVKQKGGQYTGFEISNHNSDFIIKIPFGRWQVKKEIDKYRPWEKFDFEQVQKSPKPISLLLSTQRRKRNKGWSKDEGTEAEIKKVMNGDYQTSYIEVKRGSKIGEKSAWMLNLSIDVPKIDKGVDPSIIGGIAVGVKSPLVCAINNAFSRYSISDNDLFHFNKKMFARRRILLKKNRHKRAGHGAKNKLKPITILTEKSERFRKKLIERWACEIADFFIKNKVGTVQMENLESMKRKEDSYFNIRLRGFWPYAEMQNKIEFKLKQYGIEIRKVAPNNTSKTCSKCGHLNNYFNFEYRKKNKFPHFKCEKCNFKENADYNAALNISNPKLKSTKEEPSGGSSGGSSGSETPGTMSEVEFSHEYWMRHALTLAKRAWDEREVPVGAVLVHNNRVIGEGWNRPIGRHDPTAHAEIMALRQGGLVMQNYRLIDATLYVTLEPCVMCAGAMIHSRIGRVVFGARDAKTGAAGSLMDVLHHPGMNHRVEITEGILADECAALLSDFFRMRRQEIKAQKKAQSSTDSGGSSGGSSGSETPGTSESATPESSGGSSGGSMSEVEFSHEYWMRHALTLAKRARDEREVPVGAVLVLNNRVIGEGWNRAIGLHDPTAHAEIMALRQGGLVMQNYRLIDATLYVTFEPCVMCAGAMIHSRIGRVVFGWRQSKRGAAGSLMNVLNYPGMNHRVEITEGILADECAALLCDFYRMPRQVFNAQKKAQSSINKRPAATKKAGQAKKKK

SEQ ID NO: 429 - protein, 959 aa, synthetic construct
  REGION 1..959: note = dTnpB(D354A)-20aa-ABE-C3.1
MGEKSSRRRRNGKSGAWTAAITSCVGGKMAKNTITKTLKLRIVRPYNSAEVEKIVADEKNNREKIALEKNKDKVKEACSKHLKVAAYCTTQVERNACLFCKARKLDDKFYQKLRGQFPDAVFWQEISEIFRQLQKQAAEIYNQSLIELYYEIFIKGKGIANASSVEHYLSDVCYTRAAELFKNAAIASGLRSKIKSNFRLKELKNMKSGLPTTKSDNFPIPLVKQKGGQYTGFEISNHNSDFIIKIPFGRWQVKKEIDKYRPWEKFDFEQVQKSPKPISLLLSTQRRKRNKGWSKDEGTEAEIKKVMNGDYQTSYIEVKRGSKIGEKSAWMLNLSIDVPKIDKGVDPSIIGGIAVGVKSPLVCAINNAFSRYSISDNDLFHFNKKMFARRRILLKKNRHKRAGHGAKNKLKPITILTEKSERFRKKLIERWACEIADFFIKNKVGTVQMENLESMKRKEDSYFNIRLRGFWPYAEMQNKIEFKLKQYGIEIRKVAPNNTSKTCSKCGHLNNYFNFEYRKKNKFPHFKCEKCNFKENADYNAALNISNPKLKSTKEEPSGGSSGGSSGSETPGTSESAMSEVEFSHEYWMRHALTLAKRAWDEREVPVGAVLVHNNRVIGEGWNRPIGRHDPTAHAEIMALRQGGLVMQNYRLIDATLYVTLEPCVMCAGAMIHSRIGRVVFGARDAKTGAAGSLMDVLHHPGMNHRVEITEGILADECAALLSDFFRMRRQEIKAQKKAQSSTDSGGSSGGSSGSETPGTSESATPESSGGSSGGSMSEVEFSHEYWMRHALTLAKRARDEREVPVGAVLVLNNRVIGEGWNRAIGLHDPTAHAEIMALRQGGLVMQNYRLIDATLYVTFEPCVMCAGAMIHSRIGRVVFGWRQSKRGAAGSLMNVLNYPGMNHRVEITEGILADECAALLCDFYRMPRQVFNAQKKAQSSINKRPAATKKAGQAKKKK

SEQ ID NO: 430 - protein, 963 aa, synthetic construct
  REGION 1..963: note = dTnpB(D354A)-24aa-ABE-C3.1
MGEKSSRRRRNGKSGAWTAAITSCVGGKMAKNTITKTLKLRIVRPYNSAEVEKIVADEKNNREKIALEKNKDKVKEACSKHLKVAAYCTTQVERNACLFCKARKLDDKFYQKLRGQFPDAVFWQEISEIFRQLQKQAAEIYNQSLIELYYEIFIKGKGIANASSVEHYLSDVCYTRAAELFKNAAIASGLRSKIKSNFRLKELKNMKSGLPTTKSDNFPIPLVKQKGGQYTGFEISNHNSDFIIKIPFGRWQVKKEIDKYRPWEKFDFEQVQKSPKPISLLLSTQRRKRNKGWSKDEGTEAEIKKVMNGDYQTSYIEVKRGSKIGEKSAWMLNLSIDVPKIDKGVDPSIIGGIAVGVKSPLVCAINNAFSRYSISDNDLFHFNKKMFARRRILLKKNRHKRAGHGAKNKLKPITILTEKSERFRKKLIERWACEIADFFIKNKVGTVQMENLESMKRKEDSYFNIRLRGFWPYAEMQNKIEFKLKQYGIEIRKVAPNNTSKTCSKCGHLNNYFNFEYRKKNKFPHFKCEKCNFKENADYNAALNISNPKLKSTKEEPSGGSSGGSSGSETPGTSESATPESMSEVEFSHEYWMRHALTLAKRAWDEREVPVGAVLVHNNRVIGEGWNRPIGRHDPTAHAEIMALRQGGLVMQNYRLIDATLYVTLEPCVMCAGAMIHSRIGRVVFGARDAKTGAAGSLMDVLHHPGMNHRVEITEGILADECAALLSDFFRMRRQEIKAQKKAQSSTDSGGSSGGSSGSETPGTSESATPESSGGSSGGSMSEVEFSHEYWMRHALTLAKRARDEREVPVGAVLVLNNRVIGEGWNRAIGLHDPTAHAEIMALRQGGLVMQNYRLIDATLYVTFEPCVMCAGAMIHSRIGRVVFGWRQSKRGAAGSLMNVLNYPGMNHRVEITEGILADECAALLCDFYRMPRQVFNAQKKAQSSINKRPAATKKAGQAKKKK

SEQ ID NO: 431 - protein, 967 aa, synthetic construct
  REGION 1..967: note = dTnpB(D354A)-28aa-ABE-C3.1
MGEKSSRRRRNGKSGAWTAAITSCVGGKMAKNTITKTLKLRIVRPYNSAEVEKIVADEKNNREKIALEKNKDKVKEACSKHLKVAAYCTTQVERNACLFCKARKLDDKFYQKLRGQFPDAVFWQEISEIFRQLQKQAAEIYNQSLIELYYEIFIKGKGIANASSVEHYLSDVCYTRAAELFKNAAIASGLRSKIKSNFRLKELKNMKSGLPTTKSDNFPIPLVKQKGGQYTGFEISNHNSDFIIKIPFGRWQVKKEIDKYRPWEKFDFEQVQKSPKPISLLLSTQRRKRNKGWSKDEGTEAEIKKVMNGDYQTSYIEVKRGSKIGEKSAWMLNLSIDVPKIDKGVDPSIIGGIAVGVKSPLVCAINNAFSRYSISDNDLFHFNKKMFARRRILLKKNRHKRAGHGAKNKLKPITILTEKSERFRKKLIERWACEIADFFIKNKVGTVQMENLESMKRKEDSYFNIRLRGFWPYAEMQNKIEFKLKQYGIEIRKVAPNNTSKTCSKCGHLNNYFNFEYRKKNKFPHFKCEKCNFKENADYNAALNISNPKLKSTKEEPSGGSSGGSSGSETPGTSESATPESSGGSMSEVEFSHEYWMRHALTLAKRAWDEREVPVGAVLVHNNRVIGEGWNRPIGRHDPTAHAEIMALRQGGLVMQNYRLIDATLYVTLEPCVMCAGAMIHSRIGRVVFGARDAKTGAAGSLMDVLHHPGMNHRVEITEGILADECAALLSDFFRMRRQEIKAQKKAQSSTDSGGSSGGSSGSETPGTSESATPESSGGSSGGSMSEVEFSHEYWMRHALTLAKRARDEREVPVGAVLVLNNRVIGEGWNRAIGLHDPTAHAEIMALRQGGLVMQNYRLIDATLYVTFEPCVMCAGAMIHSRIGRVVFGWRQSKRGAAGSLMNVLNYPGMNHRVEITEGILADECAALLCDFYRMPRQVFNAQKKAQSSINKRPAATKKAGQAKKKK

SEQ ID NO: 432 - protein, 975 aa, synthetic construct
  REGION 1..975: note = dTnpB(D354A)-36aa-ABE-C3.1
MGEKSSRRRRNGKSGAWTAAITSCVGGKMAKNTITKTLKLRIVRPYNSAEVEKIVADEKNNREKIALEKNKDKVKEACSKHLKVAAYCTTQVERNACLFCKARKLDDKFYQKLRGQFPDAVFWQEISEIFRQLQKQAAEIYNQSLIELYYEIFIKGKGIANASSVEHYLSDVCYTRAAELFKNAAIASGLRSKIKSNFRLKELKNMKSGLPTTKSDNFPIPLVKQKGGQYTGFEISNHNSDFIIKIPFGRWQVKKEIDKYRPWEKFDFEQVQKSPKPISLLLSTQRRKRNKGWSKDEGTEAEIKKVMNGDYQTSYIEVKRGSKIGEKSAWMLNLSIDVPKIDKGVDPSIIGGIAVGVKSPLVCAINNAFSRYSISDNDLFHFNKKMFARRRILLKKNRHKRAGHGAKNKLKPITILTEKSERFRKKLIERWACEIADFFIKNKVGTVQMENLESMKRKEDSYFNIRLRGFWPYAEMQNKIEFKLKQYGIEIRKVAPNNTSKTCSKCGHLNNYFNFEYRKKNKFPHFKCEKCNFKENADYNAALNISNPKLKSTKEEPSGGSSGGSSGSETPGTSESATPESSGGSSGGSSGSEMSEVEFSHEYWMRHALTLAKRAWDEREVPVGAVLVHNNRVIGEGWNRPIGRHDPTAHAEIMALRQGGLVMQNYRLIDATLYVTLEPCVMCAGAMIHSRIGRVVFGARDAKTGAAGSLMDVLHHPGMNHRVEITEGILADECAALLSDFFRMRRQEIKAQKKAQSSTDSGGSSGGSSGSETPGTSESATPESSGGSSGGSMSEVEFSHEYWMRHALTLAKRARDEREVPVGAVLVLNNRVIGEGWNRAIGLHDPTAHAEIMALRQGGLVMQNYRLIDATLYVTFEPCVMCAGAMIHSRIGRVVFGWRQSKRGAAGSLMNVLNYPGMNHRVEITEGILADECAALLCDFYRMPRQVFNAQKKAQSSINKRPAATKKAGQAKKKK

SEQ ID NO: 433 - protein, 979 aa, synthetic construct
  REGION 1..979: note = dTnpB(D354A)-40aa-ABE-C3.1
MGEKSSRRRRNGKSGAWTAAITSCVGGKMAKNTITKTLKLRIVRPYNSAEVEKIVADEKNNREKIALEKNKDKVKEACSKHLKVAAYCTTQVERNACLFCKARKLDDKFYQKLRGQFPDAVFWQEISEIFRQLQKQAAEIYNQSLIELYYEIFIKGKGIANASSVEHYLSDVCYTRAAELFKNAAIASGLRSKIKSNFRLKELKNMKSGLPTTKSDNFPIPLVKQKGGQYTGFEISNHNSDFIIKIPFGRWQVKKEIDKYRPWEKFDFEQVQKSPKPISLLLSTQRRKRNKGWSKDEGTEAEIKKVMNGDYQTSYIEVKRGSKIGEKSAWMLNLSIDVPKIDKGVDPSIIGGIAVGVKSPLVCAINNAFSRYSISDNDLFHFNKKMFARRRILLKKNRHKRAGHGAKNKLKPITILTEKSERFRKKLIERWACEIADFFIKNKVGTVQMENLESMKRKEDSYFNIRLRGFWPYAEMQNKIEFKLKQYGIEIRKVAPNNTSKTCSKCGHLNNYFNFEYRKKNKFPHFKCEKCNFKENADYNAALNISNPKLKSTKEEPSGGSSGGSSGSETPGTSESATPESSGGSSGGSSGSETPGTMSEVEFSHEYWMRHALTLAKRAWDEREVPVGAVLVHNNRVIGEGWNRPIGRHDPTAHAEIMALRQGGLVMQNYRLIDATLYVTLEPCVMCAGAMIHSRIGRVVFGARDAKTGAAGSLMDVLHHPGMNHRVEITEGILADECAALLSDFFRMRRQEIKAQKKAQSSTDSGGSSGGSSGSETPGTSESATPESSGGSSGGSMSEVEFSHEYWMRHALTLAKRARDEREVPVGAVLVLNNRVIGEGWNRAIGLHDPTAHAEIMALRQGGLVMQNYRLIDATLYVTFEPCVMCAGAMIHSRIGRVVFGWRQSKRGAAGSLMNVLNYPGMNHRVEITEGILADECAALLCDFYRMPRQVFNAQKKAQSSINKRPAATKKAGQAKKKK

SEQ ID NO: 434 - protein, 921 aa, synthetic construct
  REGION 1..921: note = dCas12f1(D326A)-10aa-ABE-C2
MAKNTITKTLKLRIVRPYNSAEVEKIVADEKNNREKIALEKNKDKVKEACSKHLKVAAYCTTQVERNACLFCKARKLDDKFYQKLRGQFPDAVFWQEISEIFRQLQKQAAEIYNQSLIELYYEIFIKGKGIANASSVEHYLSDVCYTRAAELFKNAAIASGLRSKIKSNFRLKELKNMKSGLPTTKSDNFPIPLVKQKGGQYTGFEISNHNSDFIIKIPFGRWQVKKEIDKYRPWEKFDFEQVQKSPKPISLLLSTQRRKRNKGWSKDEGTEAEIKKVMNGDYQTSYIEVKRGSKIGEKSAWMLNLSIDVPKIDKGVDPSIIGGIAVGVKSPLVCAINNAFSRYSISDNDLFHFNKKMFARRRILLKKNRHKRAGHGAKNKLKPITILTEKSERFRKKLIERWACEIADFFIKNKVGTVQMENLESMKRKEDSYFNIRLRGFWPYAEMQNKIEFKLKQYGIEIRKVAPNNTSKTCSKCGHLNNYFNFEYRKKNKFPHFKCEKCNFKENADYNAALNISNPKLKSTKEEPSGGSSGGSSGMSEVEFSHEYWMRHALTLAKRAWDEREVPVGAVLVHNNRVIGEGWNRPIGRHDPTAHAEIMALRQGGLVMQNYRLIDATLYVTLEPCVMCAGAMIHSRIGRVVFGARDAKTGAAGSLMDVLHHPGMNHRVEITEGILADECAALLSDFFRMRRQEIKAQKKAQSSTDSGGSSGGSSGSETPGTSESATPESSGGSSGGSMSEVEFSHEYWMRHALTLAKRARDEREVPVGAVLVLNNRVIGEGWNRAIGLHDPTAHAEIMALRQGGLVMQNYRLIDATLYVTFEPCVMCAGAMIHSRIGRVVFGVRNAKTGAAGSLMDVLHYPGMNHRVEITEGILADECAALLCYFFRMPRQVFNAQKKAQSSTDKRPAATKKAGQAKKKK

SEQ ID NO: 435 - protein, 925 aa, synthetic construct
  REGION 1..925: note = dCas12f1(D326A)-14aa-ABE-C2
MAKNTITKTLKLRIVRPYNSAEVEKIVADEKNNREKIALEKNKDKVKEACSKHLKVAAYCTTQVERNACLFCKARKLDDKFYQKLRGQFPDAVFWQEISEIFRQLQKQAAEIYNQSLIELYYEIFIKGKGIANASSVEHYLSDVCYTRAAELFKNAAIASGLRSKIKSNFRLKELKNMKSGLPTTKSDNFPIPLVKQKGGQYTGFEISNHNSDFIIKIPFGRWQVKKEIDKYRPWEKFDFEQVQKSPKPISLLLSTQRRKRNKGWSKDEGTEAEIKKVMNGDYQTSYIEVKRGSKIGEKSAWMLNLSIDVPKIDKGVDPSIIGGIAVGVKSPLVCAINNAFSRYSISDNDLFHFNKKMFARRRILLKKNRHKRAGHGAKNKLKPITILTEKSERFRKKLIERWACEIADFFIKNKVGTVQMENLESMKRKEDSYFNIRLRGFWPYAEMQNKIEFKLKQYGIEIRKVAPNNTSKTCSKCGHLNNYFNFEYRKKNKFPHFKCEKCNFKENADYNAALNISNPKLKSTKEEPSGGSSGGSSGSETPMSEVEFSHEYWMRHALTLAKRAWDEREVPVGAVLVHNNRVIGEGWNRPIGRHDPTAHAEIMALRQGGLVMQNYRLIDATLYVTLEPCVMCAGAMIHSRIGRVVFGARDAKTGAAGSLMDVLHHPGMNHRVEITEGILADECAALLSDFFRMRRQEIKAQKKAQSSTDSGGSSGGSSGSETPGTSESATPESSGGSSGGSMSEVEFSHEYWMRHALTLAKRARDEREVPVGAVLVLNNRVIGEGWNRAIGLHDPTAHAEIMALRQGGLVMQNYRLIDATLYVTFEPCVMCAGAMIHSRIGRVVFGVRNAKTGAAGSLMDVLHYPGMNHRVEITEGILADECAALLCYFFRMPRQVFNAQKKAQSSTDKRPAATKKAGQAKKKK

SEQ ID NO: 436 - protein, 927 aa, synthetic construct
  REGION 1..927: note = dCas12f1(D326A)-16aa-ABE-C2
MAKNTITKTLKLRIVRPYNSAEVEKIVADEKNNREKIALEKNKDKVKEACSKHLKVAAYCTTQVERNACLFCKARKLDDKFYQKLRGQFPDAVFWQEISEIFRQLQKQAAEIYNQSLIELYYEIFIKGKGIANASSVEHYLSDVCYTRAAELFKNAAIASGLRSKIKSNFRLKELKNMKSGLPTTKSDNFPIPLVKQKGGQYTGFEISNHNSDFIIKIPFGRWQVKKEIDKYRPWEKFDFEQVQKSPKPISLLLSTQRRKRNKGWSKDEGTEAEIKKVMNGDYQTSYIEVKRGSKIGEKSAWMLNLSIDVPKIDKGVDPSIIGGIAVGVKSPLVCAINNAFSRYSISDNDLFHFNKKMFARRRILLKKNRHKRAGHGAKNKLKPITILTEKSERFRKKLIERWACEIADFFIKNKVGTVQMENLESMKRKEDSYFNIRLRGFWPYAEMQNKIEFKLKQYGIEIRKVAPNNTSKTCSKCGHLNNYFNFEYRKKNKFPHFKCEKCNFKENADYNAALNISNPKLKSTKEEPSGGSSGGSSGSETPGTMSEVEFSHEYWMRHALTLAKRAWDEREVPVGAVLVHNNRVIGEGWNRPIGRHDPTAHAEIMALRQGGLVMQNYRLIDATLYVTLEPCVMCAGAMIHSRIGRVVFGARDAKTGAAGSLMDVLHHPGMNHRVEITEGILADECAALLSDFFRMRRQEIKAQKKAQSSTDSGGSSGGSSGSETPGTSESATPESSGGSSGGSMSEVEFSHEYWMRHALTLAKRARDEREVPVGAVLVLNNRVIGEGWNRAIGLHDPTAHAEIMALRQGGLVMQNYRLIDATLYVTFEPCVMCAGAMIHSRIGRVVFGVRNAKTGAAGSLMDVLHYPGMNHRVEITEGILADECAALLCYFFRMPRQVFNAQKKAQSSTDKRPAATKKAGQAKKKK

SEQ ID NO: 437 - protein, 931 aa, synthetic construct
  REGION 1..931: note = dCas12f1(D326A)-20aa-ABE-C2
MAKNTITKTLKLRIVRPYNSAEVEKIVADEKNNREKIALEKNKDKVKEACSKHLKVAAYCTTQVERNACLFCKARKLDDKFYQKLRGQFPDAVFWQEISEIFRQLQKQAAEIYNQSLIELYYEIFIKGKGIANASSVEHYLSDVCYTRAAELFKNAAIASGLRSKIKSNFRLKELKNMKSGLPTTKSDNFPIPLVKQKGGQYTGFEISNHNSDFIIKIPFGRWQVKKEIDKYRPWEKFDFEQVQKSPKPISLLLSTQRRKRNKGWSKDEGTEAEIKKVMNGDYQTSYIEVKRGSKIGEKSAWMLNLSIDVPKIDKGVDPSIIGGIAVGVKSPLVCAINNAFSRYSISDNDLFHFNKKMFARRRILLKKNRHKRAGHGAKNKLKPITILTEKSERFRKKLIERWACEIADFFIKNKVGTVQMENLESMKRKEDSYFNIRLRGFWPYAEMQNKIEFKLKQYGIEIRKVAPNNTSKTCSKCGHLNNYFNFEYRKKNKFPHFKCEKCNFKENADYNAALNISNPKLKSTKEEPSGGSSGGSSGSETPGTSESAMSEVEFSHEYWMRHALTLAKRAWDEREVPVGAVLVHNNRVIGEGWNRPIGRHDPTAHAEIMALRQGGLVMQNYRLIDATLYVTLEPCVMCAGAMIHSRIGRVVFGARDAKTGAAGSLMDVLHHPGMNHRVEITEGILADECAALLSDFFRMRRQEIKAQKKAQSSTDSGGSSGGSSGSETPGTSESATPESSGGSSGGSMSEVEFSHEYWMRHALTLAKRARDEREVPVGAVLVLNNRVIGEGWNRAIGLHDPTAHAEIMALRQGGLVMQNYRLIDATLYVTFEPCVMCAGAMIHSRIGRVVFGVRNAKTGAAGSLMDVLHYPGMNHRVEITEGILADECAALLCYFFRMPRQVFNAQKKAQSSTDKRPAATKKAGQAKKKK

SEQ ID NO: 438 - protein, 935 aa, synthetic construct
  REGION 1..935: note = dCas12f1(D326A)-24aa-ABE-C2
MAKNTITKTLKLRIVRPYNSAEVEKIVADEKNNREKIALEKNKDKVKEACSKHLKVAAYCTTQVERNACLFCKARKLDDKFYQKLRGQFPDAVFWQEISEIFRQLQKQAAEIYNQSLIELYYEIFIKGKGIANASSVEHYLSDVCYTRAAELFKNAAIASGLRSKIKSNFRLKELKNMKSGLPTTKSDNFPIPLVKQKGGQYTGFEISNHNSDFIIKIPFGRWQVKKEIDKYRPWEKFDFEQVQKSPKPISLLLSTQRRKRNKGWSKDEGTEAEIKKVMNGDYQTSYIEVKRGSKIGEKSAWMLNLSIDVPKIDKGVDPSIIGGIAVGVKSPLVCAINNAFSRYSISDNDLFHFNKKMFARRRILLKKNRHKRAGHGAKNKLKPITILTEKSERFRKKLIERWACEIADFFIKNKVGTVQMENLESMKRKEDSYFNIRLRGFWPYAEMQNKIEFKLKQYGIEIRKVAPNNTSKTCSKCGHLNNYFNFEYRKKNKFPHFKCEKCNFKENADYNAALNISNPKLKSTKEEPSGGSSGGSSGSETPGTSESATPESMSEVEFSHEYWMRHALTLAKRAWDEREVPVGAVLVHNNRVIGEGWNRPIGRHDPTAHAEIMALRQGGLVMQNYRLIDATLYVTLEPCVMCAGAMIHSRIGRVVFGARDAKTGAAGSLMDVLHHPGMNHRVEITEGILADECAALLSDFFRMRRQEIKAQKKAQSSTDSGGSSGGSSGSETPGTSESATPESSGGSSGGSMSEVEFSHEYWMRHALTLAKRARDEREVPVGAVLVLNNRVIGEGWNRAIGLHDPTAHAEIMALRQGGLVMQNYRLIDATLYVTFEPCVMCAGAMIHSRIGRVVFGVRNAKTGAAGSLMDVLHYPGMNHRVEITEGILADECAALLCYFFRMPRQVFNAQKKAQSSTDKRPAATKKAGQAKKKK

SEQ ID NO: 439 - protein, 939 aa, synthetic construct
  REGION 1..939: note = dCas12f1(D326A)-28aa-ABE-C2
MAKNTITKTLKLRIVRPYNSAEVEKIVADEKNNREKIALEKNKDKVKEACSKHLKVAAYCTTQVERNACLFCKARKLDDKFYQKLRGQFPDAVFWQEISEIFRQLQKQAAEIYNQSLIELYYEIFIKGKGIANASSVEHYLSDVCYTRAAELFKNAAIASGLRSKIKSNFRLKELKNMKSGLPTTKSDNFPIPLVKQKGGQYTGFEISNHNSDFIIKIPFGRWQVKKEIDKYRPWEKFDFEQVQKSPKPISLLLSTQRRKRNKGWSKDEGTEAEIKKVMNGDYQTSYIEVKRGSKIGEKSAWMLNLSIDVPKIDKGVDPSIIGGIAVGVKSPLVCAINNAFSRYSISDNDLFHFNKKMFARRRILLKKNRHKRAGHGAKNKLKPITILTEKSERFRKKLIERWACEIADFFIKNKVGTVQMENLESMKRKEDSYFNIRLRGFWPYAEMQNKIEFKLKQYGIEIRKVAPNNTSKTCSKCGHLNNYFNFEYRKKNKFPHFKCEKCNFKENADYNAALNISNPKLKSTKEEPSGGSSGGSSGSETPGTSESATPESSGGSMSEVEFSHEYWMRHALTLAKRAWDEREVPVGAVLVHNNRVIGEGWNRPIGRHDPTAHAEIMALRQGGLVMQNYRLIDATLYVTLEPCVMCAGAMIHSRIGRVVFGARDAKTGAAGSLMDVLHHPGMNHRVEITEGILADECAALLSDFFRMRRQEIKAQKKAQSSTDSGGSSGGSSGSETPGTSESATPESSGGSSGGSMSEVEFSHEYWMRHALTLAKRARDEREVPVGAVLVLNNRVIGEGWNRAIGLHDPTAHAEIMALRQGGLVMQNYRLIDATLYVTFEPCVMCAGAMIHSRIGRVVFGVRNAKTGAAGSLMDVLHYPGMNHRVEITEGILADECAALLCYFFRMPRQVFNAQKKAQSSTDKRPAATKKAGQAKKKK

SEQ ID NO: 440 - protein, 947 aa, synthetic construct
  REGION 1..947: note = dCas12f1(D326A)-36aa-ABE-C2
MAKNTITKTLKLRIVRPYNSAEVEKIVADEKNNREKIALEKNKDKVKEACSKHLKVAAYCTTQVERNACLFCKARKLDDKFYQKLRGQFPDAVFWQEISEIFRQLQKQAAEIYNQSLIELYYEIFIKGKGIANASSVEHYLSDVCYTRAAELFKNAAIASGLRSKIKSNFRLKELKNMKSGLPTTKSDNFPIPLVKQKGGQYTGFEISNHNSDFIIKIPFGRWQVKKEIDKYRPWEKFDFEQVQKSPKPISLLLSTQRRKRNKGWSKDEGTEAEIKKVMNGDYQTSYIEVKRGSKIGEKSAWMLNLSIDVPKIDKGVDPSIIGGIAVGVKSPLVCAINNAFSRYSISDNDLFHFNKKMFARRRILLKKNRHKRAGHGAKNKLKPITILTEKSERFRKKLIERWACEIADFFIKNKVGTVQMENLESMKRKEDSYFNIRLRGFWPYAEMQNKIEFKLKQYGIEIRKVAPNNTSKTCSKCGHLNNYFNFEYRKKNKFPHFKCEKCNFKENADYNAALNISNPKLKSTKEEPSGGSSGGSSGSETPGTSESATPESSGGSSGGSSGSEMSEVEFSHEYWMRHALTLAKRAWDEREVPVGAVLVHNNRVIGEGWNRPIGRHDPTAHAEIMALRQGGLVMQNYRLIDATLYVTLEPCVMCAGAMIHSRIGRVVFGARDAKTGAAGSLMDVLHHPGMNHRVEITEGILADECAALLSDFFRMRRQEIKAQKKAQSSTDSGGSSGGSSGSETPGTSESATPESSGGSSGGSMSEVEFSHEYWMRHALTLAKRARDEREVPVGAVLVLNNRVIGEGWNRAIGLHDPTAHAEIMALRQGGLVMQNYRLIDATLYVTFEPCVMCAGAMIHSRIGRVVFGVRNAKTGAAGSLMDVLHYPGMNHRVEITEGILADECAALLCYFFRMPRQVFNAQKKAQSSTDKRPAATKKAGQAKKKK

SEQ ID NO: 441 - protein, 951 aa, synthetic construct
  REGION 1..951: note = dCas12f1(D326A)-40aa-ABE-C2
MAKNTITKTLKLRIVRPYNSAEVEKIVADEKNNREKIALEKNKDKVKEACSKHLKVAAYCTTQVERNACLFCKARKLDDKFYQKLRGQFPDAVFWQEISEIFRQLQKQAAEIYNQSLIELYYEIFIKGKGIANASSVEHYLSDVCYTRAAELFKNAAIASGLRSKIKSNFRLKELKNMKSGLPTTKSDNFPIPLVKQKGGQYTGFEISNHNSDFIIKIPFGRWQVKKEIDKYRPWEKFDFEQVQKSPKPISLLLSTQRRKRNKGWSKDEGTEAEIKKVMNGDYQTSYIEVKRGSKIGEKSAWMLNLSIDVPKIDKGVDPSIIGGIAVGVKSPLVCAINNAFSRYSISDNDLFHFNKKMFARRRILLKKNRHKRAGHGAKNKLKPITILTEKSERFRKKLIERWACEIADFFIKNKVGTVQMENLESMKRKEDSYFNIRLRGFWPYAEMQNKIEFKLKQYGIEIRKVAPNNTSKTCSKCGHLNNYFNFEYRKKNKFPHFKCEKCNFKENADYNAALNISNPKLKSTKEEPSGGSSGGSSGSETPGTSESATPESSGGSSGGSSGSETPGTMSEVEFSHEYWMRHALTLAKRAWDEREVPVGAVLVHNNRVIGEGWNRPIGRHDPTAHAEIMALRQGGLVMQNYRLIDATLYVTLEPCVMCAGAMIHSRIGRVVFGARDAKTGAAGSLMDVLHHPGMNHRVEITEGILADECAALLSDFFRMRRQEIKAQKKAQSSTDSGGSSGGSSGSETPGTSESATPESSGGSSGGSMSEVEFSHEYWMRHALTLAKRARDEREVPVGAVLVLNNRVIGEGWNRAIGLHDPTAHAEIMALRQGGLVMQNYRLIDATLYVTFEPCVMCAGAMIHSRIGRVVFGVRNAKTGAAGSLMDVLHYPGMNHRVEITEGILADECAALLCYFFRMPRQVFNAQKKAQSSTDKRPAATKKAGQAKKKK

SEQ ID NO: 442 - protein, 971 aa, synthetic construct
  REGION 1..971: note = dCas12f1 variant 1(D538A, I159W)-TadAeTadA3
MGEKSSRRRRNGKSGAWTAAITSCVGGKMAKNTITKTLKLRIVRPYNSAEVEKIVADEKNNREKIALEKNKDKVKEACSKHLKVAAYCTTQVERNACLFCKARKLDDKFYQKLRGQFPDAVFWQEISEIFRQLQKQAAEIYNQSLIELYYEIFIKGKGWANASSVEHYLSDVCYTRAAELFKNAAIASGLRSKIKSNFRLKELKNMKSGLPTTKSDNFPIPLVKQKGGQYTGFEISNHNSDFIIKIPFGRWQVKKEIDKYRPWEKFDFEQVQKSPKPISLLLSTQRRKRNKGWSKDEGTEAEIKKVMNGDYQTSYIEVKRGSKIGEKSAWMLNLSIDVPKIDKGVDPSIIGGIDVGVKSPLVCAINNAFSRYSISDNDLFHFNKKMFARRRILLKKNRHKRAGHGAKNKLKPITILTEKSERFRKKLIERWACEIADFFIKNKVGTVQMENLESMKRKEDSYFNIRLRGFWPYAEMQNKIEFKLKQYGIEIRKVAPNNTSKTCSKCGHLNNYFNFEYRKKNKFPHFKCEKCNFKENAAYNAALNISNPKLKSTKEEPSGGSSGGSSGSETPGTSESATPESSGGSSGGSMSEVEFSHEYWMRHALTLAKRAWDEREVPVGAVLVHNNRVIGEGWNRPIGRHDPTAHAEIMALRQGGLVMQNYRLIDATLYVTLEPCVMCAGAMIHSRIGRVVFGARDAKTGAAGSLMDVLHHPGMNHRVEITEGILADECAALLSDFFRMRRQEIKAQKKAQSSTDSGGSSGGSSGSETPGTSESATPESSGGSSGGSMSEVEFSHEYWMRHALTLAKRARDEREVPVGAVLVLNNRVIGEGWNRAIGLHDPTAHAEIMALRQGGLVMQNYRLIDATLYVTFEPCVMCAGAMIHSRIGRVVFGWRQSKRGAAGSLMNVLNYPGMNHRVEITEGILADECAALLCDFYRMPRQVFNAQKKAQSSINKRPAATKKAGQAKKKK

SEQ ID NO: 443 - DNA, 22 bp, synthetic construct
  misc_feature 1..22: note = target gene's protospacer sequence
  source 1..22: mol_type = other DNA
ctagcacacactgggcagagtg

SEQ ID NO: 444 - DNA, 26 bp, synthetic construct
  misc_feature 1..26: note = target gene's protospacer sequence with PAM in 5'
  source 1..26: mol_type = other DNA
tttgctagcacacactgggcagagtg

SEQ ID NO: 445 - DNA, 20 bp, synthetic construct
  misc_feature 1..20: note = spacer sequence for experimental example 4.1
  source 1..20: mol_type = other DNA
atcagataggatcgtccgat

SEQ ID NO: 446 - DNA, 20 bp, synthetic construct
  misc_feature 1..20: note = spacer sequence for experimental example 4.1
  source 1..20: mol_type = other DNA
gggagggcgaggccgaaacc

SEQ ID NO: 447 - DNA, 20 bp, synthetic construct
  misc_feature 1..20: note = spacer sequence for experimental example 4.1
  source 1..20: mol_type = other DNA
ggagttttttcttccctctg

SEQ ID NO: 448 - DNA, 20 bp, synthetic construct
  misc_feature 1..20: note = spacer sequence for experimental example 4.1
  source 1..20: mol_type = other DNA
gaaggctgccaggttaaggc

SEQ ID NO: 449 - DNA, 20 bp, synthetic construct
  misc_feature 1..20: note = spacer sequence for experimental example 4.1
  source 1..20: mol_type = other DNA
tgcaccctgcacactgacct

SEQ ID NO: 450 - DNA, 20 bp, synthetic construct
  misc_feature 1..20: note = protospacer sequence for experimental example 4.2
  source 1..20: mol_type = other DNA
ttgcccagactggagtgcag

SEQ ID NO: 451 - DNA, 20 bp, synthetic construct
  misc_feature 1..20: note = protospacer sequence for experimental example 4.2
  source 1..20: mol_type = other DNA
gcccagtagatcgaggctac

SEQ ID NO: 452 - DNA, 20 bp, synthetic construct
  misc_feature 1..20: note = protospacer sequence for experimental example 4.2
  source 1..20: mol_type = other DNA
cctaatggtggtggcaatgg

SEQ ID NO: 453 - DNA, 21 bp, synthetic construct
  misc_feature 1..21: note = protospacer sequence for experimental example 4.2
  source 1..21: mol_type = other DNA
agacagggtctcactttgttg

SEQ ID NO: 454 - DNA, 20 bp, synthetic construct
  misc_feature 1..20: note = protospacer sequence for experimental example 4.2
  source 1..20: mol_type = other DNA
ttgcccagactggagtgcag

SEQ ID NO: 455 - DNA, 20 bp, synthetic construct
  misc_feature 1..20: note = protospacer sequence for experimental example 4.2
  source 1..20: mol_type = other DNA
gcccagtagatcgaggctac

SEQ ID NO: 456 - DNA, 20 bp, synthetic construct
  misc_feature 1..20: note = protospacer sequence for experimental example 4.2
  source 1..20: mol_type = other DNA
cctaatggtggtggcaatgg

SEQ ID NO: 457 - DNA, 21 bp, synthetic construct
  misc_feature 1..21: note = protospacer sequence for experimental example 4.2
  source 1..21: mol_type = other DNA
agacagggtctcactttgttg

SEQ ID NO: 458 - DNA, 22 bp, synthetic construct
  misc_feature 1..22: note = 18s_rRNA_F
  source 1..22: mol_type = other DNA
tcaactttcgatggtagtcgcc

SEQ ID NO: 459 - DNA, 24 bp, synthetic construct
  misc_feature 1..24: note = 18s_rRNA_R
  source 1..24: mol_type = other DNA
ggcctcgaaagagtcctgtattgt

SEQ ID NO: 460 - DNA, 1628 bp, synthetic construct
  misc_feature 1..1628: note = Cas12f1 Wild-type codon
  source 1..1628: mol_type = other DNA
atgccaaagaagaagcggaaagtcgccaagaacacaattacaaagacactgaagctgaggatcgtgagaccatacaacagcgctgaggtcgagaagattgtggctgatgaaaagaacaacagggaaaagatcgccctcgagaagaacaaggataaggtgaaggaggcctgctctaagcacctgaaagtggccgcctactgcaccacacaggtggagaggaacgcctgtctgttttgtaaagctcggaagctggatgataagttttaccagaagctgcggggccagttccccgatgccgtcttttggcaggagattagcgagatcttcagacagctgcagaagcaggccgccgagatctacaaccagagcctgatcgagctctactacgagatcttcatcaagggcaagggcattgccaacgcctcctccgtggagcactacctgagcgacgtgtgctacacaagagccgccgagctctttaagaacgccgctatcgcttccgggctgaggagcaagattaagagtaacttccggctcaaggagctgaagaacatgaagagcggcctgcccactacaaagagcgacaacttcccaattccactggtgaagcagaaggggggccagtacacagggttcgagatttccaaccacaacagcgactttattattaagatcccctttggcaggtggcaggtcaagaaggagattgacaagtacaggccctgggagaagtttgatttcgagcaggtgcagaagagccccaagcctatttccctgctgctgtccacacagcggcggaagaggaacaaggggtggtctaaggatgaggggaccgaggccgagattaagaaagtgatgaacggcgactaccagacaagctacatcgaggtcaagcggggcagtaagattggcgagaagagcgcctggatgctgaacctgagcattgacgtgccaaagattgataagggcgtggatcccagcatcatcggagggatcgatgtgggggtcaagagccccctcgtgtgcgccatcaacaacgccttcagcaggtacagcatctccgataacgacctgttccactttaacaagaagatgttcgcccggcggaggattttgctcaagaagaaccggcacaagcgggccggacacggggccaagaacaagctcaagcccatcactatcctgaccgagaagagcgagaggttcaggaagaagctcatcgagagatgggcctgcgagatcgccgatttctttattaagaacaaggtcggaacagtgcagatggagaacctcgagagcatgaagaggaaggaggattcctacttcaacattcggctgagggggttctggccctacgctgagatgcagaacaagattgagtttaagctgaagcagtacgggattgagatccggaaggtggcccccaacaacaccagcaagacctgcagcaagtgcgggcacctcaacaactacttcaacttcgagtaccggaagaagaacaagttcccacacttcaagtgcgagaagtgcaactttaaggagaacgccgattacaacgccgccctgaacatcagcaaccctaagctgaagagcactaaggaggagccccaaagaagaagcggaaagtc

SEQ ID NO: 461 - protein, 83 aa, synthetic construct
  REGION 1..83: note = uracil glycosylase inhibitor(UGI)
TNLSDIIEKETGKQLVIQESILMLPEEVEEVIGNKPESDILVHTAYDESTDENVMLLTSDAPEYKPWALVIQDSNGENKIKML

SEQ ID NO: 462 - DNA, 22 bp, synthetic construct
  misc_feature 1..22: note = dCas9_KRAB_R
  source 1..22: mol_type = other DNA
aagggttcgatcctctagagtc

SEQ ID NO: 463 - DNA, 18 bp, synthetic construct
  misc_feature 1..18: note = dCas9_KRAB_F
  source 1..18: mol_type = other DNA
agtggtggaggaagtggc

SEQ ID NO: 464 - DNA, 61 bp, synthetic construct
  misc_feature 1..61: note = NLS_dCas14_KRAB_F
  source 1..61: mol_type = other DNA
gatccagcctccggactctagaggatcgaacccttgccaccatggccccaaagaagaagcg

SEQ ID NO: 465 - DNA, 60 bp, synthetic construct
  misc_feature 1..60: note = NLS_dCas14_KRAB_R
  source 1..60: mol_type = other DNA
tcgcgtccatcgaccctgacccgccacttcctccaccactctttttcttttttgcctggc

SEQ ID NO: 466 - DNA, 22 bp, synthetic construct
  misc_feature 1..22: note = dCas9_KRAB_R
  source 1..22: mol_type = other DNA
aagggttcgatcctctagagtc

SEQ ID NO: 467 - DNA, 18 bp, synthetic construct
  misc_feature 1..18: note = dCas9_KRAB_F
  source 1..18: mol_type = other DNA
agtggtggaggaagtggc

SEQ ID NO: 468 - DNA, 60 bp, synthetic construct
  misc_feature 1..60: note = NLS_KRAB_dCas14_Gib_F
  source 1..60: mol_type = other DNA
gcggcggttctggtggctcaggcggcagcggccggccaccaaagaagaagcggaaggtcg

SEQ ID NO: 469 - DNA, 60 bp, synthetic construct
  misc_feature 1..60: note = NLS_KRAB_dCas14_Gib_R
  source 1..60: mol_type = other DNA
tttaaactcattactaaccggtagggatcgaaccctttcactttttcttttttgcctggc

SEQ ID NO: 470 - DNA, 22 bp, synthetic construct
  misc_feature 1..22: note = dCas9_KRAB_R
  source 1..22: mol_type = other DNA
aagggttcgatcctctagagtc

SEQ ID NO: 471 - DNA, 18 bp, synthetic construct
  misc_feature 1..18: note = dCas9_KRAB_F
  source 1..18: mol_type = other DNA
agtggtggaggaagtggc

SEQ ID NO: 472 - DNA, 61 bp, synthetic construct; identical to SEQ ID NO: 464
  misc_feature 1..61: note = NLS_dCas14_KRAB_F
  source 1..61: mol_type = other DNA

SEQ ID NO: 473 - DNA, 60 bp, synthetic construct; identical to SEQ ID NO: 465
  misc_feature 1..60: note = NLS_dCas14_KRAB_R
  source 1..60: mol_type = other DNA

SEQ ID NO: 474 - DNA, 20 bp, synthetic construct
  misc_feature 1..20: note = KRAB_MeCP2_dCas12f1_KRAB_Vector_R
  source 1..20: mol_type = other DNA
ggccatggtggcaagggttc

SEQ ID NO: 475 - DNA, 21 bp, synthetic construct
  misc_feature 1..21: note = KRAB_MeCP2_dCas12f1_KRAB_Vector_F
  source 1..21: mol_type = other DNA
ccaaagaagaagcggaaggtc

SEQ ID NO: 476 - DNA, 60 bp, synthetic construct
  misc_feature 1..60: note = KRAB_MeCP2_dCas12f1_KRAB_Gibson_F
  source 1..60: mol_type = other DNA
cctccggactctagaggatcgaacccttgccaccatggcccccaagaagaagaggaaggt

SEQ ID NO: 477 - DNA, 60 bp, synthetic construct
  misc_feature 1..60: note = KRAB_MeCP2_dCas12f1_KRAB_Gibson_R
  source 1..60: mol_type = other DNA
ctgggactccgtggataccgaccttccgcttcttctttggtgagactctctcagtcacgg

SEQ ID NO: 478 - DNA, 23 bp, synthetic construct
  misc_feature 1..23: note = dCas12f1_DNMT3A_Vector_F
  source 1..23: mol_type = other DNA
tagaagaattcgatccctaccgg

SEQ ID NO: 479 - DNA, 22 bp, synthetic construct
  misc_feature 1..22: note = dCas12f1_DNMT3A_Vector_R
  source 1..22: mol_type = other DNA
ctttttcttttttgcctggccg

SEQ ID NO: 480 - DNA, 74 bp, synthetic construct
  misc_feature 1..74: note = dCas12f1_DNMT3A_Gibson_F
  source 1..74: mol_type = other DNA
ccaaaaggccggcggccacgaaaaaggccggccaggcaaaaaagaaaaagctcgagggcggaggcgggagcgga

SEQ ID NO: 481 - DNA, 60 bp, synthetic construct
  misc_feature 1..60: note = dCas12f1_DNMT3A_Gibson_R
  source 1..60: mol_type = other DNA
tttaaactcattactaaccggtagggatcgaattcttctacacacacgcaaaatactcct

SEQ ID NO: 482 - DNA, 21 bp, synthetic construct
  misc_feature 1..21: note = DNMT3A_dCas12f1_Vector_F
  source 1..21: mol_type = other DNA
tgaaagggttcgatccctacc

SEQ ID NO: 483 - DNA, 22 bp, synthetic construct
  misc_feature 1..22: note = DNMT3A_dCas12f1_Vector_R
  source 1..22: mol_type = other DNA
tggccggccgctgccgcctgag

SEQ ID NO: 484 - DNA, 60 bp, synthetic construct
  misc_feature 1..60: note = DNMT3A_dCas12f1_Gibson_F
  source 1..60: mol_type = other DNA
agcggcggttctggtggctcaggcggcagcggccggccaccaaagaagaagcggaaggtc

SEQ ID NO: 485 - DNA, 60 bp, synthetic construct
  misc_feature 1..60: note = DNMT3A_dCas12f1_Gibson_R
  source 1..60: mol_type = other DNA
ttaaactcattactaaccggtagggatcgaaccctttcactttttcttttttgcctggcc

SEQ ID NO: 486 - DNA, 22 bp, synthetic construct
  misc_feature 1..22: note = dCas12f1_hHDAC3_Vector_F
  source 1..22: mol_type = other DNA
aagaattcgatccctaccggtt

SEQ ID NO: 487 - DNA, 23 bp, synthetic construct
  misc_feature 1..23: note = dCas12f1_hHDAC3_Vector_R
  source 1..23: mol_type = other DNA
ctttttcttttttgcctggccgg

SEQ ID NO: 488 - DNA, 60 bp, synthetic construct
  misc_feature 1..60: note = dCas12f1_hHDAC3_Gibson_F
  source 1..60: mol_type = other DNA
ggcggccacgaaaaaggccggccaggcaaaaaagaaaaaggcggccgctggatccatggc

SEQ ID NO: 489 - DNA, 60 bp, synthetic construct
  misc_feature 1..60: note = dCas12f1_hHDAC3_Gibson_R
  source 1..60: mol_type = other DNA
ccgtttaaactcattactaaccggtagggatcgaattcttttaaatctccacatcgcttt

SEQ ID NO: 490 - DNA, 23 bp, synthetic construct
  misc_feature 1..23: note = dCas12f1_KRAB_KRAB_Vector_F
  source 1..23: mol_type = other DNA
tagaagaattcgatccctaccgg

SEQ ID NO: 491 - DNA, 22 bp, synthetic construct
  misc_feature 1..22: note = dCas12f1_KRAB_KRAB_Vector_R
  source 1..22: mol_type = other DNA
tgaggcttccaccttccgtttc

SEQ ID NO: 492 - DNA, 80 bp, synthetic construct
  misc_feature 1..80: note = dCas12f1_KRAB_KRAB_Gibson_F
  source 1..80: mol_type = other DNA
ggaggtggttcgggtggctctggatcaagcccaaagaagaaacggaaggtggaagcctcaagaacactggttacgttcaa

SEQ ID NO: 493 - DNA, 80 bp, synthetic construct
  misc_feature 1..80: note = dCas14_KRAB_KRAB_Ginson_R
  source 1..80: mol_type = other DNA
gtttcagttagcctcccccgtttaaactcattactaaccggtagggatcgaattcttctataccagccaaggttcttccc

SEQ ID NO: 494 - DNA, 18 bp, synthetic construct
  misc_feature 1..18: note = dCas12f1_K_K_MeCP2_Vector_F
  source 1..18: mol_type = other DNA
agtggtggaggaagtggc

SEQ ID NO: 495 - DNA, 22 bp, synthetic construct
  misc_feature 1..22: note = dCas12f1_K_K_MeCP2_Vector_R
  source 1..22: mol_type = other DNA
ctttttcttttttgcctggccg

SEQ ID NO: 496 - DNA, 60 bp, synthetic construct
  misc_feature 1..60: note = dCas12f1_K_K_MeCP2_Gibson_F
  source 1..60: mol_type = other DNA
ggcggccacgaaaaaggccggccaggcaaaaaagaaaaagagtggtggaggaagtggcgg

SEQ ID NO: 497 - DNA, 60 bp, synthetic construct
  misc_feature 1..60: note = dCas12f1_K_K_MeCP2_Gibson_R
  source 1..60: mol_type = other DNA
tcgcgtccatcgaccctgacccgccacttcctccaccacttaccagccaaggttcttccc

SEQ ID NO: 498 - DNA, 22 bp, synthetic construct
  misc_feature 1..22: note = KRAB_dCas12f1_MeCP2_Vector_R
  source 1..22: mol_type = other DNA
ctttttcttttttgcctggccg

SEQ ID NO: 499 - DNA, 21 bp, synthetic construct
  misc_feature 1..21: note = KRAB_dCas12f1_MeCP2_Vector_F
  source 1..21: mol_type = other DNA
tgaaagggttcgatccctacc

SEQ ID NO: 500 - DNA, 60 bp, synthetic construct
  misc_feature 1..60: note = KRAB_dCas12f1_MeCP2_Gibson_F
  source 1..60: mol_type = other DNA
ggcggccacgaaaaaggccggccaggcaaaaaagaaaaaggaagcctcagtgcaggtgaa

SEQ ID NO: 501 - DNA, 60 bp, synthetic construct
  misc_feature 1..60: note = KRAB_dCas12f1_MeCP2_Gibson_R
  source 1..60: mol_type = other DNA
tttaaactcattactaaccggtagggatcgaaccctttcatgagactctctcagtcacgg

SEQ ID NO: 502 - DNA, 20 bp, synthetic construct
  misc_feature 1..20: note = KRAB_MeCP2_dCas14_KRAB_Vector_R
  source 1..20: mol_type = other DNA
ggccatggtggcaagggttc

SEQ ID NO: 503 - DNA, 21 bp, synthetic construct
  misc_feature 1..21: note = KRAB_MeCP2_dCas14_KRAB_Vector_F
  source 1..21: mol_type = other DNA
ccaaagaagaagcggaaggtc

SEQ ID NO: 504 - DNA, 60 bp, synthetic construct; identical to SEQ ID NO: 476
  misc_feature 1..60: note = KRAB_MeCP2_dCas14_KRAB_Gibson_F
  source 1..60: mol_type = other DNA

SEQ ID NO: 505 - DNA, 60 bp, synthetic construct; identical to SEQ ID NO: 477
  misc_feature 1..60: note = KRAB_MeCP2_dCas14_KRAB_Gibson_R
  source 1..60: mol_type = other DNA

SEQ ID NO: 506 - DNA, 23 bp, synthetic construct
  misc_feature 1..23: note = MeCP2_dCas14_KRAB_Vector_F
  source 1..23: mol_type = other DNA
ccaaagaagaagcggaaggtcgg

SEQ ID NO: 507 - DNA, 20 bp, synthetic construct
  misc_feature 1..20: note = MeCP2_dCas14_KRAB_Vector_R
  source 1..20: mol_type = other DNA
ggccatggtggcaagggttc

SEQ ID NO: 508 - DNA, 60 bp, synthetic construct
  misc_feature 1..60: note = MeCP2_dCas14_KRAB_Gibson_F
  source 1..60: mol_type = other DNA
cctccggactctagaggatcgaacccttgccaccatggccccaaagaagaaacggaaggt

SEQ ID NO: 509 - DNA, 60 bp, synthetic construct; identical to SEQ ID NO: 477
  misc_feature 1..60: note = MeCP2_dCas14_KRAB_Gibson_R
  source 1..60: mol_type = other DNA

SEQ ID NO: 510 - protein, 8 aa, synthetic construct
  REGION 1..8: note = FLAG
DYKDDDDK

SEQ ID NO: 511 - protein, 734 aa, synthetic construct
  REGION 1..734: note = nls-linker-krab-linker-nls-dTnpB-nls
KRPAATKKAGQAKKKKSGGSSGGSSGSETPGTSESATPESSGGSSGGSRTLVTFKDVFVDFTREEWKLLDTAQQIVYRNVMLENYKNLVSLGYQLTKPDVILRLEKGEEPWLVSGGSSGGSSGSETPGTSESATPESSGGSSGGSKRPAATKKAGQAKKKKMGEKSSRRRRNGKSGAWTAAITSCVGGKMAKNTITKTLKLRIVRPYNSAEVEKIVADEKNNREKIALEKNKDKVKEACSKHLKVAAYCTTQVERNACLFCKARKLDDKFYQKLRGQFPDAVFWQEISEIFRQLQKQAAEIYNQSLIELYYEIFIKGKGIANASSVEHYLSDVCYTRAAELFKNAAIASGLRSKIKSNFRLKELKNMKSGLPTTKSDNFPIPLVKQKGGQYTGFEISNHNSDFIIKIPFGRWQVKKEIDKYRPWEKFDFEQVQKSPKPISLLLSTQRRKRNKGWSKDEGTEAEIKKVMNGDYQTSYIEVKRGSKIGEKSAWMLNLSIDVPKIDKGVDPSIIGGIDVGVKSPLVCAINNAFSRYSISDNDLFHFNKKMFARRRILLKKNRHKRAGHGAKNKLKPITILTEKSERFRKKLIERWACEIADFFIKNKVGTVQMENLESMKRKEDSYFNIRLRGFWPYAEMQNKIEFKLKQYGIEIRKVAPNNTSKTCSKCGHLNNYFNFEYAKKNKFPHFKCEKCNFKENADYNAALNISNPKLKSTKEEPKRPAATKKAGQAKKKK

SEQ ID NO: 512 - protein, 1052 aa, synthetic construct
  REGION 1..1052: note = nls-linker-flag-linker-dnmt3a-linker-nls-linker-dtnpb-nls
KRPAATKKAGQAKKKKSGGSSGGSSGSETPGTSESATPESSGGSSGGSDYKDDDDKSGGSSGGSSGSETPGTSESATPESSGGSSGGSPSRLQMFFANNHDQEFDPPKVYPPVPAEKRKPIRVLSLFDGIATGLLVLKDLGIQVDRYIASEVCEDSITVGMVRHQGKIMYVGDVRSVTQKHIQEWGPFDLVIGGSPCNDLSIVNPARKGLYEGTGRLFFEFYRLLHDARPKEGDDRPFFWLFENVVAMGVSDKRDISRFLESNPVMIDAKEVSAAHRARYFWGNLPGMNRPLASTVNDKLELQECLEHGRIAKFSKVRTITTRSNSIKQGKDQHFPVFMNEKEDILWCTEMERVFGFPVHYTDVSNMSRLARQRLLGRSWSVPVIRHLFAPLKEYFACVSGGSSGGSSGSETPGTSESATPESSGGSSGGSKRPAATKKAGQAKKKKSGGSSGGSSGSETPGTSESATPESSGGSSGGSMGEKSSRRRRNGKSGAWTAAITSCVGGKMAKNTITKTLKLRIVRPYNSAEVEKIVADEKNNREKIALEKNKDKVKEACSKHLKVAAYCTTQVERNACLFCKARKLDDKFYQKLRGQFPDAVFWQEISEIFRQLQKQAAEIYNQSLIELYYEIFIKGKGIANASSVEHYLSDVCYTRAAELFKNAAIASGLRSKIKSNFRLKELKNMKSGLPTTKSDNFPIPLVKQKGGQYTGFEISNHNSDFIIKIPFGRWQVKKEIDKYRPWEKFDFEQVQKSPKPISLLLSTQRRKRNKGWSKDEGTEAEIKKVMNGDYQTSYIEVKRGSKIGEKSAWMLNLSIDVPKIDKGVDPSIIGGIDVGVKSPLVCAINNAFSRYSISDNDLFHFNKKMFARRRILLKKNRHKRAGHGAKNKLKPITILTEKSERFRKKLIERWACEIADFFIKNKVGTVQMENLESMKRKEDSYFNIRLRGFWPYAEMQNKIEFKLKQYGIEIRKVAPNNTSKTCSKCGHLNNYFNFEYAKKNKFPHFKCEKCNFKENADYNAALNISNPKLKSTKEEPKRPAATKKAGQAKKKK

SEQ ID NO: 513 - protein, 1068 aa, synthetic construct
  REGION 1..1068: note = nls-linker-krab-linker-nls-mecp2-nls-linker-dtnpb-nls
KRPAATKKAGQAKKKKSGGSSGGSSGSETPGTSESATPESSGGSSGGSRTLVTFKDVFVDFTREEWKLLDTAQQIVYRNVMLENYKNLVSLGYQLTKPDVILRLEKGEEPWLVSGGSSGGSSGSETPGTSESATPESSGGSSGGSKRPAATKKAGQAKKKKVQVKRVLEKSPGKLLVKMPFQASPGGKGEGGGATTSAQVMVIKRPGRKRKAEADPQAIPKKRGRKPGSVVAAAAAEAKKKAVKESSIRSVQETVLPIKKRKTRETVSIEVKEVVKPLLVSTLGEKSGKGLKTCKSPGRKSKESSPKGRSSSASSPPKKEHHHHHHHAESPKAPMPLLPPPPPPEPQSSEDPISPPEPQDLSSSICKEEKMPRAGSLESDGCPKEPAKTQPMVAAAATTTTTTTTTVAEKYKHRGEGERKDIVSSSMPRPNREEPVDSRTPVTERVSKRPAATKKAGQAKKKKSGGSSGGSSGSETPGTSESATPESSGGSSGGSMGEKSSRRRRNGKSGAWTAAITSCVGGKMAKNTITKTLKLRIVRPYNSAEVEKIVADEKNNREKIALEKNKDKVKEACSKHLKVAAYCTTQVERNACLFCKARKLDDKFYQKLRGQFPDAVFWQEISEIFRQLQKQAAEIYNQSLIELYYEIFIKGKGIANASSVEHYLSDVCYTRAAELFKNAAIASGLRSKIKSNFRLKELKNMKSGLPTTKSDNFPIPLVKQKGGQYTGFEISNHNSDFIIKIPFGRWQVKKEIDKYRPWEKFDFEQVQKSPKPISLLLSTQRRKRNKGWSKDEGTEAEIKKVMNGDYQTSYIEVKRGSKIGEKSAWMLNLSIDVPKIDKGVDPSIIGGIDVGVKSPLVCAINNAFSRYSISDNDLFHFNKKMFARRRILLKKNRHKRAGHGAKNKLKPITILTEKSERFRKKLIERWACEIADFFIKNKVGTVQMENLESMKRKEDSYFNIRLRGFWPYAEMQNKIEFKLKQYGIEIRKVAPNNTSKTCSKCGHLNNYFNFEYAKKNKFPHFKCEKCNFKENADYNAALNISNPKLKSTKEEPKRPAATKKAGQAKKKK

SEQ ID NO: 514 - protein, 718 aa, synthetic construct
  REGION 1..718: note = nls-linker-dTnpB-nls-linker-krab
KRPAATKKAGQAKKKKSGGSSGGSSGSETPGTSESATPESSGGSSGGSMGEKSSRRRRNGKSGAWTAAITSCVGGKMAKNTITKTLKLRIVRPYNSAEVEKIVADEKNNREKIALEKNKDKVKEACSKHLKVAAYCTTQVERNACLFCKARKLDDKFYQKLRGQFPDAVFWQEISEIFRQLQKQAAEIYNQSLIELYYEIFIKGKGIANASSVEHYLSDVCYTRAAELFKNAAIASGLRSKIKSNFRLKELKNMKSGLPTTKSDNFPIPLVKQKGGQYTGFEISNHNSDFIIKIPFGRWQVKKEIDKYRPWEKFDFEQVQKSPKPISLLLSTQRRKRNKGWSKDEGTEAEIKKVMNGDYQTSYIEVKRGSKIGEKSAWMLNLSIDVPKIDKGVDPSIIGGIDVGVKSPLVCAINNAFSRYSISDNDLFHFNKKMFARRRILLKKNRHKRAGHGAKNKLKPITILTEKSERFRKKLIERWACEIADFFIKNKVGTVQMENLESMKRKEDSYFNIRLRGFWPYAEMQNKIEFKLKQYGIEIRKVAPNNTSKTCSKCGHLNNYFNFEYAKKNKFPHFKCEKCNFKENADYNAALNISNPKLKSTKEEPKRPAATKKAGQAKKKKSGGSSGGSSGSETPGTSESATPESSGGSSGGSRTLVTFKDVFVDFTREEWKLLDTAQQIVYRNVMLENYKNLVSLGYQLTKPDVILRLEKGEEPWLV

SEQ ID NO: 515 - protein, 1052 aa, synthetic construct
  REGION 1..1052: note = nls-linker-dtnpb-nls-linker-krab-linker-nls-mecp2
KRPAATKKAGQAKKKKSGGSSGGSSGSETPGTSESATPESSGGSSGGSMGEKSSRRRRNGKSGAWTAAITSCVGGKMAKNTITKTLKLRIVRPYNSAEVEKIVADEKNNREKIALEKNKDKVKEACSKHLKVAAYCTTQVERNACLFCKARKLDDKFYQKLRGQFPDAVFWQEISEIFRQLQKQAAEIYNQSLIELYYEIFIKGKGIANASSVEHYLSDVCYTRAAELFKNAAIASGLRSKIKSNFRLKELKNMKSGLPTTKSDNFPIPLVKQKGGQYTGFEISNHNSDFIIKIPFGRWQVKKEIDKYRPWEKFDFEQVQKSPKPISLLLSTQRRKRNKGWSKDEGTEAEIKKVMNGDYQTSYIEVKRGSKIGEKSAWMLNLSIDVPKIDKGVDPSIIGGIDVGVKSPLVCAINNAFSRYSISDNDLFHFNKKMFARRRILLKKNRHKRAGHGAKNKLKPITILTEKSERFRKKLIERWACEIADFFIKNKVGTVQMENLESMKRKEDSYFNIRLRGFWPYAEMQNKIEFKLKQYGIEIRKVAPNNTSKTCSKCGHLNNYFNFEYAKKNKFPHFKCEKCNFKENADYNAALNISNPKLKSTKEEPKRPAATKKAGQAKKKKSGGSSGGSSGSETPGTSESATPESSGGSSGGSRTLVTFKDVFVDFTREEWKLLDTAQQIVYRNVMLENYKNLVSLGYQLTKPDVILRLEKGEEPWLVSGGSSGGSSGSETPGTSESATPESSGGSSGGSKRPAATKKAGQAKKKKVQVKRVLEKSPGKLLVKMPFQASPGGKGEGGGATTSAQVMVIKRPGRKRKAEADPQAIPKKRGRKPGSVVAAAAAEAKKKAVKESSIRSVQETVLPIKKRKTRETVSIEVKEVVKPLLVSTLGEKSGKGLKTCKSPGRKSKESSPKGRSSSASSPPKKEHHHHHHHAESPKAPMPLLPPPPPPEPQSSEDPISPPEPQDLSSSICKEEKMPRAGSLESDGCPKEPAKTQPMVAAAATTTTTTTTTVAEKYKHRGEGERKDIVSSSMPRPNREEPVDSRTPVTERVS

SEQ ID NO: 516 - protein, 815 aa, synthetic construct
  REGION 1..815: note = nls-linker-dtnpb-nls-linker-krab-linker-krab
KRPAATKKAGQAKKKKSGGSSGGSSGSETPGTSESATPESSGGSSGGSMGEKSSRRRRNGKSGAWTAAITSCVGGKMAKNTITKTLKLRIVRPYNSAEVEKIVADEKNNREKIALEKNKDKVKEACSKHLKVAAYCTTQVERNACLFCKARKLDDKFYQKLRGQFPDAVFWQEISEIFRQLQKQAAEIYNQSLIELYYEIFIKGKGIANASSVEHYLSDVCYTRAAELFKNAAIASGLRSKIKSNFRLKELKNMKSGLPTTKSDNFPIPLVKQKGGQYTGFEISNHNSDFIIKIPFGRWQVKKEIDKYRPWEKFDFEQVQKSPKPISLLLSTQRRKRNKGWSKDEGTEAEIKKVMNGDYQTSYIEVKRGSKIGEKSAWMLNLSIDVPKIDKGVDPSIIGGIDVGVKSPLVCAINNAFSRYSISDNDLFHFNKKMFARRRILLKKNRHKRAGHGAKNKLKPITILTEKSERFRKKLIERWACEIADFFIKNKVGTVQMENLESMKRKEDSYFNIRLRGFWPYAEMQNKIEFKLKQYGIEIRKVAPNNTSKTCSKCGHLNNYFNFEYAKKNKFPHFKCEKCNFKENADYNAALNISNPKLKSTKEEPKRPAATKKAGQAKKKKSGGSSGGSSGSETPGTSESATPESSGGSSGGSRTLVTFKDVFVDFTREEWKLLDTAQQIVYRNVMLENYKNLVSLGYQLTKPDVILRLEKGEEPWLVSGGSSGGSSGSETPGTSESATPESSGGSSGGSRTLVTFKDVFVDFTREEWKLLDTAQQIVYRNVMLENYKNLVSLGYQLTKPDVILRLEKGEEPWLV

SEQ ID NO: 517 - protein, 1149 aa, synthetic construct
  REGION 1..1149: note = nls-linker-dtnpb-nls-linker-krab-linker-krab-linker-nls-mecp2
KRPAATKKAGQAKKKKSGGSSGGSSGSETPGTSESATPESSGGSSGGSMGEKSSRRRRNGKSGAWTAAITSCVGGKMAKNTITKTLKLRIVRPYNSAEVEKIVADEKNNREKIALEKNKDKVKEACSKHLKVAAYCTTQVERNACLFCKARKLDDKFYQKLRGQFPDAVFWQEISEIFRQLQKQAAEIYNQSLIELYYEIFIKGKGIANASSVEHYLSDVCYTRAAELFKNAAIASGLRSKIKSNFRLKELKNMKSGLPTTKSDNFPIPLVKQKGGQYTGFEISNHNSDFIIKIPFGRWQVKKEIDKYRPWEKFDFEQVQKSPKPISLLLSTQRRKRNKGWSKDEGTEAEIKKVMNGDYQTSYIEVKRGSKIGEKSAWMLNLSIDVPKIDKGVDPSIIGGIDVGVKSPLVCAINNAFSRYSISDNDLFHFNKKMFARRRILLKKNRHKRAGHGAKNKLKPITILTEKSERFRKKLIERWACEIADFFIKNKVGTVQMENLESMKRKEDSYFNIRLRGFWPYAEMQNKIEFKLKQYGIEIRKVAPNNTSKTCSKCGHLNNYFNFEYAKKNKFPHFKCEKCNFKENADYNAALNISNPKLKSTKEEPKRPAATKKAGQAKKKKSGGSSGGSSGSETPGTSESATPESSGGSSGGSRTLVTFKDVFVDFTREEWKLLDTAQQIVYRNVMLENYKNLVSLGYQLTKPDVILRLEKGEEPWLVSGGSSGGSSGSETPGTSESATPESSGGSSGGSRTLVTFKDVFVDFTREEWKLLDTAQQIVYRNVMLENYKNLVSLGYQLTKPDVILRLEKGEEPWLVSGGSSGGSSGSETPGTSESATPESSGGSSGGSKRPAATKKAGQAKKKKVQVKRVLEKSPGKLLVKMPFQASPGGKGEGGGATTSAQVMVIKRPGRKRKAEADPQAIPKKRGRKPGSVVAAAAAEAKKKAVKESSIRSVQETVLPIKKRKTRETVSIEVKEVVKPLLVSTLGEKSGKGLKTCKSPGRKSKESSPKGRSSSASSPPKKEHHHHHHHAESPKAPMPLLPPPPPPEPQSSEDPISPPEPQDLSSSICKEEKMPRAGSLESDGCPKEPAKTQPMVAAAATTTTTTTTTVAEKYKHRGEGERKDIVSSSMPRPNREEPVDSRTPVTERVS

SEQ ID NO: 518 - protein, 1081 aa, synthetic construct
  REGION 1..1081: note = nls-linker-dtnpb-nls-linker-hHDAC3
KRPAATKKAGQAKKKKSGGSSGGSSGSETPGTSESATPESSGGSSGGSMGEKSSRRRRNGKSGAWTAAITSCVGGKMAKNTITKTLKLRIVRPYNSAEVEKIVADEKNNREKIALEKNKDKVKEACSKHLKVAAYCTTQVERNACLFCKARKLDDKFYQKLRGQFPDAVFWQEISEIFRQLQKQAAEIYNQSLIELYYEIFIKGKGIANASSVEHYLSDVCYTRAAELFKNAAIASGLRSKIKSNFRLKELKNMKSGLPTTKSDNFPIPLVKQKGGQYTGFEISNHNSDFIIKIPFGRWQVKKEIDKYRPWEKFDFEQVQKSPKPISLLLSTQRRKRNKGWSKDEGTEAEIKKVMNGDYQTSYIEVKRGSKIGEKSAWMLNLSIDVPKIDKGVDPSIIGGIDVGVKSPLVCAINNAFSRYSISDNDLFHFNKKMFARRRILLKKNRHKRAGHGAKNKLKPITILTEKSERFRKKLIERWACEIADFFIKNKVGTVQMENLESMKRKEDSYFNIRLRGFWPYAEMQNKIEFKLKQYGIEIRKVAPNNTSKTCSKCGHLNNYFNFEYAKKNKFPHFKCEKCNFKENADYNAALNISNPKLKSTKEEPKRPAATKKAGQAKKKKSGGSSGGSSGSETPGTSESATPESSGGSSGGSMAKTVAYFYDPDVGNFHYGAGHPMKPHRLALTHSLVLHYGLYKKMIVFKPYQASQHDMCRFHSEDYIDFLQRVSPTNMQGFTKSLNAFNVGDDCPVFPGLFEFCSRYTGASLQGATQLNNKICDIAINWAGGLHHAKKFEASGFCYVNDIVIGILELLKYHPRVLYIDIDIHHGDGVQEAFYLTDRVMTVSFHKYGNYFFPGTGDMYEVGAESGRYYCLNVPLRDGIDDQSYKHLFQPVINQVVDFYQPTCIVLQCGADSLGCDRLGCFNLSIRGHGECVEYVKSFNIPLLVLGGGGYTVRNVARCWTYETSLLVEEAISEELPYSEYFEYFAPDFTLHPDVSTRIENQNSRQYLDQIRQTIFENLKMLNHAPSVQIHDVPADLLTYDRTDEADAEERGPEENYSRPEAPNEFYDGDHDNDKESDVEI

SEQ ID NO: 519 - protein, 1092 aa, synthetic construct
  REGION 1..1092: note = nls-linker-FLAG-linker-krab-linker-nls-linker-dtnpb-nls-mecp2
KRPAATKKAGQAKKKKSGGSSGGSSGSETPGTSESATPESSGGSSGGSDYKDDDDKSGGSSGGSSGSETPGTSESATPESSGGSSGGSRTLVTFKDVFVDFTREEWKLLDTAQQIVYRNVMLENYKNLVSLGYQLTKPDVILRLEKGEEPWLVSGGSSGGSSGSETPGTSESATPESSGGSSGGSKRPAATKKAGQAKKKKSGGSSGGSSGSETPGTSESATPESSGGSSGGSMGEKSSRRRRNGKSGAWTAAITSCVGGKMAKNTITKTLKLRIVRPYNSAEVEKIVADEKNNREKIALEKNKDKVKEACSKHLKVAAYCTTQVERNACLFCKARKLDDKFYQKLRGQFPDAVFWQEISEIFRQLQKQAAEIYNQSLIELYYEIFIKGKGIANASSVEHYLSDVCYTRAAELFKNAAIASGLRSKIKSNFRLKELKNMKSGLPTTKSDNFPIPLVKQKGGQYTGFEISNHNSDFIIKIPFGRWQVKKEIDKYRPWEKFDFEQVQKSPKPISLLLSTQRRKRNKGWSKDEGTEAEIKKVMNGDYQTSYIEVKRGSKIGEKSAWMLNLSIDVPKIDKGVDPSIIGGIDVGVKSPLVCAINNAFSRYSISDNDLFHFNKKMFARRRILLKKNRHKRAGHGAKNKLKPITILTEKSERFRKKLIERWACEIADFFIKNKVGTVQMENLESMKRKEDSYFNIRLRGFWPYAEMQNKIEFKLKQYGIEIRKVAPNNTSKTCSKCGHLNNYFNFEYAKKNKFPHFKCEKCNFKENADYNAALNISNPKLKSTKEEPKRPAATKKAGQAKKKKVQVKRVLEKSPGKLLVKMPFQASPGGKGEGGGATTSAQVMVIKRPGRKRKAEADPQAIPKKRGRKPGSVVAAAAAEAKKKAVKESSIRSVQETVLPIKKRKTRETVSIEVKEVVKPLLVSTLGEKSGKGLKTCKSPGRKSKESSPKGRSSSASSPPKKEHHHHHHHAESPKAPMPLLPPPPPPEPQSSEDPISPPEPQDLSSSICKEEKMPRAGSLESDGCPKEPAKTQPMVAAAATTTTTTTTTVAEKYKHRGEGERKDIVSSSMPRPNREEPVDSRTPVTERVS

SEQ ID NO: 520 - protein, 1165 aa, synthetic construct
  REGION 1..1165: note = nls-linker-krab-linker-nls-mecp2-nls-linker-dtnpb-nls-linker-krab
KRPAATKKAGQAKKKKSGGSSGGSSGSETPGTSESATPESSGGSSGGSRTLVTFKDVFVDFTREEWKLLDTAQQIVYRNVMLENYKNLVSLGYQLTKPDVILRLEKGEEPWLVSGGSSGGSSGSETPGTSESATPESSGGSSGGSKRPAATKKAGQAKKKKVQVKRVLEKSPGKLLVKMPFQASPGGKGEGGGATTSAQVMVIKRPGRKRKAEADPQAIPKKRGRKPGSVVAAAAAEAKKKAVKESSIRSVQETVLPIKKRKTRETVSIEVKEVVKPLLVSTLGEKSGKGLKTCKSPGRKSKESSPKGRSSSASSPPKKEHHHHHHHAESPKAPMPLLPPPPPPEPQSSEDPISPPEPQDLSSSICKEEKMPRAGSLESDGCPKEPAKTQPMVAAAATTTTTTTTTVAEKYKHRGEGERKDIVSSSMPRPNREEPVDSRTPVTERVSKRPAATKKAGQAKKKKSGGSSGGSSGSETPGTSESATPESSGGSSGGSMGEKSSRRRRNGKSGAWTAAITSCVGGKMAKNTITKTLKLRIVRPYNSAEVEKIVADEKNNREKIALEKNKDKVKEACSKHLKVAAYCTTQVERNACLFCKARKLDDKFYQKLRGQFPDAVFWQEISEIFRQLQKQAAEIYNQSLIELYYEIFIKGKGIANASSVEHYLSDVCYTRAAELFKNAAIASGLRSKIKSNFRLKELKNMKSGLPTTKSDNFPIPLVKQKGGQYTGFEISNHNSDFIIKIPFGRWQVKKEIDKYRPWEKFDFEQVQKSPKPISLLLSTQRRKRNKGWSKDEGTEAEIKKVMNGDYQTSYIEVKRGSKIGEKSAWMLNLSIDVPKIDKGVDPSIIGGIDVGVKSPLVCAINNAFSRYSISDNDLFHFNKKMFARRRILLKKNRHKRAGHGAKNKLKPITILTEKSERFRKKLIERWACEIADFFIKNKVGTVQMENLESMKRKEDSYFNIRLRGFWPYAEMQNKIEFKLKQYGIEIRKVAPNNTSKTCSKCGHLNNYFNFEYAKKNKFPHFKCEKCNFKENADYNAALNISNPKLKSTKEEPKRPAATKKAGQAKKKKSGGSSGGSSGSETPGTSESATPESSGGSSGGSRTLVTFKDVFVDFTREEWKLLDTAQQIVYRNVMLENYKNLVSLGYQLTKPDVILRLEKGEEPWLV

SEQ ID NO: 521 - protein, 1020 aa, synthetic construct
  REGION 1..1020: note = nls-mecp2-nls-linker-dtnpb-nls-linker-krab
KRPAATKKAGQAKKKKVQVKRVLEKSPGKLLVKMPFQASPGGKGEGGGATTSAQVMVIKRPGRKRKAEADPQAIPKKRGRKPGSVVAAAAAEAKKKAVKESSIRSVQETVLPIKKRKTRETVSIEVKEVVKPLLVSTLGEKSGKGLKTCKSPGRKSKESSPKGRSSSASSPPKKEHHHHHHHAESPKAPMPLLPPPPPPEPQSSEDPISPPEPQDLSSSICKEEKMPRAGSLESDGCPKEPAKTQPMVAAAATTTTTTTTTVAEKYKHRGEGERKDIVSSSMPRPNREEPVDSRTPVTERVSKRPAATKKAGQAKKKKSGGSSGGSSGSETPGTSESATPESSGGSSGGSMGEKSSRRRRNGKSGAWTAAITSCVGGKMAKNTITKTLKLRIVRPYNSAEVEKIVADEKNNREKIALEKNKDKVKEACSKHLKVAAYCTTQVERNACLFCKARKLDDKFYQKLRGQFPDAVFWQEISEIFRQLQKQAAEIYNQSLIELYYEIFIKGKGIANASSVEHYLSDVCYTRAAELFKNAAIASGLRSKIKSNFRLKELKNMKSGLPTTKSDNFPIPLVKQKGGQYTGFEISNHNSDFIIKIPFGRWQVKKEIDKYRPWEKFDFEQVQKSPKPISLLLSTQRRKRNKGWSKDEGTEAEIKKVMNGDYQTSYIEVKRGSKIGEKSAWMLNLSIDVPKIDKGVDPSIIGGIDVGVKSPLVCAINNAFSRYSISDNDLFHFNKKMFARRRILLKKNRHKRAGHGAKNKLKPITILTEKSERFRKKLIERWACEIADFFIKNKVGTVQMENLESMKRKEDSYFNIRLRGFWPYAEMQNKIEFKLKQYGIEIRKVAPNNTSKTCSKCGHLNNYFNFEYAKKNKFPHFKCEKCNFKENADYNAALNISNPKLKSTKEEPKRPAATKKAGQAKKKKSGGSSGGSSGSETPGTSESATPESSGGSSGGSRTLVTFKDVFVDFTREEWKLLDTAQQIVYRNVMLENYKNLVSLGYQLTKPDVILRLEKGEEPWLV

SEQ ID NO: 522 - DNA, 23 bp, synthetic construct
  source 1..23: mol_type = other DNA
  misc_feature 1..23: note = protospacer sequence for experimental example 5
cacacacacagtgggctaccatt

SEQ ID NO: 523 - DNA, 23 bp, synthetic construct
  source 1..23: mol_type = other DNA
  misc_feature 1..23: note = D360A, Forward primer
cggagggatcgctgtgggggtca

SEQ ID NO: 524 - DNA, 23 bp, synthetic construct
  source 1..23: mol_type = other DNA
  misc_feature 1..23: note = E422A, Forward primer
agtgcagatggcgaacctcgaga

SEQ ID NO: 525 - DNA, 25 bp, synthetic construct
  source 1..25: mol_type = other DNA
  misc_feature 1..25: note = R490A, Forward primer
cttcgagtacgcgaagaagaacaag

SEQ ID NO: 526 - DNA, 25 bp, synthetic construct
  source 1..25: mol_type = other DNA
  misc_feature 1..25: note = R490Q, Forward primer
cttcgagtaccagaagaagaacaag

SEQ ID NO: 527 - DNA, 25 bp, synthetic construct
  source 1..25: mol_type = other DNA
  misc_feature 1..25: note = R490W, Forward primer
cttcgagtactggaagaagaacaag

SEQ ID NO: 528 - DNA, 25 bp, synthetic construct
  source 1..25: mol_type = other DNA
  misc_feature 1..25: note = R490L, Forward primer
cttcgagtacctgaagaagaacaag

SEQ ID NO: 529 - DNA, 23 bp, synthetic construct
  source 1..23: mol_type = other DNA
  misc_feature 1..23: note = D510A, Forward primer
ggagaacgccgcttacaacgccg

SEQ ID NO: 530 - DNA, 23 bp, synthetic construct
  source 1..23: mol_type = other DNA
  misc_feature 1..23: note = D510L, Forward primer
ggagaacgccctttacaacgccg

SEQ ID NO: 531 - DNA, 23 bp, synthetic construct
  source 1..23: mol_type = other DNA
  misc_feature 1..23: note = D510V, Forward primer
ggagaacgccgtatacaacgccg

SEQ ID NO: 532 - DNA, 19 bp, synthetic construct
  source 1..19: mol_type = other DNA
  misc_feature 1..19: note = D360A, Reverse primer
atgatgctgggatccacgc

SEQ ID NO: 533 - DNA, 24 bp, synthetic construct
  source 1..24: mol_type = other DNA
  misc_feature 1..24: note = E422A, Reverse primer
gttccgaccttgttcttaataaag

SEQ ID NO: 534 - DNA, 18 bp, synthetic construct
  source 1..18: mol_type = other DNA
  misc_feature 1..18: note = R490A, Reverse primer
ttgaagtagttgttgagg

SEQ ID NO: 535 - DNA, 18 bp, synthetic construct
  source 1..18: mol_type = other DNA
  misc_feature 1..18: note = R490Q, Reverse primer
ttgaagtagttgttgagg

SEQ ID NO: 536 - DNA, 20 bp, synthetic construct
  source 1..20: mol_type = other DNA
  misc_feature 1..20: note = R490W, Reverse primer
ttgaagtagttgttgaggtg

SEQ ID NO: 537 - DNA, 18 bp, synthetic construct
  source 1..18: mol_type = other DNA
  misc_feature 1..18: note = R490L, Reverse primer
ttgaagtagttgttgagg

SEQ ID NO: 538 - DNA, 19 bp, synthetic construct
  source 1..19: mol_type = other DNA
  misc_feature 1..19: note = D510A, Reverse primer
ttaaagttgcacttctcgc

SEQ ID NO: 539 - DNA, 18 bp, synthetic construct
  source 1..18: mol_type = other DNA
  misc_feature 1..18: note = D510L, Reverse primer
ttaaagttgcacttctcg

SEQ ID NO: 540 - DNA, 19 bp, synthetic construct
  source 1..19: mol_type = other DNA
  misc_feature 1..19: note = D510V, Reverse primer
ttaaagttgcacttctcgc